European Patent Specification EP 3 539 573 B1, published February 14, 2024. Title: RNA-GUIDED GENE EDITING AND GENE REGULATION. Applicant: DUKE UNIVERSITY. Application not yet assigned. The sequence listing filed with the application follows.

SEQUENCE LISTING (676 sequences)

SEQ ID NO: 1 - protein, 1483 aa, Artificial Sequence
  source: /note="Description of Artificial Sequence: Synthetic polypeptide"
MDYKDHDGDYKDHDIDYKDDDDKMAPKKKRKVGRGMDKKYSIGLAIGTNSVGWAVITDEYKVPSKKFKVLGNTDRHSIKKNLIGALLFDSGETAEATRLKRTARRRYTRRKNRICYLQEIFSNEMAKVDDSFFHRLEESFLVEEDKKHERHPIFGNIVDEVAYHEKYPTIYHLRKKLVDSTDKADLRLIYLALAHMIKFRGHFLIEGDLNPDNSDVDKLFIQLVQTYNQLFEENPINASGVDAKAILSARLSKSRRLENLIAQLPGEKKNGLFGNLIALSLGLTPNFKSNFDLAEDAKLQLSKDTYDDDLDNLLAQIGDQYADLFLAAKNLSDAILLSDILRVNTEITKAPLSASMIKRYDEHHQDLTLLKALVRQQLPEKYKEIFFDQSKNGYAGYIDGGASQEEFYKFIKPILEKMDGTEELLVKLNREDLLRKQRTFDNGSIPHQIHLGELHAILRRQEDFYPFLKDNREKIEKILTFRIPYYVGPLARGNSRFAWMTRKSEETITPWNFEEVVDKGASAQSFIERMTNFDKNLPNEKVLPKHSLLYEYFTVYNELTKVKYVTEGMRKPAFLSGEQKKAIVDLLFKTNRKVTVKQLKEDYFKKIECFDSVEISGVEDRFNASLGTYHDLLKIIKDKDFLDNEENEDILEDIVLTLTLFEDREMIEERLKTYAHLFDDKVMKQLKRRRYTGWGRLSRKLINGIRDKQSGKTILDFLKSDGFANRNFMQLIHDDSLTFKEDIQKAQVSGQGDSLHEHIANLAGSPAIKKGILQTVKVVDELVKVMGRHKPENIVIEMARENQTTQKGQKNSRERMKRIEEGIKELGSQILKEHPVENTQLQNEKLYLYYLQNGRDMYVDQELDINRLSDYDVDAIVPQSFLKDDSIDNKVLTRSDKNRGKSDNVPSEEVVKKMKNYWRQLLNAKLITQRKFDNLTKAERGGLSELDKAGFIKRQLVETRQITKHVAQILDSRMNTKYDENDKLIREVKVITLKSKLVSDFRKDFQFYKVREINNYHHAHDAYLNAVVGTALIKKYPKLESEFVYGDYKVYDVRKMIAKSEQEIGKATAKYFFYSNIMNFFKTEITLANGEIRKRPLIETNGETGEIVWDKGRDFATVRKVLSMPQVNIVKKTEVQTGGFSKESILPKRNSDKLIARKKDWDPKKYGGFDSPTVAYSVLVVAKVEKGKSKKLKSVKELLGITIMERSSFEKNPIDFLEAKGYKEVKKDLIIKLPKYSLFELENGRKRMLASAGELQKGNELALPSKYVNFLYLASHYEKLKGSPEDNEQKQLFVEQHKHYLDEIIEQISEFSKRVILADANLDKVLSAYNKHRDKPIREQAENIIHLFTLTNLGAPAAFKYFDTTIDRKRYTSTKEVLDATLIHQSITGLYETRIDLSQLGGDPIAGSKASPKKKRKVGRADALDDFDLDMLGSDALDDFDLDMLGSDALDDFDLDMLGSDALDDFDLDMLINYPYDVPDYAS

SEQ ID NO: 2 - DNA, 350 bp, Artificial Sequence
  source: /note="Description of Artificial Sequence: Synthetic polynucleotide"
gagggcctatttcccatgattccttcatatttgcatatacgatacaaggctgttagagagataattggaattaatttgactgtaaacacaaagatattagtacaaaatacgtgacgtagaaagtaataatttcttgggtagtttgcagttttaaaattatgttttaaaatggactatcatatgcttatcgtaacttgaaagtatttcgatttcttggctttatatatcttgtggaaaggacgaaacaccgggtcttcgagaagacctgttttagagctagaaatagcaagttaaaataaggctagtccgttatcaacttgaaaaagtggcaccgagtcggtgcttttttt

SEQ ID NO: 3 - DNA, 338 bp, Homo sapiens
acccccggcagcagcccgccccgagcgcgccgcctgtttattcagccgggagtccggcacgcgccaggcgcacgcactgcaacaacaaacccagctgaatggagagtttgcaaggagcgggagaaaggaacgggagggggggagaggagaggaggagggggagtttagggagtgggtgggaggaagaggtaagaggaggggggggagtgggggctgcagccgctcgctgcagcagcggggagtggggggcgaggcggggccagggctgcgcgtggggctgggtgtcccattgaaaaggcggacgcactccggcagcccagcactctctcacttctggc

SEQ ID NO: 4 - DNA, 305 bp, Mus musculus
ccgccccgagcgcgcggcctgtttattcagccgggagtccggcacgcgccgggcgcacgcactgcaacaacaaaccaggctgaatggagagtttgcaaggagcgggcgcgggcaactggagggggggggggcgagagggagggagctgaggaggtgggggaagaggaggggtagtgggggctgcagccgctcgctgcagcagcggggagtggggggcgaggcggggccagggctgcgcgtggggctgggtgtcccattgaaaaggcggccgcaccgcagccgcccagcagtctctcacttctggc

SEQ ID NO: 5 - DNA, 19 bp, Artificial Sequence
  source: /note="Description of Artificial Sequence: Synthetic oligonucleotide"
gctgggtgtcccattgaaa

SEQ ID NO: 6 - DNA, 19 bp, Artificial Sequence
  source: /note="Description of Artificial Sequence: Synthetic oligonucleotide"
cagccgctcgctgcagcag

SEQ ID NO: 7 - DNA, 19 bp, Artificial Sequence
  source: /note="Description of Artificial Sequence: Synthetic oligonucleotide"
tggagagtttgcaaggagc

SEQ ID NO: 8 - DNA, 19 bp, Artificial Sequence
  source: /note="Description of Artificial Sequence: Synthetic oligonucleotide"
gtttattcagccgggagtc

SEQ ID NO: 9 - DNA, 20 bp, Artificial Sequence
  source: /note="Description of Artificial Sequence: Synthetic oligonucleotide"
cgccaggaggggtgggtcta

SEQ ID NO: 10 - DNA, 19 bp, Artificial Sequence
  source: /note="Description of Artificial Sequence: Synthetic oligonucleotide"
ccttggtgagactggtaga

SEQ ID NO: 11 - DNA, 19 bp, Artificial Sequence
  source: /note="Description of Artificial Sequence: Synthetic oligonucleotide"
gtcttcaggttctgttgct

SEQ ID NO: 12 - DNA, 19 bp, Artificial Sequence
  source: /note="Description of Artificial Sequence: Synthetic oligonucleotide"
atattcctgatttaaaagt

SEQ ID NO: 13 - DNA, 19 bp, Artificial Sequence
  source: /note="Description of Artificial Sequence: Synthetic oligonucleotide"
ttaaaagtcggctggtagc

SEQ ID NO: 14 - DNA, 19 bp, Artificial Sequence
  source: /note="Description of Artificial Sequence: Synthetic oligonucleotide"
cgggccgggggcggggtcc

SEQ ID NO: 15 - DNA, 19 bp, Artificial Sequence
  source: /note="Description of Artificial Sequence: Synthetic oligonucleotide"
gcccgagccgcgtgtggaa

SEQ ID NO: 16 - DNA, 19 bp, Artificial Sequence
  source: /note="Description of Artificial Sequence: Synthetic oligonucleotide"
ccttcattgcggcgggctg

SEQ ID NO: 17 - DNA, 19 bp, Artificial Sequence
  source: /note="Description of Artificial Sequence: Synthetic oligonucleotide"
ccgacccctcccgggtccc

SEQ ID NO: 18 - DNA, 19 bp, Artificial Sequence
  source: /note="Description of Artificial Sequence: Synthetic oligonucleotide"
caggaccgcgcttcccacg

SEQ ID NO: 19 - DNA, 19 bp, Artificial Sequence
  source: /note="Description of Artificial Sequence: Synthetic oligonucleotide"
tgcaccctgggagcgcgag

SEQ ID NO: 20 - DNA, 19 bp, Artificial Sequence
  source: /note="Description of Artificial Sequence: Synthetic oligonucleotide"
ccgcacgcacctgttccca

SEQ ID NO: 21 - DNA, 19 bp, Artificial Sequence
  source: /note="Description of Artificial Sequence: Synthetic oligonucleotide"
aaaacagcgagggagaaac

SEQ ID NO: 22 - DNA, 19 bp, Artificial Sequence
  source: /note="Description of Artificial Sequence: Synthetic oligonucleotide"
ttaacttgattgtgaaatc

SEQ ID NO: 23 - DNA, 19 bp, Artificial Sequence
  source: /note="Description of Artificial Sequence: Synthetic oligonucleotide"
aaaacaatgcatatttgca

SEQ ID NO: 24 - DNA, 19 bp, Artificial Sequence
  source: /note="Description of Artificial Sequence: Synthetic oligonucleotide"
aaaatccagtattttaatg

SEQ ID NO: 25 - DNA, 19 bp, Artificial Sequence
  source: /note="Description of Artificial Sequence: Synthetic oligonucleotide"
acccagcactgcagcctgg

SEQ ID NO: 26 - DNA, 19 bp, Artificial Sequence
  source: /note="Description of Artificial Sequence: Synthetic oligonucleotide"
aacttatgcggcgtttcct

SEQ ID NO: 27 - DNA, 19 bp, Artificial Sequence
  source: /note="Description of Artificial Sequence: Synthetic oligonucleotide"
tcactttaaaaccacctct

SEQ ID NO: 28 - DNA, 19 bp, Artificial Sequence
  source: /note="Description of Artificial Sequence: Synthetic oligonucleotide"
gcatctttttctctttaat

SEQ ID NO: 29 - DNA, 19 bp, Artificial Sequence
  source: /note="Description of Artificial Sequence: Synthetic oligonucleotide"
tgtactctctgaggtgctc

SEQ ID NO: 30 - DNA, 19 bp, Artificial Sequence
  source: /note="Description of Artificial Sequence: Synthetic oligonucleotide"
acgcagataagaaccagtt

SEQ ID NO: 31 - DNA, 19 bp, Artificial Sequence
  source: /note="Description of Artificial Sequence: Synthetic oligonucleotide"
catcaagtcagccatcagc

SEQ ID NO: 32 - DNA, 19 bp, Artificial Sequence
  source: /note="Description of Artificial Sequence: Synthetic oligonucleotide"
gagtcaccctcctggaaac

SEQ ID NO: 33 - DNA, 19 bp, Artificial Sequence
  source: /note="Description of Artificial Sequence: Synthetic oligonucleotide"
gctagggatgaagaataaa

SEQ ID NO: 34 - DNA, 19 bp, Artificial Sequence
  source: /note="Description of Artificial Sequence: Synthetic oligonucleotide"
ttgaccaatagccttgaca

SEQ ID NO: 35 - DNA, 19 bp, Artificial Sequence
  source: /note="Description of Artificial Sequence: Synthetic oligonucleotide"
tgcaaatatctgtctgaaa

SEQ ID NO: 36 - DNA, 19 bp, Artificial Sequence
  source: /note="Description of Artificial Sequence: Synthetic oligonucleotide"
aaattagcagtatcctctt

SEQ ID NO: 37 - DNA, 19 bp, Artificial Sequence
  source: /note="Description of Artificial Sequence: Synthetic oligonucleotide"
cctgggctccggggcgttt

SEQ ID NO: 38 - DNA, 19 bp, Artificial Sequence
  source: /note="Description of Artificial Sequence: Synthetic oligonucleotide"
ggcccctgcggccaccccg

SEQ ID NO: 39 - DNA, 19 bp, Artificial Sequence
  source: /note="Description of Artificial Sequence: Synthetic oligonucleotide"
ctccctccctgcccggtag

SEQ ID NO: 40 - DNA, 19 bp, Artificial Sequence
  source: /note="Description of Artificial Sequence: Synthetic oligonucleotide"
aggtttggaaagggcgtgc

SEQ ID NO: 41 - DNA, 20 bp, Artificial Sequence
  source: /note="Description of Artificial Sequence: Synthetic primer"
ggagcttctcgacttcacca

SEQ ID NO: 42 - DNA, 20 bp, Artificial Sequence
  source: /note="Description of Artificial Sequence: Synthetic primer"
gatttgtgggcctgaagaaa

SEQ ID NO: 43 - DNA, 20 bp, Artificial Sequence
  source: /note="Description of Artificial Sequence: Synthetic primer"
aaggaggagggcagaatcat

SEQ ID NO: 44 - DNA, 21 bp, Artificial Sequence
  source: /note="Description of Artificial Sequence: Synthetic primer"
aaaccttcctcagctatgccc

SEQ ID NO: 45 - DNA, 20 bp, Artificial Sequence
  source: /note="Description of Artificial Sequence: Synthetic primer"
agctgatggccctaaacaga

SEQ ID NO: 46 - DNA, 20 bp, Artificial Sequence
  source: /note="Description of Artificial Sequence: Synthetic primer"
caggaggactctggcaccta

SEQ ID NO: 47 - DNA, 20 bp, Artificial Sequence
  source: /note="Description of Artificial Sequence: Synthetic primer"
ggaatccatggagggaagat

SEQ ID NO: 48 - DNA, 21 bp, Artificial Sequence
  source: /note="Description of Artificial Sequence: Synthetic primer"
gctgagtgaactgcactgtga

SEQ ID NO: 49 - DNA, 20 bp, Artificial Sequence
  source: /note="Description of Artificial Sequence: Synthetic primer"
ctctctgctcctttgccaca

SEQ ID NO: 50 - DNA, 20 bp, Artificial Sequence
  source: /note="Description of Artificial Sequence: Synthetic primer"
caatgaccccttcattgacc

SEQ ID NO: 51 - DNA, 20 bp, Artificial Sequence
  source: /note="Description of Artificial Sequence: Synthetic primer"
ggaacaagagctgctggact

SEQ ID NO: 52 - DNA, 20 bp, Artificial Sequence
  source: /note="Description of Artificial Sequence: Synthetic primer"
aactttggcattgtggaagg

SEQ ID NO: 53 - DNA, 20 bp, Artificial Sequence
  source: /note="Description of Artificial Sequence: Synthetic primer"
aacgccactgacaagaaagc

SEQ ID NO: 54 - DNA, 20 bp, Artificial Sequence
  source: /note="Description of Artificial Sequence: Synthetic primer"
cagatccatggaggaaggaa

SEQ ID NO: 55 - DNA, 21 bp, Artificial Sequence
  source: /note="Description of Artificial Sequence: Synthetic primer"
gggtactcctggaagatgtcc

SEQ ID NO: 56 - DNA, 20 bp, Artificial Sequence
  source: /note="Description of Artificial Sequence: Synthetic primer"
gtttgcgacgcatgttcctc

SEQ ID NO: 57 - DNA, 20 bp, Artificial Sequence
  source: /note="Description of Artificial Sequence: Synthetic primer"
aagcccttgctgtagtggtg

SEQ ID NO: 58 - DNA, 20 bp, Artificial Sequence
  source: /note="Description of Artificial Sequence: Synthetic primer"
cggcaggaaagcatctgtat

SEQ ID NO: 59 - DNA, 20 bp, Artificial Sequence
  source: /note="Description of Artificial Sequence: Synthetic primer"
tgttctcgctcaggtcagtg

SEQ ID NO: 60 - DNA, 20 bp, Artificial Sequence
  source: /note="Description of Artificial Sequence: Synthetic primer"
gaattctttgccgaaatgga

SEQ ID NO: 61 - DNA, 20 bp, Artificial Sequence
  source: /note="Description of Artificial Sequence: Synthetic primer"
gtgctcttcgggtttcagga

SEQ ID NO: 62 - DNA, 20 bp, Artificial Sequence
  source: /note="Description of Artificial Sequence: Synthetic primer"
ttgattttggagggatctcg

SEQ ID NO: 63 - DNA, 20 bp, Artificial Sequence
  source: /note="Description of Artificial Sequence: Synthetic primer"
gtttttctgcctccccattt

SEQ ID NO: 64 - DNA, 20 bp, Artificial Sequence
  source: /note="Description of Artificial Sequence: Synthetic primer"
ggatgcagggatgatgttct

SEQ ID NO: 65 - DNA, 20 bp, Artificial Sequence
  source: /note="Description of Artificial Sequence: Synthetic oligonucleotide"
gattggctttgatttcccta

SEQ ID NO: 66 - DNA, 23 bp, Artificial Sequence
  source: /note="Description of Artificial Sequence: Synthetic oligonucleotide"
gtgtagagtaagtcagcctatgg

SEQ ID NO: 67 - DNA, 20 bp, Artificial Sequence
  source: /note="Description of Artificial Sequence: Synthetic oligonucleotide"
gcctactcagactgttactc

SEQ ID NO: 68 - DNA, 23 bp, Artificial Sequence
  source: /note="Description of Artificial Sequence: Synthetic oligonucleotide"
gttggacagaacttaccgactgg

SEQ ID NO: 69 - DNA, 20 bp, Artificial Sequence
  source: /note="Description of Artificial Sequence: Synthetic oligonucleotide"
gcagttgcctaagaactggt

SEQ ID NO: 70 - DNA, 20 bp, Artificial Sequence
  source: /note="Description of Artificial Sequence: Synthetic oligonucleotide"
ggggctccaccctcacgagt

SEQ ID NO: 71 - DNA, 23 bp, Artificial Sequence
  source: /note="Description of Artificial Sequence: Synthetic oligonucleotide"
gtttgcttcgctataaaacgagg

SEQ ID NO: 72 - DNA, 23 bp, Artificial Sequence
  source: /note="Description of Artificial Sequence: Synthetic oligonucleotide"
gtctgaggatggggccgcaatgg

SEQ ID NO: 73 - DNA, 23 bp, Artificial Sequence
  source: /note="Description of Artificial Sequence: Synthetic oligonucleotide"
ggatctgtcaaatcgcctgcagg

SEQ ID NO: 74 - DNA, 23 bp, Artificial Sequence
  source: /note="Description of Artificial Sequence: Synthetic oligonucleotide"
gccaggatggcattgggcagcgg

SEQ ID NO: 75 - DNA, 23 bp, Artificial Sequence
  source: /note="Description of Artificial Sequence: Synthetic oligonucleotide"
gctgaatctgcggtggcaggagg

SEQ ID NO: 76 - DNA, 23 bp, Artificial Sequence
  source: /note="Description of Artificial Sequence: Synthetic oligonucleotide"
gttcttttgttcttctagcctgg

SEQ ID NO: 77 - DNA, 23 bp, Artificial Sequence
  source: /note="Description of Artificial Sequence: Synthetic oligonucleotide"
ggaaaagcttgagcaagtcaagg

SEQ ID NO: 78 - DNA, 23 bp, Artificial Sequence
  source: /note="Description of Artificial Sequence: Synthetic oligonucleotide"
ggaagagttgcccctgcgccagg

SEQ ID NO: 79 - DNA, 23 bp, Artificial Sequence
  source: /note="Description of Artificial Sequence: Synthetic oligonucleotide"
gacaaatctccagtggataaagg

SEQ ID NO: 80 - DNA, 23 bp, Artificial Sequence
  source: /note="Description of Artificial Sequence: Synthetic oligonucleotide"
gtgtttctcaggtaaagctctgg

SEQ ID NO: 81 - DNA, 23 bp, Artificial Sequence
  source: /note="Description of Artificial Sequence: Synthetic oligonucleotide"
ggaaggaccatttgacgttaagg

SEQ ID NO: 82 - DNA, 23 bp, Artificial Sequence
  source: /note="Description of Artificial Sequence: Synthetic oligonucleotide"
gaactgctatttcagtttcctgg

SEQ ID NO: 83 - DNA, 23 bp, Artificial Sequence
  source: /note="Description of Artificial Sequence: Synthetic oligonucleotide"
gccagccactcagccagtgaagg

SEQ ID NO: 84 - DNA, 23 bp, Artificial Sequence
  source: /note="Description of Artificial Sequence: Synthetic oligonucleotide"
ggtatgcttttctgttaaagagg

SEQ ID NO: 85 - DNA, 23 bp, Artificial Sequence
  source: /note="Description of Artificial Sequence: Synthetic oligonucleotide"
gctcctggactgaccactattgg

SEQ ID NO: 86 - DNA, 23 bp, Artificial Sequence
  source: /note="Description of Artificial Sequence: Synthetic oligonucleotide"
ggaacagaggcgtccccagttgg

SEQ ID NO: 87 - DNA, 23 bp, Artificial Sequence
  source: /note="Description of Artificial Sequence: Synthetic oligonucleotide"
ggaggctagaacaatcattacgg

SEQ ID NO: 88 - DNA, 23 bp, Artificial Sequence
  source: /note="Description of Artificial Sequence: Synthetic oligonucleotide"
gacaagaacaccttcagaaccgg

SEQ ID NO: 89 - DNA, 23 bp, Artificial Sequence
  source: /note="Description of Artificial Sequence: Synthetic oligonucleotide"
gggtttctgtgattttcttttgg

SEQ ID NO: 90 - DNA, 23 bp, Artificial Sequence
  source: /note="Description of Artificial Sequence: Synthetic oligonucleotide"
gggccaaagacctccgccagtgg

SEQ ID NO: 91 - DNA, 23 bp, Artificial Sequence
  source: /note="Description of Artificial Sequence: Synthetic oligonucleotide"
gttggagaagcattcataaaagg

SEQ ID NO: 92 - DNA, 23 bp, Artificial Sequence
  source: /note="Description of Artificial Sequence: Synthetic oligonucleotide"
gtcgctcactcaccctgcaaagg

SEQ ID NO: 93 - DNA, 23 bp, Artificial Sequence
  source: /note="Description of Artificial Sequence: Synthetic oligonucleotide"
gaaaagagctgatgaaacaatgg

SEQ ID NO: 94 - DNA, 23 bp, Artificial Sequence
  source: /note="Description of Artificial Sequence: Synthetic oligonucleotide"
gtacacttttcaaaatgctttgg

SEQ ID NO: 95 - DNA, 23 bp, Artificial Sequence
  source: /note="Description of Artificial Sequence: Synthetic oligonucleotide"
ggagatgatcatcaagcagaagg

SEQ ID NO: 96 - DNA, 23 bp, Artificial Sequence
  source: /note="Description of Artificial Sequence: Synthetic oligonucleotide"
gctttgaaagagcaataaaatgg

SEQ ID NO: 97 - DNA, 23 bp, Artificial Sequence
  source: /note="Description of Artificial Sequence: Synthetic oligonucleotide"
gcacaaaagtcaaatcggaatgg

SEQ ID NO: 98 - DNA, 23 bp, Artificial Sequence
  source: /note="Description of Artificial Sequence: Synthetic oligonucleotide"
gatttcaatataagattcggagg

SEQ ID NO: 99 - DNA, 23 bp, Artificial Sequence
  source: /note="Description of Artificial Sequence: Synthetic oligonucleotide"
gcttaagcaatcccgaactctgg

SEQ ID NO: 100 - DNA, 20 bp, Artificial Sequence
  source: /note="Description of Artificial Sequence: Synthetic oligonucleotide"
gccttctttatcccctatcg

SEQ ID NO: 101-103 - skipped (3 entries)

SEQ ID NO: 104 - DNA, 25 bp, Artificial Sequence
  source: /note="Description of Artificial Sequence: Synthetic oligonucleotide"
  modified_base (21)..(22): a, c, t, g, unknown or other
gaggccaaacctcggcttacnngrr

SEQ ID NO: 105 - DNA, 25 bp, Artificial Sequence
  source: /note="Description of Artificial Sequence: Synthetic oligonucleotide"
  modified_base (21)..(22): a, c, t, g, unknown or other
gttcgaaaatttcaggtaagnngrr

SEQ ID NO: 106 - DNA, 26 bp, Artificial Sequence
  source: /note="Description of Artificial Sequence: Synthetic oligonucleotide"
  modified_base (21)..(22): a, c, t, g, unknown or other
ggcagaacaggagataacagnngrrt

SEQ ID NO: 107 - DNA, 26 bp, Artificial Sequence
  source: /note="Description of Artificial Sequence: Synthetic oligonucleotide"
ggcggccctcgcccttctctggggat

SEQ ID NO: 108 - DNA, 23 bp, Artificial Sequence
  source: /note="Description of Artificial Sequence: Synthetic oligonucleotide"
gtagtgatcgtggatacgagagg

SEQ ID NO: 109 - DNA, 23 bp, Artificial Sequence
  source: /note="Description of Artificial Sequence: Synthetic oligonucleotide"
gtacagccctcggtgtatattgg

SEQ ID NO: 110 - DNA, 23 bp, Artificial Sequence
  source: /note="Description of Artificial Sequence: Synthetic oligonucleotide"
gggaaggaattaagcccgaatgg

SEQ ID NO: 111 - DNA, 23 bp, Artificial Sequence
  source: /note="Description of Artificial Sequence: Synthetic oligonucleotide"
gggaacagctttcgtagttgagg

SEQ ID NO: 112 - DNA, 23 bp, Artificial Sequence
  source: /note="Description of Artificial Sequence: Synthetic oligonucleotide"
gataaagtccagtgtcgatcagg

SEQ ID NO: 113 - DNA, 23 bp, Artificial Sequence
  source: /note="Description of Artificial Sequence: Synthetic oligonucleotide"
gaaaaccagagcttcggtcaagg

SEQ ID NO: 114 - DNA, 34 bp, Artificial Sequence
  source: /note="Description of Artificial Sequence: Synthetic oligonucleotide"
ggagtcttctgggcaggcttaaaggctaacctgg

SEQ ID NO: 115 - DNA, 34 bp, Artificial Sequence
  source: /note="Description of Artificial Sequence: Synthetic oligonucleotide"
gtcgggtgagcatgtctttaatctacctcgatgg

SEQ ID NO: 116 - DNA, 26 bp, Artificial Sequence
  source: /note="Description of Artificial Sequence: Synthetic oligonucleotide"
ggtgtcaccagagtaacagtctgagt

SEQ ID NO: 117 - DNA, 25 bp, Artificial Sequence
  source: /note="Description of Artificial Sequence: Synthetic oligonucleotide"
gtgatcatcaagcagaaggtatgag

SEQ ID NO: 118 - DNA, 29 bp, Artificial Sequence
  source: /note="Description of Artificial Sequence: Synthetic oligonucleotide"
gaacttcgaaaatttcaggtaagccgagg

SEQ ID NO: 119 - DNA, 29 bp, Artificial Sequence
  source: /note="Description of Artificial Sequence: Synthetic oligonucleotide"
ggaaactcatcaaatatgcgtgttagtgt

SEQ ID NO: 120 - DNA, 29 bp, Artificial Sequence
  source: /note="Description of Artificial Sequence: Synthetic oligonucleotide"
gtcatttacactaacacgcatatttgatg

SEQ ID NO: 121 - DNA, 29 bp, Artificial Sequence
  source: /note="Description of Artificial Sequence: Synthetic oligonucleotide"
ggaatgaaactcatcaaatatgcgtgtta

SEQ ID NO: 122 - DNA, 29 bp, Artificial Sequence
  source: /note="Description of Artificial Sequence: Synthetic oligonucleotide"
gtcatcaatatctttgaaggactctgggt

SEQ ID NO: 123 - DNA, 29 bp, Artificial Sequence
  source: /note="Description of Artificial Sequence: Synthetic oligonucleotide"
gtgttttcataggaaaaataggcaagttg

SEQ ID NO: 124 - DNA, 29 bp, Artificial Sequence
  source: /note="Description of Artificial Sequence: Synthetic oligonucleotide"
gaattggaaaatgtgatgggaaacagata

SEQ ID NO: 125 - DNA, 29 bp, Artificial Sequence
  source: /note="Description of Artificial Sequence: Synthetic oligonucleotide"
gatgatcatcaagcagaaggtatgagaaa

SEQ ID NO: 126 - DNA, 29 bp, Artificial Sequence
  source: /note="Description of Artificial Sequence: Synthetic oligonucleotide"
gagatgatcatcaagcagaaggtatgaga

SEQ ID NO: 127 - DNA, 29 bp, Artificial Sequence
  source: /note="Description of Artificial Sequence: Synthetic oligonucleotide"
gcattttttctcataccttctgcttgatg

SEQ ID NO: 128 - DNA, 29 bp, Artificial Sequence
  source: /note="Description of Artificial Sequence: Synthetic oligonucleotide"
gtcctactcagactgttactctggtgaca

SEQ ID NO: 129 - DNA, 29 bp, Artificial Sequence
  source: /note="Description of Artificial Sequence: Synthetic oligonucleotide"
gacaggttgtgtcaccagagtaacagtct

SEQ ID NO: 130 - DNA, 29 bp, Artificial Sequence
  source: /note="Description of Artificial Sequence: Synthetic oligonucleotide"
gttatcattttttctcataccttctgctt

SEQ ID NO: 131 - DNA, 29 bp, Artificial Sequence
  source: /note="Description of Artificial Sequence: Synthetic oligonucleotide"
gttgcctaagaactggtgggaaatggtct

SEQ ID NO: 132 - DNA, 29 bp, Artificial Sequence
  source: /note="Description of Artificial Sequence: Synthetic oligonucleotide"
gaaacagttgcctaagaactggtgggaaa

SEQ ID NO: 133 - DNA, 29 bp, Artificial Sequence
  source: /note="Description of Artificial Sequence: Synthetic oligonucleotide"
gtttcccaccagttcttaggcaactgttt

SEQ ID NO: 134 - DNA, 29 bp, Artificial Sequence
  source: /note="Description of Artificial Sequence: Synthetic oligonucleotide"
gtggctttgatttccctagggtccagctt

SEQ ID NO: 135 - DNA, 29 bp, Artificial Sequence
  source: /note="Description of Artificial Sequence: Synthetic oligonucleotide"
gtagggaaatcaaagccaatgaaacgttc

SEQ ID NO: 136 - DNA, 29 bp, Artificial Sequence
  source: /note="Description of Artificial Sequence: Synthetic oligonucleotide"
ggaccctagggaaatcaaagccaatgaaa

SEQ ID NO: 137 - DNA, 29 bp, Artificial Sequence
  source: /note="Description of Artificial Sequence: Synthetic oligonucleotide"
gtgagggctccaccctcacgagtgggttt

SEQ ID NO: 138 - DNA, 29 bp, Artificial Sequence
  source: /note="Description of Artificial Sequence: Synthetic oligonucleotide"
gaaggattgagggctccaccctcacgagt

SEQ ID NO: 139 - DNA, 29 bp, Artificial Sequence
  source: /note="Description of Artificial Sequence: Synthetic oligonucleotide"
ggctccaccctcacgagtgggtttggttc

SEQ ID NO: 140 - DNA, 29 bp, Artificial Sequence
  source: /note="Description of Artificial Sequence: Synthetic oligonucleotide"
gtatcccctatcgaggaaaccacgagttt

SEQ ID NO: 141 - DNA, 29 bp, Artificial Sequence
  source: /note="Description of Artificial Sequence: Synthetic oligonucleotide"
ggataaagaaggcctatttcatagagttg

SEQ ID NO: 142 - DNA, 29 bp, Artificial Sequence
  source: /note="Description of Artificial Sequence: Synthetic oligonucleotide"
gaggccttctttatcccctatcgaggaaa

SEQ ID NO: 143 - DNA, 27 bp, Artificial Sequence
  source: /note="Description of Artificial Sequence: Synthetic oligonucleotide"
gtgagggctccaccctcacgagtgggt

SEQ ID NO: 144 - DNA, 27 bp, Artificial Sequence
  source: /note="Description of Artificial Sequence: Synthetic oligonucleotide"
ggataaagaaggcctatttcatagagt

SEQ ID NO: 145 - DNA, 4932 bp, Artificial Sequence
  source: /note="Description of Artificial Sequence: Synthetic polynucleotide"
gccaccatggacaagaagtactccattgggctcgatatcggcacaaacagcgtcggctgggccgtcattacggacgagtacaaggtgccgagcaaaaaattcaaagttctgggcaataccgatcgccacagcataaagaagaacctcattggcgccctcctgttcgactccggggagacggccgaagccacgcggctcaaaagaacagcacggcgcagatatacccgcagaaagaatcggatctgctacctgcaggagatctttagtaatgagatggctaaggtggatgactctttcttccataggctggaggagtcctttttggtggaggaggataaaaagcacgagcgccacccaatctttggcaatatcgtggacgaggtggcgtaccatgaaaagtacccaaccatatatcatctgaggaagaagcttgtagacagtactgataaggctgacttgcggttgatctatctcgcgctggcgcatatgatcaaatttcggggacacttcctcatcgagggggacctgaacccagacaacagcgatgtcgacaaactctttatccaactggttcagacttacaatcagcttttcgaagagaacccgatcaacgcatccggagttgacgccaaagcaatcctgagcgctaggctgtccaaatcccggcggctcgaaaacctcatcgcacagctccctggggagaagaagaacggcctgtttggtaatcttatcgccctgtcactcgggctgacccccaactttaaatctaacttcgacctggccgaagatgccaagcttcaactgagcaaagacacctacgatgatgatctcgacaatctgctggcccagatcggcgaccagtacgcagacctttttttggcggcaaagaacctgtcagacgccattctgctgagtgatattctgcgagtgaacacggagatcaccaaagctccgctgagcgctagtatgatcaagcgctatgatgagcaccaccaagacttgactttgctgaaggcccttgtcagacagcaactgcctgagaagtacaaggaaattttcttcgatcagtctaaaaatggctacgccggatacattgacggcggagcaagccaggaggaattttacaaatttattaagcccatcttggaaaaaatggacggcaccgaggagctgctggtaaagcttaacagagaagatctgttgcgcaaacagcgcactttcgacaatggaagcatcccccaccagattcacctgggcgaactgcacgctatcctcaggcggcaagaggatttctacccctttttgaaagataacagggaaaagattgagaaaatcctcacatttcggataccctactatgtaggccccctcgcccggggaaattccagattcgcgtggatgactcgcaaatcagaagagaccatcactccctggaacttcgaggaagtcgtggataagggggcctctgcccagtccttcatcgaaaggatgactaactttgataaaaatctgcctaacgaaaaggtgcttcctaaacactctctgctgtacgagtacttcacagtttataacgagctcaccaaggtcaaatacgtcacagaagggatgagaaagccagcattcctgtctggagagcagaagaaagctatcgtggacctcctcttcaagacgaaccggaaagttaccgtgaaacagctcaaagaagactatttcaaaaagattgaatgtttcgactctgttgaaatcagcggagtggaggatcgcttcaacgcatccctgggaacgtatcacgatctcctgaaaatcattaaagacaaggacttcctggacaatgaggagaacgaggacattcttgaggacattgtcctcacccttacgttgtttgaagatagggagatgattgaagaacgcttgaaaacttacgctcatctcttcgacgacaaagtcatgaaacagctcaagaggcgccgatatacaggatgggggcggctgtcaagaaaactgatcaatgggatccgagacaagcagagtggaaagacaatcctggattttcttaagtccgatggatttgccaaccggaacttcatgcagttgatccatgatgactctctcacctttaaggaggacatccagaaagcacaagtttctggccagggggacagtcttcacgagcacatcgctaatcttgcaggtagcccagctatcaaaaagggaatactgcagaccgttaaggtcgtggatgaactcgtcaaagtaatgggaaggcataagcccgagaatatcgttatcgagatggcccgagagaaccaaactacccagaagggacagaagaacagtagggaaaggatgaagaggattgaagagggtataaaagaactggggtcccaaatccttaaggaacacccagttgaaaacacccagcttcagaatgagaagctctacctgtactacctgcagaacggcagggacatgtacgtggatcaggaactggacatcaatcggctctccgactacgacgtggatcatatcgtgccccagtcttttctcaaagatgattctattgataataaagtgttgacaagatccgataaaaatagagggaagagtgataacgtcccctcagaagaagttgtcaagaaaatgaaaaattattggcggcagctgctgaacgccaaactgatcacacaacggaagttcgataatctgactaaggctgaacgaggtggcctgtctgagttggataaagccggcttcatcaaaaggcagcttgttgagacacgccagatcaccaagcacgtggcccaaattctcgattcacgcatgaacaccaagtacgatgaaaatgacaaactgattcgagaggtgaaagttattactctgaagtctaagctggtctcagatttcagaaaggactttcagttttataaggtgagagagatcaacaattaccaccatgcgcatgatgcctacctgaatgcagtggtaggcactgcacttatcaaaaaatatcccaagcttgaatctgaatttgtttacggagactataaagtgtacgatgttaggaaaatgatcgcaaagtctgagcaggaaataggcaaggccaccgctaagtacttcttttacagcaatattatgaattttttcaagaccgagattacactggccaatggagagattcggaagcgaccacttatcgaaacaaacggagaaacaggagaaatcgtgtgggacaagggtagggatttcgcgacagtccggaaggtcctgtccatgccgcaggtgaacatcgttaaaaagaccgaagtacagaccggaggcttctccaaggaaagtatcctcccgaaaaggaacagcgacaagctgatcgcacgcaaaaaagattgggaccccaagaaatacggcggattcgattctcctacagtcgcttacagtgtactggttgtggccaaagtggagaaagggaagtctaaaaaactcaaaagcgtcaaggaactgctgggcatcacaatcatggagcgatcaagcttcgaaaaaaaccccatcgactttctcgaggcgaaaggatataaagaggtcaaaaaagacctcatcattaagcttcccaagtactctctctttgagcttgaaaacggccggaaacgaatgctcgctagtgcgggcgagctgcagaaaggtaacgagctggcactgccctctaaatacgttaatttcttgtatctggccagccactatgaaaagctcaaagggtctcccgaagataatgagcagaagcagctgttcgtggaacaacacaaacactaccttgatgagatcatcgagcaaataagcgaattctccaaaagagtgatcctcgccgacgctaacctcgataaggtgctttctgcttacaataagcacagggataagcccatcagggagcaggcagaaaacattatccacttgtttactctgaccaacttgggcgcgcctgcagccttcaagtacttcgacaccaccatagacagaaagcggtacacctctacaaaggaggtcctggacgccacactgattcatcagtcaattacggggctctatgaaacaagaatcgacctctctcagctcggtggagacagcagggctgaccccaagaagaagaggaaggtggctagcgagggcagaggaagtcttctaacatgcggtgacgtggaggagaatcccggccctggtaccgtgagcaagggcgaggagctgttcaccggggtggtgcccatcctggtcgagctggacggcgacgtaaacggccacaagttcagcgtgtccggcgagggcgagggcgatgccacctacggcaagctgaccctgaagttcatctgcaccaccggcaagctgcccgtgccctggcccaccctcgtgaccaccctgacctacggcgtgcagtgcttcagccgctaccccgaccacatgaagcagcacgacttcttcaagtccgccatgcccgaaggctacgtccaggagcgcaccatcttcttcaaggacgacggcaactacaagacccgcgccgaggtgaagttcgagggcgacaccctggtgaaccgcatcgagctgaagggcatcgacttcaaggaggacggcaacatcctggggcacaagctggagtacaactacaacagccacaacgtctatatcatggccgacaagcagaagaacggcatcaaggtgaacttcaagatccgccacaacatcgaggacggcagcgtgcagctcgccgaccactaccagcagaacacccccatcggcgacggccccgtgctgctgcccgacaaccactacctgagcacccagtccgccctgagcaaagaccccaacgagaagcgcgatcacatggtcctgctggagttcgtgaccgccgccgggatcactctcggcatggacgagctgtacaagaccggttag

SEQ ID NO: 146-149 - skipped (4 entries)

SEQ ID NO: 150 - DNA, 23 bp, Artificial Sequence
  source: /note="Description of Artificial Sequence: Synthetic oligonucleotide"
tcctactcagactgttactctgg

SEQ ID NO: 151 - DNA, 23 bp, Artificial Sequence
  source: /note="Description of Artificial Sequence: Synthetic oligonucleotide"
tcctactcacactgttactcagg

SEQ ID NO: 152 - DNA, 23 bp, Artificial Sequence
  source: /note="Description of Artificial Sequence: Synthetic oligonucleotide"
acctgctcacactgttactccag

SEQ ID NO: 153 - DNA, 23 bp, Artificial Sequence
  source: /note="Description of Artificial Sequence: Synthetic oligonucleotide"
gcattctcaaactgttactcagg

SEQ ID NO: 154 - DNA, 23 bp, Artificial Sequence
  source: /note="Description of Artificial Sequence: Synthetic oligonucleotide"
ggattctcacactgttactcggg

SEQ ID NO: 155 - DNA, 23 bp, Artificial Sequence
  source: /note="Description of Artificial Sequence: Synthetic oligonucleotide"
acatacttatactgttactctag

SEQ ID NO: 156 - DNA, 23 bp, Artificial Sequence
  source: /note="Description of Artificial Sequence: Synthetic oligonucleotide"
tattcctaagactgttactcaag

SEQ ID NO: 157 - DNA, 23 bp, Artificial Sequence
  source: /note="Description of Artificial Sequence: Synthetic oligonucleotide"
aaggactaagactgttactcggg

SEQ ID NO: 158 - DNA, 23 bp, Artificial Sequence
  source: /note="Description of Artificial Sequence: Synthetic oligonucleotide"
gagctctcatactgttactctag

SEQ ID NO: 159 - DNA, 23 bp, Artificial Sequence
  source: /note="Description of Artificial Sequence: Synthetic oligonucleotide"
gcaaaatgagactgttactccag

SEQ ID NO: 160 - DNA, 23 bp, Artificial Sequence
  source: /note="Description of Artificial Sequence: Synthetic oligonucleotide"
cctcattcagactgttactcaag

SEQ ID NO: 161 - DNA, 23 bp, Artificial Sequence
  source: /note="Description of Artificial Sequence: Synthetic oligonucleotide"
cattggctttgatttccctaggg

SEQ ID NO: 162 - DNA, 23 bp, Artificial Sequence
  source: /note="Description of Artificial Sequence: Synthetic oligonucleotide"
aattggcattgatttccctagag

SEQ ID NO: 163 - DNA, 23 bp, Artificial Sequence
  source: /note="Description of Artificial Sequence: Synthetic oligonucleotide"
cattggctttaatttccctatag

SEQ ID NO: 164 - DNA, 23 bp, Artificial Sequence
  source: /note="Description of Artificial Sequence: Synthetic oligonucleotide"
gataggctgtgatttccctagag

SEQ ID NO: 165 - DNA, 23 bp, Artificial Sequence
  source: /note="Description of Artificial Sequence: Synthetic oligonucleotide"
gaatagccttgatttccctaaag

SEQ ID NO: 166 - DNA, 23 bp, Artificial Sequence
  source: /note="Description of Artificial Sequence: Synthetic oligonucleotide"
aatttgctttgatttccctgagg

SEQ ID NO: 167 - DNA, 23 bp, Artificial Sequence
  source: /note="Description of Artificial Sequence: Synthetic oligonucleotide"
gatgtgctttgatttcccttggg

SEQ ID NO: 168 - DNA, 23 bp, Artificial Sequence
  source: /note="Description of Artificial Sequence: Synthetic oligonucleotide"
aattggttttaatttccctaaag

SEQ ID NO: 169 - DNA, 23 bp, Artificial Sequence
  source: /note="Description of Artificial Sequence: Synthetic oligonucleotide"
aattgggtttgatttccctttgg

SEQ ID NO: 170 - DNA, 23 bp, Artificial Sequence
  source: /note="Description of Artificial Sequence: Synthetic oligonucleotide"
gatgggtttttatttccctagag

SEQ ID NO: 171 - DNA, 23 bp, Artificial Sequence
  source: /note="Description of Artificial Sequence: Synthetic oligonucleotide"
gaatggttttgatttccctggag

SEQ ID NO: 172 - DNA, 23 bp, Artificial Sequence
  source: /note="Description of Artificial Sequence: Synthetic oligonucleotide"
acagttgcctaagaactggtggg

SEQ ID NO: 173 - DNA, 23 bp, Artificial Sequence
  source: /note="Description of Artificial Sequence: Synthetic oligonucleotide"
ccagttgtctaagaactggggag

SEQ ID NO: 174 - DNA, 23 bp, Artificial Sequence
  source: /note="Description of Artificial Sequence: Synthetic oligonucleotide"
gcagttgcctgtgaactggtagg

SEQ ID NO: 175 - DNA, 23 bp, Artificial Sequence
  source: /note="Description of Artificial Sequence: Synthetic oligonucleotide"
gcagatgcagaagaactggtgag

SEQ ID NO: 176 - DNA, 23 bp, Artificial Sequence
  source: /note="Description of Artificial Sequence: Synthetic oligonucleotide"
gcagttccagaagaactggtgag

SEQ ID NO: 177 - DNA, 23 bp, Artificial Sequence
  source: /note="Description of Artificial Sequence: Synthetic oligonucleotide"
caacttgcctatgaactggtagg

SEQ ID NO: 178 - DNA, 23 bp, Artificial Sequence
  source: /note="Description of Artificial Sequence: Synthetic oligonucleotide"
acacctgcctaagaactggaggg

SEQ ID NO: 179 - DNA, 23 bp, Artificial Sequence
  source: /note="Description of Artificial Sequence: Synthetic oligonucleotide"
tcaggtggctaagaactgggtgg

SEQ ID NO: 180 - DNA, 23 bp, Artificial Sequence
  source: /note="Description of Artificial Sequence: Synthetic oligonucleotide"
gaagttggccaagaactggagag

SEQ ID NO: 181 - DNA, 23 bp, Artificial Sequence
  source: /note="Description of Artificial Sequence: Synthetic oligonucleotide"
gctgctgcccaagaactggcagg

SEQ ID NO: 182 - DNA, 23 bp, Artificial Sequence
  source: /note="Description of Artificial Sequence: Synthetic oligonucleotide"
tcagctggctaagaacgggtaag

SEQ ID NO: 183 - DNA, 23 bp, Artificial Sequence
  source: /note="Description of Artificial Sequence: Synthetic oligonucleotide"
agggctccaccctcacgagtggg

SEQ ID NO: 184 - DNA, 23 bp, Artificial Sequence
  source: /note="Description of Artificial Sequence: Synthetic oligonucleotide"
gcagctcagccctcacgagtcag

SEQ ID NO: 185 - DNA, 23 bp, Artificial Sequence
  source: /note="Description of Artificial Sequence: Synthetic oligonucleotide"
ggggcttcagcatcacgagtgag

SEQ ID NO: 186 - DNA, 23 bp, Artificial Sequence
  source: /note="Description of Artificial Sequence: Synthetic oligonucleotide"
ggggctctcccctcactagtgag

SEQ ID NO: 187 - DNA, 23 bp, Artificial Sequence
  source: /note="Description of Artificial Sequence: Synthetic oligonucleotide"
ggggatccaccttcaccagtcag

SEQ ID NO: 188 - DNA, 23 bp, Artificial Sequence
  source: /note="Description of Artificial Sequence: Synthetic oligonucleotide"
agggctggaccctcacaagtaag

SEQ ID NO: 189 - DNA, 23 bp, Artificial Sequence
  source: /note="Description of Artificial Sequence: Synthetic oligonucleotide"
tggtctcctcccccacgagtggg

SEQ ID NO: 190 - DNA, 23 bp, Artificial Sequence
  source: /note="Description of Artificial Sequence: Synthetic oligonucleotide"
agggctcccaccccacgagtgag

SEQ ID NO: 191 - DNA, 23 bp, Artificial Sequence
  source: /note="Description of Artificial Sequence: Synthetic oligonucleotide"
gaggctccatactcaccagtgag

SEQ ID NO: 192 - DNA, 23 bp, Artificial Sequence
  source: /note="Description of Artificial Sequence: Synthetic oligonucleotide"
ggagctgccccttcacgagtggg

SEQ ID NO: 193 - DNA, 23 bp, Artificial Sequence
  source: /note="Description of Artificial Sequence: Synthetic oligonucleotide"
atgactccaccctcaagagtaag

SEQ ID NO: 194 - DNA, 23 bp, Artificial Sequence
  source: /note="Description of Artificial Sequence: Synthetic oligonucleotide"
gccttctttatcccctatcgagg

SEQ ID NO: 195 - DNA, 23 bp, Artificial Sequence
  source: /note="Description of Artificial Sequence: Synthetic oligonucleotide"
gtctgctgtgtcccctatcgggg

SEQ ID NO: 196 - DNA, 23 bp, Artificial Sequence
  source: /note="Description of Artificial Sequence: Synthetic oligonucleotide"
cccttctctatcccctgtcgtgg

SEQ ID NO: 197 - DNA, 23 bp, Artificial Sequence
  source: /note="Description of Artificial Sequence: Synthetic oligonucleotide"
gccttctttatcccctctcttgg

SEQ ID NO: 198 - DNA, 23 bp, Artificial Sequence
  source: /note="Description of Artificial Sequence: Synthetic oligonucleotide"
gcgctctttttcccctatcttag

SEQ ID NO: 199 - DNA, 23 bp, Artificial Sequence
  source: /note="Description of Artificial Sequence: Synthetic oligonucleotide"
gccctctgtctcccctgtcgcag

SEQ ID NO: 200 - DNA, 23 bp, Artificial Sequence
  source: /note="Description of Artificial Sequence: Synthetic oligonucleotide"
tccatctttgtcccctattgagg

SEQ ID NO: 201 - DNA, 23 bp, Artificial Sequence
  source: /note="Description of Artificial Sequence: Synthetic oligonucleotide"
accttctctctcccctatagagg

SEQ ID NO: 202 - DNA, 23 bp, Artificial Sequence
  source: /note="Description of Artificial Sequence: Synthetic oligonucleotide"
gttttctttttcccctatgggag

SEQ ID NO: 203 - DNA, 23 bp, Artificial Sequence
  source: /note="Description of Artificial Sequence: Synthetic oligonucleotide"
tgcttcttaatcccctatcaaag

SEQ ID NO: 204 - DNA, 23 bp, Artificial Sequence
  source: /note="Description of Artificial Sequence: Synthetic oligonucleotide"
accttcttactcccctatccggg

SEQ ID NO: 205 - DNA, 22 bp, Artificial Sequence
  source: /note="Description of Artificial Sequence: Synthetic primer"
gagaggttatgtggctttacca

SEQ ID NO: 206 - DNA, 20 bp, Artificial Sequence
  source: /note="Description of Artificial Sequence: Synthetic primer"
aaaaatgcttcccactttgc

SEQ ID NO: 207 - DNA, 20 bp, Artificial Sequence
  source: /note="Description of Artificial Sequence: Synthetic primer"
ctcattctcatgcctggaca

SEQ ID NO: 208 - DNA, 25 bp, Artificial Sequence
  source: /note="Description of Artificial Sequence: Synthetic primer"
gagtttggctcaaattgttactctt

SEQ ID NO: 209 - DNA, 25 bp, Artificial Sequence
  source: /note="Description of Artificial Sequence: Synthetic primer"
gggaaatggtctaggagagtaaagt

SEQ ID NO: 210 - DNA, 25 bp, Artificial Sequence
  source: /note="Description of Artificial Sequence: Synthetic primer"
gtttggctcaaattgttactcttca

SEQ ID NO: 211 - DNA, 25 bp, Artificial Sequence
  source: /note="Description of Artificial Sequence: Synthetic primer"
gtgagagtaatgtgtttgctgagag

SEQ ID NO: 212 - DNA, 20 bp, Artificial Sequence
  source: /note="Description of Artificial Sequence: Synthetic primer"
cgggcttggacagaacttac

SEQ ID NO: 213 - DNA, 20 bp, Artificial Sequence
  source: /note="Description of Artificial Sequence: Synthetic primer"
ctgcgtagtgccaaaacaaa

SEQ ID NO: 214 - DNA, 24 bp, Artificial Sequence
  source: /note="Description of Artificial Sequence: Synthetic primer"
taatttcattgaagagtggctgaa

SEQ ID NO: 215 - DNA, 24 bp, Artificial Sequence
  source: /note="Description of Artificial Sequence: Synthetic primer"
aagccctgtgtggtagtagtcagt

SEQ ID NO: 216 - DNA, 24 bp, Artificial Sequence
  source: /note="Description of Artificial Sequence: Synthetic primer"
tgagtcatgttggataaccagtct

SEQ ID NO: 217 - DNA, 24 bp, Artificial Sequence
  source: /note="Description of Artificial Sequence: Synthetic primer"
gaaggtcaggaacatacaattcaa

SEQ ID NO: 218 - DNA, 24 bp, Artificial Sequence
  source: /note="Description of Artificial Sequence: Synthetic primer"
gatatgggcatgtcagtttcatag

SEQ ID NO: 219 - DNA, 24 bp, Artificial Sequence
  source: /note="Description of Artificial Sequence: Synthetic primer"
tgctgttgattaatggttgatagg

SEQ ID NO: 220 - DNA, 23 bp, Artificial Sequence
  source: /note="Description of Artificial Sequence: Synthetic primer"
ttttaaattgccatgtttgtgtc

SEQ ID NO: 221 - DNA, 24 bp, Artificial Sequence
  source: /note="Description of Artificial Sequence: Synthetic primer"
atgaataacctaatgggcagaaaa

SEQ ID NO: 222 - DNA, 24 bp, Artificial Sequence
  source: /note="Description of Artificial Sequence: Synthetic primer"
tcaagtcgcttcattttgatagac

SEQ ID NO: 223 - DNA, 24 bp, Artificial Sequence
  source: /note="Description of Artificial Sequence: Synthetic primer"
cacaacaaaacatatagccaaagc

SEQ ID NO: 224 - DNA, 25 bp, Artificial Sequence
  source: /note="Description of Artificial Sequence: Synthetic primer"
tgctgctaaaataacacaaatcagt

SEQ ID NO: 225 - DNA, 23 bp, Artificial Sequence
  source: /note="Description of Artificial Sequence: Synthetic primer"
ctgtgcctattgtggttatcctg

SEQ ID NO: 226 - DNA, 24 bp, Artificial Sequence
  source: /note="Description of Artificial Sequence: Synthetic primer"
attgatctgcaatacatgtggagt

SEQ ID NO: 227 - DNA, 24 bp, Artificial Sequence
  source: /note="Description of Artificial Sequence: Synthetic primer"
tttgcctctgctattacagtatgg

SEQ ID NO: 228 - DNA, 24 bp, Artificial Sequence
  source: /note="Description of Artificial Sequence: Synthetic primer"
tgtagggtggttggctaaaataat

SEQ ID NO: 229 - DNA, 24 bp, Artificial Sequence
  source: /note="Description of Artificial Sequence: Synthetic primer"
tttttgcacagtcaataacacaaa

SEQ ID NO: 230 - DNA, 24 bp, Artificial Sequence
  source: /note="Description of Artificial Sequence: Synthetic primer"
ggctggtctcacaattgtacttta

SEQ ID NO: 231 - DNA, 24 bp, Artificial Sequence
  source: /note="Description of Artificial Sequence: Synthetic primer"
cattatggactgaaaatctcagca

SEQ ID NO: 232 - DNA, 24 bp, Artificial Sequence
  source: /note="Description of Artificial Sequence: Synthetic primer"
atcatcctagccataacacaatga

SEQ ID NO: 233 - DNA, 24 bp, Artificial Sequence
  source: /note="Description of Artificial Sequence: Synthetic primer"
ttcagctttaacgtgattttctgt

SEQ ID NO: 234 - DNA, 24 bp, Artificial Sequence
  source: /note="Description of Artificial Sequence: Synthetic primer"
ggattcagaagctgtttacgaagt

SEQ ID NO: 235 - DNA, 24 bp, Artificial Sequence
  source: /note="Description of Artificial Sequence: Synthetic primer"
tttagctggattggaaaaacaaat

SEQ ID NO: 236 - DNA, 24 bp, Artificial Sequence
  source: /note="Description of Artificial Sequence: Synthetic primer"
aactcaccccattgttggtatatt

SEQ ID NO: 237 - DNA, 24 bp, Artificial Sequence
  source: /note="Description of Artificial Sequence: Synthetic primer"
ccttgtccaaataccgaaatacat

SEQ ID NO: 238 - DNA, 24 bp, Artificial Sequence
  source: /note="Description of Artificial Sequence: Synthetic primer"
cacataattcatgaacttggcttc

SEQ ID NO: 239 - DNA, 24 bp, Artificial Sequence
  source: /note="Description of Artificial Sequence: Synthetic primer"
tagtagctggggaggaagatacag

SEQ ID NO: 240 - DNA, 24 bp, Artificial Sequence
  source: /note="Description of Artificial Sequence: Synthetic primer"
tttttgttttaattgcgactgtgt

SEQ ID NO: 241 - DNA, 24 bp, Artificial Sequence
  source: /note="Description of Artificial Sequence: Synthetic primer"
agaaaaggggttttcttttgactt

SEQ ID NO: 242 - DNA, 24 bp, Artificial Sequence
  source: /note="Description of Artificial Sequence: Synthetic primer"
cattgtgactggatgagaagaaac

SEQ ID NO: 243 - DNA, 24 bp, Artificial Sequence
  source: /note="Description of Artificial Sequence: Synthetic primer"
aacggctgttattaaagtcctcag

SEQ ID NO: 244 - DNA, 24 bp, Artificial Sequence
  source: /note="Description of Artificial Sequence: Synthetic primer"
caagtcagaagtcacttgctttgt

SEQ ID NO: 245 - DNA, 24 bp, Artificial Sequence
  source: /note="Description of Artificial Sequence: Synthetic primer"
ttttatgtgcaggaatcagtctgt

SEQ ID NO: 246 - DNA, 18 bp, Artificial Sequence
  source: /note="Description of Artificial Sequence: Synthetic primer"
tggcggcgttttcattat

SEQ ID NO: 247 - DNA, 26 bp, Artificial Sequence
  source: /note="Description of Artificial Sequence: Synthetic primer"
ttcgatccgtaatgattgttctagcc

SEQ ID NO: 248 - DNA, 20 bp, Artificial Sequence
  source: /note="Description of Artificial Sequence: Synthetic primer"
ggtcttccagagtgctgagg

SEQ ID NO: 249 - DNA, 24 bp, Artificial Sequence
  source: /note="Description of Artificial Sequence: Synthetic primer"
tgtgtgcttctgtacacatcatct

SEQ ID NO: 250 - DNA, 24 bp, Artificial Sequence
  source: /note="Description of Artificial Sequence: Synthetic primer"
agatttcaaccctcaaaaactgag

SEQ ID NO: 251 - DNA, 24 bp, Artificial Sequence
  source: /note="Description of Artificial Sequence: Synthetic primer"
taaactctttcttttccgcaattc

SEQ ID NO: 252 - DNA, 24 bp, Artificial Sequence
  source: /note="Description of Artificial Sequence: Synthetic primer"
caaggtgacctgctacctaaaaat

SEQ ID NO: 253 - DNA, 24 bp, Artificial Sequence
  source: /note="Description of Artificial Sequence: Synthetic primer"
tatgaccaaggctatgtgttcact

SEQ ID NO: 254 - DNA, 24 bp, Artificial Sequence
  source: /note="Description of Artificial Sequence: Synthetic primer"
acagcctctctccagtaacattct

SEQ ID NO: 255 - DNA, 24 bp, Artificial Sequence
  source: /note="Description of Artificial Sequence: Synthetic primer"
tattcttgcagtggtttcacattt

SEQ ID NO: 256 - DNA, 24 bp, Artificial Sequence
  source: /note="Description of Artificial Sequence: Synthetic primer"
atattttaagccaagacccaacaa

SEQ ID NO: 257 - DNA, 24 bp, Artificial Sequence
  source: /note="Description of Artificial Sequence: Synthetic primer"
ctttcaactgtctgtctgattgct

SEQ ID NO: 258 - DNA, 24 bp, Artificial Sequence
  source: /note="Description of Artificial Sequence: Synthetic primer"
aacagcctctcttcattgttctct

SEQ ID NO: 259 - DNA, 24 bp, Artificial Sequence
  source: /note="Description of Artificial Sequence: Synthetic primer"
ctctggaacttgtctctgtcttga

SEQ ID NO: 260 - DNA, 24 bp, Artificial Sequence
  source: /note="Description of Artificial Sequence: Synthetic primer"
ctttcctgcgttctcatgttacta

SEQ ID NO: 261 - DNA, 24 bp, Artificial Sequence
  source: /note="Description of Artificial Sequence: Synthetic primer"
ccttatatccgtatcgctcactct

SEQ ID NO: 262 - DNA, 24 bp, Artificial Sequence
  source: /note="Description of Artificial Sequence: Synthetic primer"
catatctgtctaacttccgcacac

SEQ ID NO: 263 - DNA, 24 bp, Artificial Sequence
  source: /note="Description of Artificial Sequence: Synthetic primer"
acaggtgttatgttgtctgcatct

SEQ ID NO: 264 - DNA, 24 bp, Artificial Sequence
  source: /note="Description of Artificial Sequence: Synthetic primer"
actccattcccagattagttatgc

SEQ ID NO: 265 - DNA, 24 bp, Artificial Sequence
  source: /note="Description of Artificial Sequence: Synthetic primer"
ctgttttctttgtgagagtggaga

SEQ ID NO: 266 - DNA, 24 bp, Artificial Sequence
  source: /note="Description of Artificial Sequence: Synthetic primer"
tgtaaggtggtcaaacttgctcta

SEQ ID NO: 267 - DNA, 25 bp, Artificial Sequence
  source: /note="Description of Artificial Sequence: Synthetic primer"
tttttcctagtacccacagattttt

SEQ ID NO: 268 - DNA, 24 bp, Artificial Sequence
  source: /note="Description of Artificial Sequence: Synthetic primer"
tccctgattctctcatttgtgtta

SEQ ID NO: 269 - DNA, 24 bp, Artificial Sequence
  source: /note="Description of Artificial Sequence: Synthetic primer"
ttgggaacatcagagaaagtatga

SEQ ID NO: 270 - DNA, 24 bp, Artificial Sequence
  source: /note="Description of Artificial Sequence: Synthetic primer"
acaaattacagtctcctgggaaag

SEQ ID NO: 271 - DNA, 24 bp, Artificial Sequence
  source: /note="Description of Artificial Sequence: Synthetic primer"
agtagcttaccttggcagagaaaa

SEQ ID NO: 272 - DNA, 24 bp, Artificial Sequence
  source: /note="Description of Artificial Sequence: Synthetic primer"
tgacatactgttaccctttgcagt

SEQ ID NO: 273 - DNA, 23 bp, Artificial Sequence
  source: /note="Description of Artificial Sequence: Synthetic primer"
gaaaggctcagtgaatgtttgtt

SEQ ID NO: 274 - DNA, 24 bp, Artificial Sequence
  source: /note="Description of Artificial Sequence: Synthetic primer"
cactgcatcatctcattaaatcaa

SEQ ID NO: 275 - DNA, 24 bp, Artificial Sequence
  source: /note="Description of Artificial Sequence: Synthetic primer"
cccatatattcatgattacccaca

SEQ ID NO: 276 - DNA, 24 bp, Artificial Sequence
  source: /note="Description of Artificial Sequence: Synthetic primer"
tatcagaacgagcactaaaagcac

SEQ ID NO: 277 - DNA, 20 bp, Artificial Sequence
  source: /note="Description of Artificial Sequence: Synthetic primer"
ttgggaggctgaggtacaag

SEQ ID NO: 278 - DNA, 24 bp, Artificial Sequence
  source: /note="Description of Artificial Sequence: Synthetic primer"
gaatgaaaaacaaacagaaggtga

SEQ ID NO: 279 - DNA, 24 bp, Artificial Sequence
  source: /note="Description of Artificial Sequence: Synthetic primer"
ctcctcatctgtacccttcaatct

SEQ ID NO: 280 - DNA, 24 bp, Artificial Sequence
  source: /note="Description of Artificial Sequence: Synthetic primer"
agagtggcatctagtgtcagtgag

SEQ ID NO: 281 - DNA, 24 bp, Artificial Sequence
  source: /note="Description of Artificial Sequence: Synthetic primer"
taccaaaagcttctcctgtttacc

SEQ ID NO: 282 - DNA, 24 bp, Artificial Sequence
  source: /note="Description of Artificial Sequence: Synthetic primer"
gtaagttggatggcctattctttg

SEQ ID NO: 283 - DNA, 24 bp, Artificial Sequence
  source: /note="Description of Artificial Sequence: Synthetic primer"
gaaggaaatgcaaggatacaagat

SEQ ID NO: 284 - DNA, 24 bp, Artificial Sequence
  source: /note="Description of Artificial Sequence: Synthetic primer"
tgattgaaagaatcattccagaaa

SEQ ID NO: 285 - DNA, 24 bp, Artificial Sequence
  source: /note="Description of Artificial Sequence: Synthetic primer"
tcagaaggaaaattgaaattggtt

SEQ ID NO: 286 - DNA, 24 bp, Artificial Sequence
  source: /note="Description of Artificial Sequence: Synthetic primer"
cagatgtgttcttcatcattcctc

SEQ ID NO: 287 - DNA, 24 bp, Artificial Sequence
  source: /note="Description of Artificial Sequence: Synthetic primer"
ttctctttagggaaagctctcaaa

SEQ ID NO: 288 - DNA, 24 bp, Artificial Sequence
  source: /note="Description of Artificial Sequence: Synthetic primer"
gggtatagatcatatggagggaag

SEQ ID NO: 289 - DNA, 20 bp, Artificial Sequence
  source: /note="Description of Artificial Sequence: Synthetic primer"
agatgatctgcccacctcag

SEQ ID NO: 290 - DNA, 24 bp, Artificial Sequence
  source: /note="Description of Artificial Sequence: Synthetic primer"
ctttcttcctcatttagtggcaat

SEQ ID NO: 291 - DNA, 24 bp, Artificial Sequence
  source: /note="Description of Artificial Sequence: Synthetic primer"
atgaattgcagattgatggtactg

SEQ ID NO: 292 - DNA, 24 bp, Artificial Sequence
  source: /note="Description of Artificial Sequence: Synthetic primer"
tctcaccaagaaccaaattgtcta

SEQ ID NO: 293 - DNA, 24 bp, Artificial Sequence
  source: /note="Description of Artificial Sequence: Synthetic primer"
gtaggataccttggcaacagtctt

SEQ ID NO: 294 - DNA, 24 bp, Artificial Sequence
  source: /note="Description of Artificial Sequence: Synthetic primer"
ttaacgaattgtgagatttgctgt

SEQ ID NO: 295 - DNA, 24 bp, Artificial Sequence
  source: /note="Description of Artificial Sequence: Synthetic primer"
tcagaaagtcaagtagcacacaca

SEQ ID NO: 296 - DNA, 23 bp, Artificial Sequence
  source: /note="Description of Artificial Sequence: Synthetic primer"
agaagcacacactcaggtaaagc

SEQ ID NO: 297 - DNA, 24 bp, Artificial Sequence
  source: /note="Description of Artificial Sequence: Synthetic primer"
tctttgggggaataatgactaaaa

SEQ ID NO: 298 - DNA, 24 bp, Artificial Sequence
  source: /note="Description of Artificial Sequence: Synthetic primer"
tttggcatttatgggaataaaact

SEQ ID NO: 299 - DNA, 23 bp, Artificial Sequence
  source: /note="Description of Artificial Sequence: Synthetic primer"
actaattctggtcaagcccatca

SEQ ID NO: 300 - DNA, 24 bp, Artificial Sequence
  source: /note="Description of Artificial Sequence: Synthetic primer"
ttaagacatcggatgaacagaaag

SEQ ID NO: 301 - DNA, 23 bp, Artificial Sequence
  source: /note="Description of Artificial Sequence: Synthetic primer"
agaagctttctgacatgatctgc

SEQ ID NO: 302 - DNA, 24 bp, Artificial Sequence
  source: /note="Description of Artificial Sequence: Synthetic primer"
tcaattgcattaggacttagacca

SEQ ID NO: 303 - DNA, 24 bp, Artificial Sequence
  source: /note="Description of Artificial Sequence: Synthetic primer"
gttaaattacctgtgaagcccttg

SEQ ID NO: 304 - DNA, 24 bp, Artificial Sequence
  source: /note="Description of Artificial Sequence: Synthetic primer"
cggaaaacagatccactttatgat

SEQ ID NO: 305 - DNA, 24 bp, Artificial Sequence
  source: /note="Description of Artificial Sequence: Synthetic primer"
aaatccactggaaacatcttgagt

SEQ ID NO: 306 - DNA, 24 bp, Artificial Sequence
  source: /note="Description of Artificial Sequence: Synthetic primer"
agtctcttcagaatcatgccctat

SEQ ID NO: 307 - DNA, 22 bp, Artificial Sequence
  source: /note="Description of Artificial Sequence: Synthetic primer"
gcttggtggcacatacctgtag

SEQ ID NO: 308 - DNA, 24 bp, Artificial Sequence
  source: /note="Description of Artificial Sequence: Synthetic primer"
ggtaggtagatttgcttgcttgtt

SEQ ID NO: 309 - DNA, 24 bp, Artificial Sequence
  source: /note="Description of Artificial Sequence: Synthetic primer"
agctctcagcagagtagggattta

SEQ ID NO: 310 - DNA, 21 bp, Artificial Sequence
  source: /note="Description of Artificial Sequence: Synthetic primer"
gtgagtctactgcaccccatc

SEQ ID NO: 311 - DNA, 24 bp, Artificial Sequence
  source: /note="Description of Artificial Sequence: Synthetic primer"
tgacactgtgaagtcaattctgtc

SEQ ID NO: 312 - DNA, 24 bp, Artificial Sequence
  source: /note="Description of Artificial Sequence: Synthetic primer"
tcaagaacttgacaatgagcaaat

SEQ ID NO: 313 - DNA, 22 bp, Artificial Sequence
  source: /note="Description of Artificial Sequence: Synthetic primer"
tatccgatccactgttgtgtgt

SEQ ID NO: 314 - DNA, 23 bp, Artificial Sequence
  source: /note="Description of Artificial Sequence: Synthetic primer"
caggagacccaaaaccactctac

SEQ ID NO: 315 - DNA, 24 bp, Artificial Sequence
  source: /note="Description of Artificial Sequence: Synthetic primer"
ttgttctacaaatagggcttcctt

SEQ ID NO: 316 - DNA, 24 bp, Artificial Sequence
  source: /note="Description of Artificial Sequence: Synthetic primer"
tgttaagtttgggcttatgttcct

SEQ ID NO: 317 - DNA, 23 bp, Artificial Sequence
  source: /note="Description of Artificial Sequence: Synthetic primer"
cacaagtctcactgcacaaacat

SEQ ID NO: 318 - DNA, 24 bp, Artificial Sequence
  source: /note="Description of Artificial Sequence: Synthetic primer"
tgacccatgattatctctctttga

SEQ ID NO: 319 - DNA, 24 bp, Artificial Sequence
  source: /note="Description of Artificial Sequence: Synthetic primer"
ttcagcttctgattggttttaatg

SEQ ID NO: 320 - DNA, 24 bp, Artificial Sequence
  source: /note="Description of Artificial Sequence: Synthetic primer"
ccaattccttaattttccctacag

SEQ ID NO: 321 - DNA, 21 bp, Artificial Sequence
  source: /note="Description of Artificial Sequence: Synthetic primer"
atctcagaccaggagggagac

SEQ ID NO: 322 - DNA, 24 bp, Artificial Sequence
  source: /note="Description of Artificial Sequence: Synthetic primer"
cctcagggtcagtacatttttcag

SEQ ID NO: 323 - DNA, 24 bp, Artificial Sequence
  source: /note="Description of Artificial Sequence: Synthetic primer"
ttcttaggacattgctccacatac

SEQ ID NO: 324 - DNA, 24 bp, Artificial Sequence
  source: /note="Description of Artificial Sequence: Synthetic primer"
gcaaacataatgcaactcgtaatc

SEQ ID NO: 325 - DNA, 21 bp, Artificial Sequence
  source: /note="Description of Artificial Sequence: Synthetic primer"
gcaagggagtctgtgtctttg

SEQ ID NO: 326 - DNA, 24 bp, Artificial Sequence
  source: /note="Description of Artificial Sequence: Synthetic primer"
tcatttaagtggctgttctgtgtt

SEQ ID NO: 327 - DNA, 24 bp, Artificial Sequence
  source: /note="Description of Artificial Sequence: Synthetic primer"
acaaaacagagagaaaaggcagag

SEQ ID NO: 328 - DNA, 23 bp, Artificial Sequence
  source: /note="Description of Artificial Sequence: Synthetic primer"
gttttgatttctggtgcctacag

SEQ ID NO: 329 - DNA, 20 bp, Artificial Sequence
  source: /note="Description of Artificial Sequence: Synthetic primer"
actgaagctgaagcccagtc

SEQ ID NO: 330 - DNA, 23 bp, Artificial Sequence
  source: /note="Description of Artificial Sequence: Synthetic primer"
acatgagctctcaggtttctgac

SEQ ID NO: 331 - DNA, 25 bp, Artificial Sequence
  source: /note="Description of Artificial Sequence: Synthetic primer"
tcaaacttagatggttccctatgtt

SEQ ID NO: 332 - DNA, 24 bp, Artificial Sequence
  source: /note="Description of Artificial Sequence: Synthetic primer"
gtaccctgaaaatgtagggtgact

SEQ ID NO: 333 - DNA, 20 bp, Artificial Sequence
  source: /note="Description of Artificial Sequence: Synthetic primer"
cacttcccaagtgaggcaat

SEQ ID NO: 334 - DNA, 24 bp, Artificial Sequence
  source: /note="Description of Artificial Sequence: Synthetic primer"
ctatacttggggctgacttgctac

SEQ ID NO: 335 - DNA, 24 bp, Artificial Sequence
  source: /note="Description of Artificial Sequence: Synthetic primer"
tcgtataggttactttggctcaca

SEQ ID NO: 336 - DNA, 24 bp, Artificial Sequence
  source: /note="Description of Artificial Sequence: Synthetic primer"
agggatctttactcctcagtgtgt

SEQ ID NO: 337 - DNA, 24 bp, Artificial Sequence
  source: /note="Description of Artificial Sequence: Synthetic primer"
tgtagaagttggaatatcctgctg

SEQ ID NO: 338 - DNA, 24 bp, Artificial Sequence
  source: /note="Description of Artificial Sequence: Synthetic primer"
gtcaacaatttgatctcaggcttc

SEQ ID NO: 339 - DNA, 24 bp, Artificial Sequence
  source: /note="Description of Artificial Sequence: Synthetic primer"
ctcagtactaaagatggacgcttg

SEQ ID NO: 340 - DNA, 24 bp, Artificial Sequence
  source: /note="Description of Artificial Sequence: Synthetic primer"
aatcatttcagtcttcccaacaat

SEQ ID NO: 341 - DNA, 24 bp, Artificial Sequence
  source: /note="Description of Artificial Sequence: Synthetic primer"
gggaatcacagtagatgtttgtca

SEQ ID NO: 342 - DNA, 24 bp, Artificial Sequence
  source: /note="Description of Artificial Sequence: Synthetic primer"
agaccaggaggtaagaacattttg

SEQ ID NO: 343 - DNA, 24 bp, Artificial Sequence
  source: /note="Description of Artificial Sequence: Synthetic primer"
ccacatagaaagagacttgcagaa

SEQ ID NO: 344 - DNA, 24 bp, Artificial Sequence
  source: /note="Description of Artificial Sequence: Synthetic primer"
agagatgccaaaagaacagtcaat

SEQ ID NO: 345 - DNA, 24 bp, Artificial Sequence
  source: /note="Description of Artificial Sequence: Synthetic primer"
tgtgccttaggctatgtaaactgt

SEQ ID NO: 346 - DNA, 24 bp, Artificial Sequence
  source: /note="Description of Artificial Sequence: Synthetic primer"
aaacccttgtaaccaaaattacca

SEQ ID NO: 347 - DNA, 24 bp, Artificial Sequence
  source: /note="Description of Artificial Sequence: Synthetic primer"
taactgcatcagaagtccttgcta

SEQ ID NO: 348 - DNA, 22 bp, Artificial Sequence
  source: /note="Description of Artificial Sequence: Synthetic primer"
ggagaccaagctgctaaagtca

SEQ ID NO: 349 - DNA, 37 bp, Artificial Sequence
  source: /note="Description of Artificial Sequence: Synthetic primer"
gtggtgccgcgggagtttggctcaaattgttactctt

SEQ ID NO: 350 - DNA, 37 bp, Artificial Sequence
  source: /note="Description of Artificial Sequence: Synthetic primer"
gtggtgccgcgggggaaatggtctaggagagtaaagt

SEQ ID NO: 351 - DNA, 34 bp, Artificial Sequence
  source: /note="Description of Artificial Sequence: Synthetic primer"
gtggtgccgcgggagaggttatgtggctttacca

SEQ ID NO: 352 - DNA, 32 bp, Artificial Sequence
  source: /note="Description of Artificial Sequence: Synthetic primer"
gtggtgccgcggctcattctcatgcctggaca

SEQ ID NO: 353 - DNA, 32 bp, Artificial Sequence
  source: /note="Description of Artificial Sequence: Synthetic primer"
gtggtgccgcggcgggcttggacagaacttac

SEQ ID NO: 354 - DNA, 32 bp, Artificial Sequence
  source: /note="Description of Artificial Sequence: Synthetic primer"
gtggtgccgcggctgcgtagtgccaaaacaaa

SEQ ID NO: 355 - DNA, 36 bp, Artificial Sequence
  source: /note="Description of Artificial Sequence: Synthetic primer"
gtggtgccgcggtaatttcattgaagagtggctgaa

SEQ ID NO: 356 - DNA, 36 bp, Artificial Sequence
  source: /note="Description of Artificial Sequence: Synthetic primer"
gtggtgccgcggaagccctgtgtggtagtagtcagt

SEQ ID NO: 357 - DNA, 36 bp, Artificial Sequence
  source: /note="Description of Artificial Sequence: Synthetic primer"
gtggtgccgcggcaagtcagaagtcacttgctttgt

SEQ ID NO: 358 - DNA, 36 bp, Artificial Sequence
  source: /note="Description of Artificial Sequence: Synthetic primer"
gtggtgccgcggttttatgtgcaggaatcagtctgt

SEQ ID NO: 359 - DNA, 36 bp, Artificial Sequence
  source: /note="Description of Artificial Sequence: Synthetic primer"
gtggtgccgcggtgtgtgcttctgtacacatcatct

SEQ ID NO: 360 - DNA, 36 bp, Artificial Sequence
  source: /note="Description of Artificial Sequence: Synthetic primer"
gtggtgccgcggagatttcaaccctcaaaaactgag

SEQ ID NO: 361 - DNA, 36 bp, Artificial Sequence
  source: /note="Description of Artificial Sequence: Synthetic primer"
gtggtgccgcggttgggaacatcagagaaagtatga

SEQ ID NO: 362 - DNA, 36 bp, Artificial Sequence
  source: /note="Description of Artificial Sequence: Synthetic primer"
gtggtgccgcggacaaattacagtctcctgggaaag

SEQ ID NO: 363 - DNA, 32 bp, Artificial Sequence
  source: /note="Description of Artificial Sequence: Synthetic primer"
gtggtgccgcggcacttcccaagtgaggcaat

SEQ ID NO: 364 - DNA, 36 bp, Artificial Sequence
  source: /note="Description of Artificial Sequence: Synthetic primer"
gtggtgccgcggctatacttggggctgacttgctac

SEQ ID NO: 365 - DNA, 34 bp, Artificial Sequence
  source: /note="Description of Artificial Sequence: Synthetic primer"
gtggtgccgcggttggctctttagcttgtgtttc

SEQ ID NO: 366 - DNA, 32 bp, Artificial Sequence
  source: /note="Description of Artificial Sequence: Synthetic primer"
gtggtgccgcggtgagactcccaaaggcaatc

SEQ ID NO: 367 - DNA, 34 bp, Artificial Sequence; identical to SEQ ID NO: 365
  source: /note="Description of Artificial Sequence: Synthetic primer"

SEQ ID NO: 368 - DNA, 32 bp, Artificial Sequence
  source: /note="Description of Artificial Sequence: Synthetic primer"
gtggtgccgcggactgaggggtgatcttggtg

SEQ ID NO: 369 - DNA, 32 bp, Artificial Sequence
  source: /note="Description of Artificial Sequence: Synthetic primer"
gtggtgccgcgggcagagaaagccagtcggta

SEQ ID NO: 370 - DNA, 32 bp, Artificial Sequence; identical to SEQ ID NO: 366
  source: /note="Description of Artificial Sequence: Synthetic primer"

SEQ ID NO: 371 - DNA, 32 bp, Artificial Sequence; identical to SEQ ID NO: 369
  source: /note="Description of Artificial Sequence: Synthetic primer"

SEQ ID NO: 372 - DNA, 32 bp, Artificial Sequence; identical to SEQ ID NO: 368
  source: /note="Description of Artificial Sequence: Synthetic primer"

SEQ ID NO: 373 - DNA, 32 bp, Artificial Sequence
  source: /note="Description of Artificial Sequence: Synthetic primer"
gtggtgccgcggccagagttcctagggcagag

SEQ ID NO: 374 - DNA, 32 bp, Artificial Sequence
  source: /note="Description of Artificial Sequence: Synthetic primer"
gtggtgccgcggagctagtccccacattccac

SEQ ID NO: 375 - DNA, 32 bp, Artificial Sequence; identical to SEQ ID NO: 373
  source: /note="Description of Artificial Sequence: Synthetic primer"

SEQ ID NO: 376 - DNA, 32 bp, Artificial Sequence
  source: /note="Description of Artificial Sequence: Synthetic primer"
gtggtgccgcggggtggagggaaactttaggc

SEQ ID NO: 377 - DNA, 32 bp, Artificial Sequence; identical to SEQ ID NO: 352
  source: /note="Description of Artificial Sequence: Synthetic primer"

SEQ ID NO: 378 - DNA, 32 bp, Artificial Sequence; identical to SEQ ID NO: 374
  source: /note="Description of Artificial Sequence: Synthetic primer"

SEQ ID NO: 379 - DNA, 34 bp, Artificial Sequence
  source: /note="Description of Artificial Sequence: Synthetic primer"
gtggtgccgcggtctcatgcctggacaagtaact

SEQ ID NO: 380 - DNA, 32 bp, Artificial Sequence; identical to SEQ ID NO: 376
  source: /note="Description of Artificial Sequence: Synthetic primer"

SEQ ID NO: 381 - DNA, 32 bp, Artificial Sequence
  source: /note="Description of Artificial Sequence: Synthetic primer"
gtggtgccgcggggcttggacagaacttaccg

SEQ ID NO: 382 - DNA, 32 bp, Artificial Sequence
  source: /note="Description of Artificial Sequence: Synthetic primer"
gtggtgccgcggcaccactgtctgcctaagga

SEQ ID NO: 383 - DNA, 32 bp, Artificial Sequence; identical to SEQ ID NO: 381
  source: /note="Description of Artificial Sequence: Synthetic primer"

SEQ ID NO: 384 - DNA, 32 bp, Artificial Sequence; identical to SEQ ID NO: 376
  source: /note="Description of Artificial Sequence: Synthetic primer"

SEQ ID NO: 385 - DNA, 33 bp, Artificial Sequence
  source: /note="Description of Artificial Sequence: Synthetic primer"
gtggtgccgcggcgtagtgccaaaacaaacagt

SEQ ID NO: 386 - DNA, 32 bp, Artificial Sequence; identical to SEQ ID NO: 382
  source: /note="Description of Artificial Sequence: Synthetic primer"

SEQ ID NO: 387 - DNA, 33 bp, Artificial Sequence; identical to SEQ ID NO: 385
  source: /note="Description of Artificial Sequence: Synthetic primer"

SEQ ID NO: 388 - DNA, 32 bp, Artificial Sequence; identical to SEQ ID NO: 376
  source: /note="Description of Artificial Sequence: Synthetic primer"

SEQ ID NO: 389 - DNA, 32 bp, Artificial Sequence
  source: /note="Description of Artificial Sequence: Synthetic primer"
gtggtgccgcgggcgagggcctacttgatatg

SEQ ID NO: 390 - DNA, 32 bp, Artificial Sequence
  source: /note="Description of Artificial Sequence: Synthetic primer"
gtggtgccgcggcttcccaagtgaggcaatgc

SEQ ID NO: 391 - DNA, 33 bp, Artificial Sequence
  source: /note="Description of Artificial Sequence: Synthetic primer"
gtggtgccgcggacgttttgtgctgctgtaaca

SEQ ID NO: 392 - DNA, 32 bp, Artificial Sequence
  source: /note="Description of Artificial Sequence: Synthetic primer"
gtggtgccgcggctgcaggcacattctcttcc

SEQ ID NO: 393 - DNA, 32 bp, Artificial Sequence
  source: /note="Description of Artificial Sequence: Synthetic primer"
gtggtgccgcgggccctgtgtggtagtagtca

SEQ ID NO: 394 - DNA, 32 bp, Artificial Sequence; identical to SEQ ID NO: 390
  source: /note="Description of Artificial Sequence: Synthetic primer"

SEQ ID NO: 395 - DNA, 33 bp, Artificial Sequence
  source: /note="Description of Artificial Sequence: Synthetic primer"
gtggtgccgcggcagtattaaggggtgggagct

SEQ ID NO: 396 - DNA, 32 bp, Artificial Sequence
  source: /note="Description of Artificial Sequence: Synthetic primer"
gtggtgccgcggtctcttcctcacacagctga

SEQ ID NO: 397 - DNA, 32 bp, Artificial Sequence
  source: /note="Description of Artificial Sequence: Synthetic primer"
gtggtgccgcggggagcttggagggaagagaa

SEQ ID NO: 398 - DNA, 32 bp, Artificial Sequence; identical to SEQ ID NO: 390
  source: /note="Description of Artificial Sequence: Synthetic primer"

SEQ ID NO: 399 - DNA, 32 bp, Artificial Sequence
  source: /note="Description of Artificial Sequence: Synthetic primer"
gtggtgccgcggatggatggggaagacactgg

SEQ ID NO: 400 - DNA, 32 bp, Artificial Sequence; identical to SEQ ID NO: 392
  source: /note="Description of Artificial Sequence: Synthetic primer"

SEQ ID NO: 401 - DNA, 32 bp, Artificial Sequence
  source: /note="Description of Artificial Sequence: Synthetic primer"
gtggtgccgcggggatgaaacagggcaggaac

SEQ ID NO: 402 - DNA, 31 bp, Artificial Sequence
  source: /note="Description of Artificial Sequence: Synthetic primer"
gtggtgccgcggttcccaagtgaggcaatgc

SEQ ID NO: 403 - DNA, 32 bp, Artificial Sequence
  source: /note="Description of Artificial Sequence: Synthetic primer"
gtggtgccgcggtttgcagagccatgatgagg

SEQ ID NO: 404 - DNA, 30 bp, Artificial Sequence
  source: /note="Description of Artificial Sequence: Synthetic primer"
gtggtgccgcggcgacagccaaaacagccg

SEQ ID NO: 405 - DNA, 44 bp, Artificial Sequence
  source: /note="Description of Artificial Sequence: Synthetic oligonucleotide"
aaaatattttagctcctactcagactgttactctggtgacacaa

SEQ ID NO: 406 - DNA, 44 bp, Artificial Sequence
  source: /note="Description of Artificial Sequence: Synthetic oligonucleotide"
ttgtgtcaccagagtaacagtctgagtaggagctaaaatatttt

SEQ ID NO: 407 - DNA, 36 bp, Artificial Sequence
  source: /note="Description of Artificial Sequence: Synthetic oligonucleotide"
tagctcctactcagactgttactctggtgacacaac

SEQ ID NO: 408 - DNA, 28 bp, Artificial Sequence
  source: /note="Description of Artificial Sequence: Synthetic oligonucleotide"
tagctcctactcagactggtgacccaac

SEQ ID NO: 409 - DNA, 24 bp, Artificial Sequence
  source: /note="Description of Artificial Sequence: Synthetic oligonucleotide"
tagctcctactctggtgacacaac

SEQ ID NO: 410 - DNA, 28 bp, Artificial Sequence
  source: /note="Description of Artificial Sequence: Synthetic oligonucleotide"
tagctcctactcagactggtgacacaac

SEQ ID NO: 411 - DNA, 16 bp, Artificial Sequence
  source: /note="Description of Artificial Sequence: Synthetic oligonucleotide"
tagctcctactcagac

SEQ ID NO: 412 - DNA, 27 bp, Artificial Sequence
  source: /note="Description of Artificial Sequence: Synthetic oligonucleotide"
tagctcctactcagactgttacacaac

SEQ ID NO: 413 - DNA, 30 bp, Artificial Sequence
  source: /note="Description of Artificial Sequence: Synthetic oligonucleotide"
tagctcctactcagactgtggtgaggtgac

SEQ ID NO: 414 - DNA, 32 bp, Artificial Sequence
  source: /note="Description of Artificial Sequence: Synthetic oligonucleotide"
tagctcctactcagactctctggtgacacaac

SEQ ID NO: 415 - DNA, 31 bp, Artificial Sequence
  source: /note="Description of Artificial Sequence: Synthetic oligonucleotide"
tagctcctactcagacctctggtgacacaac

SEQ ID NO: 416 - DNA, 32 bp, Artificial Sequence
  source: /note="Description of Artificial Sequence: Synthetic oligonucleotide"
tagctcctactcaggctgtctggtgacacaac

SEQ ID NO: 417 - DNA, 33 bp, Artificial Sequence
  source: /note="Description of Artificial Sequence: Synthetic oligonucleotide"
tagctcctactcagactactctggtgacacaac

SEQ ID NO: 418 - DNA, 28 bp, Artificial Sequence
  source: /note="Description of Artificial Sequence: Synthetic oligonucleotide"
tagctcctactcagactgttgacacaac

SEQ ID NO: 419 - DNA, 13 bp, Artificial Sequence
  source: /note="Description of Artificial Sequence: Synthetic oligonucleotide"
ctggtgacacaac

SEQ ID NO: 420 - DNA, 29 bp, Artificial Sequence
  source: /note="Description of Artificial Sequence: Synthetic oligonucleotide"
tagctcctactcagactgttagacacaac

SEQ ID NO: 421 - DNA, 33 bp, Artificial Sequence
  source: /note="Description of Artificial Sequence: Synthetic oligonucleotide"
tagctcctactcagactgctctggtgacacaac

SEQ ID NO: 422 - DNA, 20 bp, Artificial Sequence
  source: /note="Description of Artificial Sequence: Synthetic oligonucleotide"
cagactgttactctggtgac

SEQ ID NO: 423 - DNA, 29 bp, Artificial Sequence
  source: /note="Description of Artificial Sequence: Synthetic oligonucleotide"
cagaccacctgtggtctcctactggtgac

SEQ ID NO: 424 - DNA, 18 bp, Artificial Sequence
  source: /note="Description of Artificial Sequence: Synthetic oligonucleotide"
gctttgatttccctaggg

SEQ ID NO: 425 - DNA, 25 bp, Artificial Sequence
  source: /note="Description of Artificial Sequence: Synthetic oligonucleotide"
gctttgatttccagttcttaggcaa

SEQ ID NO: 426 - DNA, 18 bp, Artificial Sequence
  source: /note="Description of Artificial Sequence: Synthetic oligonucleotide"
gctttgattcttaggcaa

SEQ ID NO: 427 - DNA, 62 bp, Artificial Sequence
  source: /note="Description of Artificial Sequence: Synthetic oligonucleotide"
  modified_base (13)..(53): a, c, t, g, unknown or other
gctttgatttccnnnnnnnnnnnnnnnnnnnnnnnnnnnnnnnnnnnnnnnnncttaggcaa

SEQ ID NO: 428 - DNA, 18 bp, Artificial Sequence
  source: /note="Description of Artificial Sequence: Synthetic oligonucleotide"
tcttaaccattaccatag

SEQ ID NO: 429 - DNA, 32 bp, Artificial Sequence
  source: /note="Description of Artificial Sequence: Synthetic oligonucleotide"
tcttaaccattaccatagagttcttaggcaac

SEQ ID NO: 430 - DNA, 30 bp, Artificial Sequence
  source: /note="Description of Artificial Sequence: Synthetic oligonucleotide"
tcttaaccattaccaaagttcttaggcaac

SEQ ID NO: 431 - DNA, 31 bp, Artificial Sequence
  source: /note="Description of Artificial Sequence: Synthetic oligonucleotide"
tcttaaccattaccataggttcttaggcaac

SEQ ID NO: 432 - DNA, 14 bp, Artificial Sequence
  source: /note="Description of Artificial Sequence: Synthetic oligonucleotide"
gaaccaaacccact

SEQ ID NO: 433 - DNA, 24 bp, Artificial Sequence
  source: /note="Description of Artificial Sequence: Synthetic oligonucleotide"
gaaccaaacccacttaggggataa

SEQ ID NO: 434 - DNA, 2328 bp, Artificial Sequence
  source: /note="Description of Artificial Sequence: Synthetic polynucleotide"
atgaggtctgactacaaagaccatgacggtgattataaagatcatgacatcgattacaaggatgacgatgacaagatggcccccaagaagaagaggaaggtgggcctcgagcccggagaaaaaccgtacaagtgccctgagtgcgggaaatcattctccgaccctggggcgctcgtccggcaccaaaggacgcatacaggggaaaagccgtataagtgccccgagtgtggaaagagcttctcgcagagagcccaccttgaacgacaccaaagaacacacactggtgagaaaccctataagtgtccagagtgcggcaaatcgtttagcagatccgatgacttggtgcgccaccagcggacacacacgggtgaaaagccctacaaatgcccggagtgtgggaagtcgttttcaaggtcggatcatctgactacccatcagcgcacccatacgggagcggccgcccgcgccctggtgaagagcgagctggaggagaagaagtccgagctgcggcacaagctgaagtacgtgccccacgagtacatcgagctgatcgagatcgccaggaaccccacccaggaccgcatcctggagatgaaggtgatggagttcttcatgaaggtgtacggctacaggggagagcacctgggcggaagcagaaagcctgacggcgccatctatacagtgggcagccccatcgattacggcgtgatcgtggacacaaaggcctacagcggcggctacaatctgcctatcggccaggccgacgagatgcagagatacgtgaaggagaaccagacccggaataagcacatcaaccccaacgagtggtggaaggtgtaccctagcagcgtgaccgagttcaagttcctgttcgtgagcggccacttcaagggcaactacaaggcccagctgaccaggctgaaccgcaaaaccaactgcaatggcgccgtgctgagcgtggaggagctgctgatcggcggcgagatgatcaaagccggcaccctgacactggaggaggtgcggcgcaagttcaacaacggcgagatcaacttcgagggcagaggaagtcttctaacatgcggtgacgtggaggagaatcccggccctagatctgactacaaagaccatgacggtgattataaagatcatgacatcgattacaaggatgacgatgacaagatggcccccaagaagaagaggaaggtgggcctcgagccgggagagaagccgtacaagtgtcccgaatgtggaaagagcttctcacagtcgggggaccttcggcgccaccagcgcacacatactggtgaaaagccgtataagtgtccagaatgtggcaaatcattctccacatcagggagcctggtcaggcaccagcgaacccacacgggtgagaagccctataagtgccccgaatgcgggaagtccttttcgcagagagcccacttggagaggcaccagaggacccatacgggggagaaaccttacaagtgccctgaatgcggaaagtcgttctcgacccatctggatctcatcagacatcagagaacgcacactggagagaaaccctacaaatgtcccgagtgtgggaagtcgtttagccgaaaggacaatctcaaaaaccatcaacggacacacacgggtgaaaaaccatacaaatgcccggagtgcggcaaatcgttttcccaacttgcgcacttgcgggcacaccaacgcacgcatactggagcggccgcccgcgccctggtgaagagcgagctggaggagaagaagtccgagctgcggcacaagctgaagtacgtgccccacgagtacatcgagctgatcgagatcgccaggaaccccacccaggaccgcatcctggagatgaaggtgatggagttcttcatgaaggtgtacggctacaggggagagcacctgggcggaagcagaaagcctgacggcgccatctatacagtgggcagccccatcgattacggcgtgatcgtggacacaaaggcctacagcggcggctacaatctgcctatcggccaggccgacgagatggagagatacgtggaggagaaccagacacgggataagcacctcaaccccaacgagtggtggaaggtgtaccctagcagcgtgaccgagttcaagttcctgttcgtgagcggccacttcaagggcaactacaaggcccagctgaccaggctgaaccacatcaccaactgcaatggcgccgtgctgagcgtggaggagctgctgatcggcggcgagatgatcaaagccggcaccctgacactggaggaggtgcggcgcaagttcaacaacggcgagatcaacttctga

SEQ ID NO: 435 - protein, 775 aa, Artificial Sequence
  source: /note="Description of Artificial Sequence: Synthetic polypeptide"
MRSDYKDHDGDYKDHDIDYKDDDDKMAPKKKRKVGLEPGEKPYKCPECGKSFSDPGALVRHQRTHTGEKPYKCPECGKSFSQRAHLERHQRTHTGEKPYKCPECGKSFSRSDDLVRHQRTHTGEKPYKCPECGKSFSRSDHLTTHQRTHTGAAARALVKSELEEKKSELRHKLKYVPHEYIELIEIARNPTQDRILEMKVMEFFMKVYGYRGEHLGGSRKPDGAIYTVGSPIDYGVIVDTKAYSGGYNLPIGQADEMQRYVKENQTRNKHINPNEWWKVYPSSVTEFKFLFVSGHFKGNYKAQLTRLNRKTNCNGAVLSVEELLIGGEMIKAGTLTLEEVRRKFNNGEINFEGRGSLLTCGDVEENPGPRSDYKDHDGDYKDHDIDYKDDDDKMAPKKKRKVGLEPGEKPYKCPECGKSFSQSGDLRRHQRTHTGEKPYKCPECGKSFSTSGSLVRHQRTHTGEKPYKCPECGKSFSQRAHLERHQRTHTGEKPYKCPECGKSFSTHLDLIRHQRTHTGEKPYKCPECGKSFSRKDNLKNHQRTHTGEKPYKCPECGKSFSQLAHLRAHQRTHTGAAARALVKSELEEKKSELRHKLKYVPHEYIELIEIARNPTQDRILEMKVMEFFMKVYGYRGEHLGGSRKPDGAIYTVGSPIDYGVIVDTKAYSGGYNLPIGQADEMERYVEENQTRDKHLNPNEWWKVYPSSVTEFKFLFVSGHFKGNYKAQLTRLNHITNCNGAVLSVEELLIGGEMIKAGTLTLEEVRRKFNNGEINF

SEQ ID NO: 436 - DNA, 4725 bp, Artificial Sequence
  source: /note="Description of Artificial Sequence: Synthetic polynucleotide"
tggccactccctctatgcgcactcgctcgctcggtggggcctggcgaccaaaggtcgccagacggacgtgctttgcacgtccggccccaccgagcgagcgagtgcgcatagagggagtggccaactccatcactagaggtatggcagtgacgtaacgcgaagcgcgcgaagcgagaccacgcctaccagctgcgtcagcagtcaggtgacccttttgcgacagtttgcgacaccacgtggccgctgagggtatatattctcgagtgagcgaaccaggagctccattttgaccgcgaaatttgaacgagcagcagccatgccggggttctacgagattgtcctgaaggtcccgagtgacctggacgagcacctgccgggcatttctaactcgtttgttaactgggtggccgagaaggaatgggagctgccgccggattctgacatggatccgaatctgattgagcaggcacccctgaccgtggccgaaaagcttcagcgcgagttcctggtggagtggcgccgcgtgagtaaggccccggaggccctcttttttgtccagttcgaaaagggggagacctacttccacctgcacgtgctgattgagaccatcggggtcaaatccatggtggtcggccgctacgtgagccagattaaagagaagctggtgacccgcatctaccgcggggtcgagccgcagcttccgaactggttcgcggtgaccaaaacgcgaaatggcgccgggggcgggaacaaggtggtggacgactgctacatccccaactacctgctccccaagacccagcccgagctccagtgggcgtggactaacatggaccagtatttaagcgcctgtttgaatctcgcggagcgtaaacggctggtggcgcagcatctgacgcacgtgtcgcagacgcaggagcagaacaaagagaatcagaaccccaattctgacgcgccggtcatcaggtcaaaaacctcagccaggtacatggagctggtcgggtggctggtggaccgcgggatcacgtcagaaaagcaatggattcaggaggaccaggcctcgtacatctccttcaacgccgcctccaactcgcggtcccagatcaaggccgcgctggacaatgcctccaagatcatgagcctgacaaagacggctccggactacctggtgggcagcaacccgccggaggacattaccaaaaatcggatctaccaaatcctggagctgaacgggtacgatccgcagtacgcggcctccgtcttcctgggctgggcgcaaaagaagttcgggaagaggaacaccatctggctctttgggccggccacgacgggtaaaaccaacatcgcggaagccatcgcccacgccgtgcccttctacggctgcgtaaactggaccaatgagaactttcccttcaacgattgcgtcgacaagatggtgatctggtgggaggagggcaagatgacggccaaggtcgtggagagcgccaaggccattctgggcggaagcaaggtgcgcgtggaccaaaagtgcaagtcatcggcccagatcgaacccactcccgtgatcgtcacctccaacaccaacatgtgcgccgtgattgacgggaacagcaccaccttcgagcatcagcagccgctgcaggaccggatgtttaaatttgaacttacccgccgtttggaccatgactttgggaaggtcaccaaacaggaagtaaaggactttttccggtgggcttccgatcacgtgactgacgtggctcatgagttctacgtcagaaagggtggagctaagaaacgccccgcctccaatgacgcggatgtaagcgagccaaaacggcagtgcacgtcacttgcgcagccgacaacgtcagacgcggaagcaccggcggactacgcggacaggtaccaaaacaaatgttctcgtcacgtgggcatgaatctgatgctttttccctgtaaaacatgcgagagaatgaatcaaatttccaatgtctgttttacgcatggtcaaagagactgtggggaatgcttccctggaatgtcagaatctcaacccgtttctgtcgtcaaaaagaagacttatcagaaactgtgtccaattcatcatatcctgggaagggcacccgagattgcctgttcggcctgcgatttggccaatgtggacttggatgactgtgtttctgagcaataaatgacttaaaccaggtatggctgctgacggttatcttccagattggctcgaggacaacctttctgaaggcattcgtgagtggtgggctctgaaacctggagtccctcaacccaaagcgaaccaacaacaccaggacaaccgtcggggtcttgtgcttccgggttacaaatacctcggacccggtaacggactcgacaaaggagagccggtcaacgaggcggacgcggcagccctcgaacacgacaaagcttacgaccagcagctcaaggccggtgacaacccgtacctcaagtacaaccacgccgacgccgagtttcaggagcgtcttcaagaagatacgtcttttgggggcaaccttggcagagcagtcttccaggccaaaaagaggatccttgagcctcttggtctggttgaggaagcagctaaaacggctcctggaaagaagaggcctgtagatcagtctcctcaggaaccggactcatcatctggtgttggcaaatcgggcaaacagcctgccagaaaaagactaaatttcggtcagactggcgactcagagtcagtcccagaccctcaacctctcggagaaccaccagcagcccccacaagtttgggatctaatacaatggcttcaggcggtggcgcaccaatggcagacaataacgagggtgccgatggagtgggtaattcctcaggaaattggcattgcgattcccaatggctgggcgacagagtcatcaccaccagcaccagaacctgggccctgcccacttacaacaaccatctctacaagcaaatctccagcgcttcaacgggagcttcaaacgacaaccactactttggctacagcaccccttgggggtattttgactttaacagattccactgccacttctcaccacgtgactggcagcgactcattaacaacaactggggattccggcccaagaaactcagcttcaagctcttcaacatccaagttaaagaggtcacgcagaacgatggcacgacgactattgccaataaccttaccagcacggttcaagtgtttacggactcggagtatcagctcccgtacgtgctcgggtcggcgcaccaaggctgtctcccgccgtttccagcggacgtcttcatggtccctcagtatggatacctcaccctgaacaacggaagtcaagcggtgggacgctcatccttttactgcctggagtacttcccttcgcagatgctaaggactggaaataacttccaattcagctataccttcgaggatgtaccttttcacagcagctacgctcacagccagagtttggatcgcttgatgaatcctcttattgatcagtatctgtactacctgaacagaacgcaaggaacaacctctggaacaaccaaccaatcacggctgctttttagccaggctgggcctcagtctatgtctttgcaggccagaaattggctacctgggccctgctaccggcaacagagactttcaaagactgctaacgacaacaacaacagtaactttccttggacagcggccagcaaatatcatctcaatggccgcgactcgctggtgaatccaggaccagctatggccagtcacaaggacgatgaagaaaaatttttccctatgcacggcaatctaatatttggcaaagaagggacaacggcaagtaacgcagaattagataatgtaatgattacggatgaagaagagattcgtaccaccaatcctgtggcaacagagcagtatggaactgtggcaaataacttgcagagctcaaatacagctcccacgactagaactgtcaatgatcagggggccttacctggcatggtgtggcaagatcgtgacgtgtaccttcaaggacctatctgggcaaagattcctcacacggatggacactttcatccttctcctctgatgggaggctttggactgaaacatccgcctcctcaaatcatgatcaaaaatactccggtaccggcaaatcctccgacgactttcagcccggccaagtttgcttcatttatcactcagtactccactggacaggtcagcgtggaaattgagtgggagctacagaaagaaaacagcaaacgttggaatccagagattcagtacacttccaactacaacaagtctgttaatgtggactttactgtagacactaatggtgtttatagtgaacctcgccctattggaacccggtatctcacacgaaacttgtaatcctggttaatcaataaaccgtttaattcgtttcagttgaactttggctcttgtgcacttcttatcttatcttgtttccatggctactgcgtagataagcagcggcctgcggcgcttgcgcttcgcggtttacaactgctggttaatatttaactctcgccatacctctagtgatggagttggccactccctctatgcgcactcgctcgctcggtggggccggacgtgcaaagcacgtccgtctggcgacctttggtcgccaggccccaccgagcgagcgagtgcgcatagagggagtggccaa

SEQ ID NO: 437 - protein, 737 aa, Artificial Sequence
  source: /note="Description of Artificial Sequence: Synthetic polypeptide"
MAADGYLPDWLEDNLSEGIREWWALKPGVPQPKANQQHQDNRRGLVLPGYKYLGPGNGLDKGEPVNEADAAALEHDKAYDQQLKAGDNPYLKYNHADAEFQERLQEDTSFGGNLGRAVFQAKKRILEPLGLVEEAAKTAPGKKRPVDQSPQEPDSSSGVGKSGKQPARKRLNFGQTGDSESVPDPQPLGEPPAAPTSLGSNTMASGGGAPMADNNEGADGVGNSSGNWHCDSQWLGDRVITTSTRTWALPTYNNHLYKQISSASTGASNDNHYFGYSTPWGYFDFNRFHCHFSPRDWQRLINNNWGFRPKKLSFKLFNIQVKEVTQNDGTTTIANNLTSTVQVFTDSEYQLPYVLGSAHQGCLPPFPADVFMVPQYGYLTLNNGSQAVGRSSFYCLEYFPSQMLRTGNNFQFSYTFEDVPFHSSYAHSQSLDRLMNPLIDQYLYYLNRTQGTTSGTTNQSRLLFSQAGPQSMSLQARNWLPGPCYRQQRLSKTANDNNNSNFPWTAASKYHLNGRDSLVNPGPAMASHKDDEEKFFPMHGNLIFGKEGTTASNAELDNVMITDEEEIRTTNPVATEQYGTVANNLQSSNTAPTTRTVNDQGALPGMVWQDRDVYLQGPIWAKIPHTDGHFHPSPLMGGFGLKHPPPQIMIKNTPVPANPPTTFSPAKFASFITQYSTGQVSVEIEWELQKENSKRWNPEIQYTSNYNKSVNVDFTVDTNGVYSEPRPIGTRYLTRNL

SEQ ID NO: 438 - protein, 406 aa, Artificial Sequence
  source: /note="Description of Artificial Sequence: Synthetic polypeptide"
MDYKDHDGDYKDHDIDYKDDDDKMAPKKKRKVGRLEPGEKPYKCPECGKSFSRKDALRGHQRTHTGEKPYKCPECGKSFSHRTTLTNHQRTHTGEKPYKCPECGKSFSQRNALAGHQRTHTGEKPYKCPECGKSFSHKNALQNHQRTHTGEKPYKCPECGKSFSDPGHLVRHQRTHTGEKPYKCPECGKSFSTSGNLVRHQRTHTGAAARALVKSELEEKKSELRHKLKYVPHEYIELIEIARNPTQDRILEMKVMEFFMKVYGYRGEHLGGSRKPDGAIYTVGSPIDYGVIVDTKAYSGGYNLPIGQADEMERYVEENQTRDKHLNPNEWWKVYPSSVTEFKFLFVSGHFKGNYKAQLTRLNHITNCNGAVLSVEELLIGGEMIKAGTLTLEEVRRKFNNGEINF

SEQ ID NO: 439 - protein, 406 aa, Artificial Sequence
  source: /note="Description of Artificial Sequence: Synthetic polypeptide"
MDYKDHDGDYKDHDIDYKDDDDKMAPKKKRKVGRLEPGEKPYKCPECGKSFSQQRSLVGHQRTHTGEKPYKCPECGKSFSDKKDLTRHQRTHTGEKPYKCPECGKSFSTSGHLVRHQRTHTGEKPYKCPECGKSFSQRAHLERHQRTHTGEKPYKCPECGKSFSTSGSLVRHQRTHTGEKPYKCPECGKSFSTSGNLVRHQRTHTGAAARALVKSELEEKKSELRHKLKYVPHEYIELIEIARNPTQDRILEMKVMEFFMKVYGYRGEHLGGSRKPDGAIYTVGSPIDYGVIVDTKAYSGGYNLPIGQADEMQRYVKENQTRNKHINPNEWWKVYPSSVTEFKFLFVSGHFKGNYKAQLTRLNRKTNCNGAVLSVEELLIGGEMIKAGTLTLEEVRRKFNNGEINF

SEQ ID NO: 440 - protein, 320 aa, Artificial Sequence
  source: /note="Description of Artificial Sequence: Synthetic polypeptide"
MDYKDHDGDYKDHDIDYKDDDDKMAPKKKRKVGRLEPGERPFQCRICMRNFSSKQALAVHTRTHTGEKPFQCRICMRNFSQSTTLKRHLRTHTGEKPFQCRICMRNFSRSDHLSLHLKTHLRGSQLVKSELEEKKSELRHKLKYVPHEYIELIEIARNPTQDRILEMKVMEFFMKVYGYRGEHLGGSRKPDGAIYTVGSPIDYGVIVDTKAYSGGYNLPIGQADEMQRYVKENQTRNKHINPNEWWKVYPSSVTEFKFLFVSGHFKGNYKAQLTRLNRKTNCNGAVLSVEELLIGGEMIKAGTLTLEEVRRKFNNGEINF

SEQ ID NO: 441 - protein, 320 aa, Artificial Sequence
  source: /note="Description of Artificial Sequence: Synthetic polypeptide"
MDYKDHDGDYKDHDIDYKDDDDKMAPKKKRKVGRLEPGERPFQCRICMRNFSRRAHLQNHTRTHTGEKPFQCRICMRNFSQSTTLKRHLRTHTGEKPFQCRICMRNFSDGGHLTRHLKTHLRGSQLVKSELEEKKSELRHKLKYVPHEYIELIEIARNPTQDRILEMKVMEFFMKVYGYRGEHLGGSRKPDGAIYTVGSPIDYGVIVDTKAYSGGYNLPIGQADEMERYVEENQTRDKHLNPNEWWKVYPSSVTEFKFLFVSGHFKGNYKAQLTRLNHITNCNGAVLSVEELLIGGEMIKAGTLTLEEVRRKFNNGEINF

SEQ ID NO: 442 - DNA, 42 bp, Artificial Sequence
  source: /note="Description of Artificial Sequence: Synthetic oligonucleotide"
caaactagaaatgccatcttccttgatgttggaggtacctgc

SEQ ID NO: 443 - protein, 406 aa, Artificial Sequence; identical to SEQ ID NO: 438
  source: /note="Description of Artificial Sequence: Synthetic polypeptide"

SEQ ID NO: 444 - protein, 406 aa, Artificial Sequence; identical to SEQ ID NO: 439
  source: /note="Description of Artificial Sequence: Synthetic polypeptide"

SEQ ID NO: 445 - DNA, 25 bp, Artificial Sequence
  source: /note="Description of Artificial Sequence: Synthetic oligonucleotide"
  Variation (1)..(1): /replace=" "
  Variation (25)..(25): /replace=" "
  misc_feature (1)..(25): /note="Variations given in the sequence have no preference with respect to those in the annotations"
tatctgcccatgactggcgcaggga

SEQ ID NO: 446 - protein, 320 aa, Artificial Sequence; identical to SEQ ID NO: 440
  source: /note="Description of Artificial Sequence: Synthetic polypeptide"

SEQ ID NO: 447 - protein, 320 aa, Artificial Sequence; identical to SEQ ID NO: 441
  source: /note="Description of Artificial Sequence: Synthetic polypeptide"

SEQ ID NO: 448 - DNA, 42 bp, Artificial Sequence
  source: /note="Description of Artificial Sequence: Synthetic oligonucleotide"
actagaaatgccatcttccttgatgttggaggtacctgctct

SEQ ID NO: 449 - protein, 406 aa, Artificial Sequence
  source: /note="Description of Artificial Sequence: Synthetic polypeptide"
MDYKDHDGDYKDHDIDYKDDDDKMAPKKKRKVGRLEPGEKPYKCPECGKSFSHRTTLTNHQRTHTGEKPYKCPECGKSFSQRNALAGHQRTHTGEKPYKCPECGKSFSHKNALQNHQRTHTGEKPYKCPECGKSFSDPGHLVRHQRTHTGEKPYKCPECGKSFSTSGNLVRHQRTHTGEKPYKCPECGKSFSQSSNLVRHQRTHTGAAARALVKSELEEKKSELRHKLKYVPHEYIELIEIARNPTQDRILEMKVMEFFMKVYGYRGEHLGGSRKPDGAIYTVGSPIDYGVIVDTKAYSGGYNLPIGQADEMERYVEENQTRDKHLNPNEWWKVYPSSVTEFKFLFVSGHFKGNYKAQLTRLNHITNCNGAVLSVEELLIGGEMIKAGTLTLEEVRRKFNNGEINF

SEQ ID NO: 450 - protein, 406 aa, Artificial Sequence
  source: /note="Description of Artificial Sequence: Synthetic polypeptide"
MDYKDHDGDYKDHDIDYKDDDDKMAPKKKRKVGRLEPGEKPYKCPECGKSFSQRNALAGHQRTHTGEKPYKCPECGKSFSQQRSLVGHQRTHTGEKPYKCPECGKSFSDKKDLTRHQRTHTGEKPYKCPECGKSFSTSGHLVRHQRTHTGEKPYKCPECGKSFSQRAHLERHQRTHTGEKPYKCPECGKSFSTSGSLVRHQRTHTGAAARALVKSELEEKKSELRHKLKYVPHEYIELIEIARNPTQDRILEMKVMEFFMKVYGYRGEHLGGSRKPDGAIYTVGSPIDYGVIVDTKAYSGGYNLPIGQADEMQRYVKENQTRNKHINPNEWWKVYPSSVTEFKFLFVSGHFKGNYKAQLTRLNRKTNCNGAVLSVEELLIGGEMIKAGTLTLEEVRRKFNNGEINF

SEQ ID NO: 451 - protein, 378 aa, Artificial Sequence
  source: /note="Description of Artificial Sequence: Synthetic polypeptide"
MDYKDHDGDYKDHDIDYKDDDDKMAPKKKRKVGRLEPGEKPYKCPECGKSFSQRNALAGHQRTHTGEKPYKCPECGKSFSHKNALQNHQRTHTGEKPYKCPECGKSFSDPGHLVRHQRTHTGEKPYKCPECGKSFSTSGNLVRHQRTHTGEKPYKCPECGKSFSQSSNLVRHQRTHTGAAARALVKSELEEKKSELRHKLKYVPHEYIELIEIARNPTQDRILEMKVMEFFMKVYGYRGEHLGGSRKPDGAIYTVGSPIDYGVIVDTKAYSGGYNLPIGQADEMERYVEENQTRDKHLNPNEWWKVYPSSVTEFKFLFVSGHFKGNYKAQLTRLNHITNCNGAVLSVEELLIGGEMIKAGTLTLEEVRRKFNNGEINF

SEQ ID NO: 452 - protein, 378 aa, Artificial Sequence
  source: /note="Description of Artificial Sequence: Synthetic polypeptide"
MDYKDHDGDYKDHDIDYKDDDDKMAPKKKRKVGRLEPGEKPYKCPECGKSFSQQRSLVGHQRTHTGEKPYKCPECGKSFSDKKDLTRHQRTHTGEKPYKCPECGKSFSTSGHLVRHQRTHTGEKPYKCPECGKSFSQRAHLERHQRTHTGEKPYKCPECGKSFSTSGSLVRHQRTHTGAAARALVKSELEEKKSELRHKLKYVPHEYIELIEIARNPTQDRILEMKVMEFFMKVYGYRGEHLGGSRKPDGAIYTVGSPIDYGVIVDTKAYSGGYNLPIGQADEMQRYVKENQTRNKHINPNEWWKVYPSSVTEFKFLFVSGHFKGNYKAQLTRLNRKTNCNGAVLSVEELLIGGEMIKAGTLTLEEVRRKFNNGEINF

SEQ ID NO: 453 - DNA, 26 bp, Artificial Sequence
  source: /note="Description of Artificial Sequence: Synthetic oligonucleotide"
  Variation (1)..(1): /replace=" "
  Variation (26)..(26): /replace=" "
  misc_feature (1)..(26): /note="Variations given in the sequence have no preference with respect to those in the annotations"
tgccatcttccttgatgttggaggta

SEQ ID NO: 454 - protein, 322 aa, Artificial Sequence
  source: /note="Description of Artificial Sequence: Synthetic polypeptide"
MDYKDHDGDYKDHDIDYKDDDDKMAPKKKRKVGRLEPGERPFQCRICMRNFSSPSKLARHTRTHTGEKPFQCRICMRNFSVRHNLTRHLRTHTGEKPFQCRICMRNFSQRNNLGRHLKTHTGAAARALVKSELEEKKSELRHKLKYVPHEYIELIEIARNPTQDRILEMKVMEFFMKVYGYRGEHLGGSRKPDGAIYTVGSPIDYGVIVDTKAYSGGYNLPIGQADEMQRYVKENQTRNKHINPNEWWKVYPSSVTEFKFLFVSGHFKGNYKAQLTRLNRKTNCNGAVLSVEELLIGGEMIKAGTLTLEEVRRKFNNGEINF

SEQ ID NO: 455 - protein, 322 aa, Artificial Sequence
  source: /note="Description of Artificial Sequence: Synthetic polypeptide"
MDYKDHDGDYKDHDIDYKDDDDKMAPKKKRKVGRLEPGERPFQCRICMRNFSIPNHLARHTRTHTGEKPFQCRICMRNFSQSAHLKRHLRTHTGEKPFQCRICMRNFSHHNSLTRHLKTHTGAAARALVKSELEEKKSELRHKLKYVPHEYIELIEIARNPTQDRILEMKVMEFFMKVYGYRGEHLGGSRKPDGAIYTVGSPIDYGVIVDTKAYSGGYNLPIGQADEMERYVEENQTRDKHLNPNEWWKVYPSSVTEFKFLFVSGHFKGNYKAQLTRLNHITNCNGAVLSVEELLIGGEMIKAGTLTLEEVRRKFNNGEINF

SEQ ID NO: 456 - DNA, 6626 bp, Artificial Sequence
  source: /note="Description of Artificial Sequence: Synthetic polynucleotide"
ggggggggggggggggggttggccactccctctctgcgcgctcgctcgctcactgaggccgggcgaccaaaggtcgcccgacgcccgggctttgcccgggcggcctcagtgagcgagcgagcgcgcagagagggagtggccaactccatcactaggggttcctagatctgaattcggtacccgttacataacttacggtaaatggcccgcctggctgaccgcccaacgacccccgcccattgacgtcaataatgacgtatgttcccatagtaacgccaatagggactttccattgacgtcaatgggtggagtatttacggtaaactgcccacttggcagtacatcaagtgtatcatatgccaagtacgccccctattgacgtcaatgacggtaaatggcccgcctggcattatgcccagtacatgaccttatgggactttcctacttggcagtacatctacgtattagtcatcgctattaccatggtgatgcggttttggcagtacatcaatgggcgtggatagcggtttgactcacggggatttccaagtctccaccccattgacgtcaatgggagtttgttttggcaccaaaatcaacgggactttccaaaatgtcgtaacaactccgccccattgacgcaaatgggcggtaggcgtgtacggtgggaggtctatataagcagagctcgtttagtgaaccgtcagatcgcctggagacgccatccacgctgttttgacctccatagaagacaccgggaccgatccagcctccggactctagaggatccggtactcgaggaactgaaaaaccagaaagttaactggtaagtttagtctttttgtcttttatttcaggtcccggatccggtggtggtgcaaatcaaagaactgctcctcagtggatgttgcctttacttctaggcctgtacggaagtgttacttctgctctaaaagctgcggaattgtacccgcggcccgggatccaccggtggctagcgtctataggcccacccccttggtggaattcgccatgaggtctgactacaaagaccatgacggtgattataaagatcatgacatcgattacaaggatgacgatgacaagatggcccccaagaagaagaggaaggtgggcctcgagcccggagaaaaaccgtacaagtgccctgagtgcgggaaatcattctccgaccctggggcgctcgtccggcaccaaaggacgcatacaggggaaaagccgtataagtgccccgagtgtggaaagagcttctcgcagagagcccaccttgaacgacaccaaagaacacacactggtgagaaaccctataagtgtccagagtgcggcaaatcgtttagcagatccgatgacttggtgcgccaccagcggacacacacgggtgaaaagccctacaaatgcccggagtgtgggaagtcgttttcaaggtcggatcatctgactacccatcagcgcacccatacgggagcggccgcccgcgccctggtgaagagcgagctggaggagaagaagtccgagctgcggcacaagctgaagtacgtgccccacgagtacatcgagctgatcgagatcgccaggaaccccacccaggaccgcatcctggagatgaaggtgatggagttcttcatgaaggtgtacggctacaggggagagcacctgggcggaagcagaaagcctgacggcgccatctatacagtgggcagccccatcgattacggcgtgatcgtggacacaaaggcctacagcggcggctacaatctgcctatcggccaggccgacgagatgcagagatacgtgaaggagaaccagacccggaataagcacatcaaccccaacgagtggtggaaggtgtaccctagcagcgtgaccgagttcaagttcctgttcgtgagcggccacttcaagggcaactacaaggcccagctgaccaggctgaaccgcaaaaccaactgcaatggcgccgtgctgagcgtggaggagctgctgatcggcggcgagatgatcaaagccggcaccctgacactggaggaggtgcggcgcaagttcaacaacggcgagatcaacttcgagggcagaggaagtcttctaacatgcggtgacgtggaggagaatcccggccctagatctgactacaaagaccatgacggtgattataaagatcatgacatcgattacaaggatgacgatgacaagatggcccccaagaagaagaggaaggtgggcctcgagccgggagagaagccgtacaagtgtcccgaatgtggaaagagcttctcacagtcgggggaccttcggcgccaccagcgcacacatactggtgaaaagccgtataagtgtccagaatgtggcaaatcattctccacatcagggagcctggtcaggcaccagcgaacccacacgggtgagaagccctataagtgccccgaatgcgggaagtccttttcgcagagagcccacttggagaggcaccagaggacccatacgggggagaaaccttacaagtgccctgaatgcggaaagtcgttctcgacccatctggatctcatcagacatcagagaacgcacactggagagaaaccctacaaatgtcccgagtgtgggaagtcgtttagccgaaaggacaatctcaaaaaccatcaacggacacacacgggtgaaaaaccatacaaatgcccggagtgcggcaaatcgttttcccaacttgcgcacttgcgggcacaccaacgcacgcatactggagcggccgcccgcgccctggtgaagagcgagctggaggagaagaagtccgagctgcggcacaagctgaagtacgtgccccacgagtacatcgagctgatcgagatcgccaggaaccccacccaggaccgcatcctggagatgaaggtgatggagttcttcatgaaggtgtacggctacaggggagagcacctgggcggaagcagaaagcctgacggcgccatctatacagtgggcagccccatcgattacggcgtgatcgtggacacaaaggcctacagcggcggctacaatctgcctatcggccaggccgacgagatggagagatacgtggaggagaaccagacacgggataagcacctcaaccccaacgagtggtggaaggtgtaccctagcagcgtgaccgagttcaagttcctgttcgtgagcggccacttcaagggcaactacaaggcccagctgaccaggctgaaccacatcaccaactgcaatggcgccgtgctgagcgtggaggagctgctgatcggcggcgagatgatcaaagccggcaccctgacactggaggaggtgcggcgcaagttcaacaacggcgagatcaacttctgattaattaactaatctagagtcgactagagctcgctgatcagcctcgactgtgccttctagttgccagccatctgttgtttgcccctcccccgtgccttccttgaccctggaaggtgccactcccactgtcctttcctaataaaatgaggaaattgcatcgcattgtctgagtaggtgtcattctattctggggggtggggtggggcaggacagcaagggggaggattgggaagacaatagcaggcatgctggggagagatctaggaacccctagtgatggagttggccactccctctctgcgcgctcgctcgctcactgaggccgcccgggcaaagcccgggcgtcgggcgacctttggtcgcccggcctcagtgagcgagcgagcgcgcagagagggagtggccaacccccccccccccccccctgcagcccagctgcattaatgaatcggccaacgcgcggggagaggcggtttgcgtattgggcgctcttccgcttcctcgctcactgactcgctgcgctcggtcgttcggctgcggcgagcggtatcagctcactcaaaggcggtaatacggttatccacagaatcaggggataacgcaggaaagaacatgtgagcaaaaggccagcaaaaggccaggaaccgtaaaaaggccgcgttgctggcgtttttccataggctccgcccccctgacgagcatcacaaaaatcgacgctcaagtcagaggtggcgaaacccgacaggactataaagataccaggcgtttccccctggaagctccctcgtgcgctctcctgttccgaccctgccgcttaccggatacctgtccgcctttctcccttcgggaagcgtggcgctttctcaatgctcacgctgtaggtatctcagttcggtgtaggtcgttcgctccaagctgggctgtgtgcacgaaccccccgttcagcccgaccgctgcgccttatccggtaactatcgtcttgagtccaacccggtaagacacgacttatcgccactggcagcagccactggtaacaggattagcagagcgaggtatgtaggcggtgctacagagttcttgaagtggtggcctaactacggctacactagaaggacagtatttggtatctgcgctctgctgaagccagttaccttcggaaaaagagttggtagctcttgatccggcaaacaaaccaccgctggtagcggtggtttttttgtttgcaagcagcagattacgcgcagaaaaaaaggatctcaagaagatcctttgatcttttctacggggtctgacgctcagtggaacgaaaactcacgttaagggattttggtcatgagattatcaaaaaggatcttcacctagatccttttaaattaaaaatgaagttttaaatcaatctaaagtatatatgagtaaacttggtctgacagttaccaatgcttaatcagtgaggcacctatctcagcgatctgtctatttcgttcatccatagttgcctgactccccgtcgtgtagataactacgatacgggagggcttaccatctggccccagtgctgcaatgataccgcgagacccacgctcaccggctccagatttatcagcaataaaccagccagccggaagggccgagcgcagaagtggtcctgcaactttatccgcctccatccagtctattaattgttgccgggaagctagagtaagtagttcgccagttaatagtttgcgcaacgttgttgccattgctacaggcatcgtggtgtcacgctcgtcgtttggtatggcttcattcagctccggttcccaacgatcaaggcgagttacatgatcccccatgttgtgcaaaaaagcggttagctccttcggtcctccgatcgttgtcagaagtaagttggccgcagtgttatcactcatggttatggcagcactgcataattctcttactgtcatgccatccgtaagatgcttttctgtgactggtgagtactcaaccaagtcattctgagaatagtgtatgcggcgaccgagttgctcttgcccggcgtcaatacgggataataccgcgccacatagcagaactttaaaagtgctcatcattggaaaacgttcttcggggcgaaaactctcaaggatcttaccgctgttgagatccagttcgatgtaacccactcgtgcacccaactgatcttcagcatcttttactttcaccagcgtttctgggtgagcaaaaacaggaaggcaaaatgccgcaaaaaagggaataagggcgacacggaaatgttgaatactcatactcttcctttttcaatattattgaagcatttatcagggttattgtctcatgagcggatacatatttgaatgtatttagaaaaataaacaaataggggttccgcgcacatttccccgaaaagtgccacctgacgtctaagaaaccattattatcatgacattaacctataaaaataggcgtatcacgaggccctttcgtctcgcgcgtttcggtgatgacggtgaaaacctctgacacatgcagctcccggagacggtcacagcttgtctgtaagcggatgccgggagcagacaagcccgtcagggcgcgtcagcgggtgttggcgggtgtcggggctggcttaactatgcggcatcagagcagattgtactgagagtgcaccatatgcggtgtgaaataccgcacagatgcgtaaggagaaaataccgcatcaggaaattgtaaacgttaatattttgttaaaattcgcgttaaatttttgttaaatcagctcattttttaaccaataggccgaaatcggcaaaatcccttataaatcaaaagaatagaccgagatagggttgagtgttgttccagtttggaacaagagtccactattaaagaacgtggactccaacgtcaaagggcgaaaaaccgtctatcagggcgatggcccactacgtgaaccatcaccctaatcaagttttttggggtcgaggtgccgtaaagcactaaatcggaaccctaaagggagcccccgatttagagcttgacggggaaagccggcgaacgtggcgagaaaggaagggaagaaagcgaaaggagcgggcgctagggcgctggcaagtgtagcggtcacgctgcgcgtaaccaccacacccgccgcgcttaatgcgccgctacagggcgcgtcgcgccattcgccattcaggctacgcaactgttgggaagggcgatcggtgcgggcctcttcgctattacgccagctggctgca

SEQ ID NO: 457 - DNA, 22 bp, Artificial Sequence
  source: /note="Description of Artificial Sequence: Synthetic primer"
gagaggttatgtggctttacca

SEQ ID NO: 458 - DNA, 20 bp, Artificial Sequence
  source: /note="Description of Artificial Sequence: Synthetic primer"
ctgcgtagtgccaaaacaaa

SEQ ID NO: 459 - DNA, 3252 bp, Artificial Sequence
  source: /note="Description of Artificial Sequence: Synthetic polynucleotide"
atgaaaaggaactacattctggggctggacatcgggattacaagcgtggggtatgggattattgactatgaaacaagggacgtgatcgacgcaggcgtcagactgttcaaggaggccaacgtggaaaacaatgagggacggagaagcaagaggggagccaggcgcctgaaacgacggagaaggcacagaatccagagggtgaagaaactgctgttcgattacaacctgctgaccgaccattctgagctgagtggaattaatccttatgaagccagggtgaaaggcctgagtcagaagctgtcagaggaagagttttccgcagctctgctgcacctggctaagcgccgaggagtgcataacgtcaatgaggtggaagaggacaccggcaacgagctgtctacaaaggaacagatctcacgcaatagcaaagctctggaagagaagtatgtcgcagagctgcagctggaacggctgaagaaagatggcgaggtgagagggtcaattaataggttcaagacaagcgactacgtcaaagaagccaagcagctgctgaaagtgcagaaggcttaccaccagctggatcagagcttcatcgatacttatatcgacctgctggagactcggagaacctactatgagggaccaggagaagggagccccttcggatggaaagacatcaaggaatggtacgagatgctgatgggacattgcacctattttccagaagagctgagaagcgtcaagtacgcttataacgcagatctgtacaacgccctgaatgacctgaacaacctggtcatcaccagggatgaaaacgagaaactggaatactatgagaagttccagatcatcgaaaacgtgtttaagcagaagaaaaagcctacactgaaacagattgctaaggagatcctggtcaacgaagaggacatcaagggctaccgggtgacaagcactggaaaaccagagttcaccaatctgaaagtgtatcacgatattaaggacatcacagcacggaaagaaatcattgagaacgccgaactgctggatcagattgctaagatcctgactatctaccagagctccgaggacatccaggaagagctgactaacctgaacagcgagctgacccaggaagagatcgaacagattagtaatctgaaggggtacaccggaacacacaacctgtccctgaaagctatcaatctgattctggatgagctgtggcatacaaacgacaatcagattgcaatctttaaccggctgaagctggtcccaaaaaaggtggacctgagtcagcagaaagagatcccaaccacactggtggacgatttcattctgtcacccgtggtcaagcggagcttcatccagagcatcaaagtgatcaacgccatcatcaagaagtacggcctgcccaatgatatcattatcgagctggctagggagaagaacagcaaggacgcacagaagatgatcaatgagatgcagaaacgaaaccggcagaccaatgaacgcattgaagagattatccgaactaccgggaaagagaacgcaaagtacctgattgaaaaaatcaagctgcacgatatgcaggagggaaagtgtctgtattctctggaggccatccccctggaggacctgctgaacaatccattcaactacgaggtcgatcatattatccccagaagcgtgtccttcgacaattcctttaacaacaaggtgctggtcaagcaggaagagaactctaaaaagggcaataggactcctttccagtacctgtctagttcagattccaagatctcttacgaaacctttaaaaagcacattctgaatctggccaaaggaaagggccgcatcagcaagaccaaaaaggagtacctgctggaagagcgggacatcaacagattctccgtccagaaggattttattaaccggaatctggtggacacaagatacgctactcgcggcctgatgaatctgctgcgatcctatttccgggtgaacaatctggatgtgaaagtcaagtccatcaacggcgggttcacatcttttctgaggcgcaaatggaagtttaaaaaggagcgcaacaaagggtacaagcaccatgccgaagatgctctgattatcgcaaatgccgacttcatctttaaggagtggaaaaagctggacaaagccaagaaagtgatggagaaccagatgttcgaagagaagcaggccgaatctatgcccgaaatcgagacagaacaggagtacaaggagattttcatcactcctcaccagatcaagcatatcaaggatttcaaggactacaagtactctcaccgggtggataaaaagcccaacagagagctgatcaatgacaccctgtatagtacaagaaaagacgataaggggaataccctgattgtgaacaatctgaacggactgtacgacaaagataatgacaagctgaaaaagctgatcaacaaaagtcccgagaagctgctgatgtaccaccatgatcctcagacatatcagaaactgaagctgattatggagcagtacggcgacgagaagaacccactgtataagtactatgaagagactgggaactacctgaccaagtatagcaaaaaggataatggccccgtgatcaagaagatcaagtactatgggaacaagctgaatgcccatctggacatcacagacgattaccctaacagtcgcaacaaggtggtcaagctgtcactgaagccatacagattcgatgtctatctggacaacggcgtgtataaatttgtgactgtcaagaatctggatgtcatcaaaaaggagaactactatgaagtgaatagcaagtgctacgaagaggctaaaaagctgaaaaagattagcaaccaggcagagttcatcgcctccttttacaacaacgacctgattaagatcaatggcgaactgtatagggtcatcggggtgaacaatgatctgctgaaccgcattgaagtgaatatgattgacatcacttaccgagagtatctggaaaacatgaatgataagcgcccccctcgaattatcaaaacaattgcctctaagactcagagtatcaaaaagtactcaaccgacattctgggaaacctgtatgaggtgaagagcaaaaagcaccctcagattatcaaaaagggcagcggaggcaagcgtcctgctgctactaagaaagctggtcaagctaagaaaaagaaaggatcctacccatacgatgttccagattacgcttaa

SEQ ID NO: 460 - DNA, 83 bp, Artificial Sequence
  source: /note="Description of Artificial Sequence: Synthetic oligonucleotide"
gttttagtactctggaaacagaatctactaaaacaaggcaaaatgccgtgtttatctcgtcaacttgttggcgagattttttt

SEQ ID NO: 461 - DNA, 3333 bp, Artificial Sequence
  source: /note="Description of Artificial Sequence: Synthetic polynucleotide"
atggtgcctaagaagaagagaaaggtggctgccttcaaacctaattcaatcaactacatcctcggcctcgatatcggcatcgcatccgtcggctgggcgatggtagaaattgacgaagaagaaaaccccatccgcctgattgatttgggcgtgcgcgtatttgagcgtgccgaagtaccgaaaacaggcgactcccttgccatggcaaggcgtttggcgcgcagtgttcgccgcctgacccgccgtcgcgcccaccgcctgcttcggacccgccgcctattgaaacgcgaaggcgtattacaagccgccaattttgacgaaaacggcttgattaaatccttaccgaatacaccatggcaacttcgcgcagccgcattagaccgcaaactgacgcctttagagtggtcggcagtcttgttgcatttaatcaaacatcgcggctatttatcgcaacggaaaaacgagggcgaaactgccgataaggagcttggcgctttgcttaaaggcgtagccggcaatgcccatgccttacagacaggcgatttccgcacaccggccgaattggctttaaataaatttgagaaagaaagcggccatatccgcaatcagcgcagcgattattcgcatacgttcagccgcaaagatttacaggcggagctgattttgctgtttgaaaaacaaaaagaatttggcaatccgcatgtttcaggcggccttaaagaaggtattgaaaccctactgatgacgcaacgccctgccctgtccggcgatgccgttcaaaaaatgttggggcattgcaccttcgaaccggcagagccgaaagccgctaaaaacacctacacagccgaacgtttcatctggctgaccaagctgaacaacctgcgtattttagagcaaggcagcgagcggccattgaccgataccgaacgcgccacgcttatggacgagccatacagaaaatccaaactgacttacgcacaagcccgtaagctgctgggtttagaagataccgcctttttcaaaggcttgcgctatggtaaagacaatgccgaagcctcaacattgatggaaatgaaggcctaccatgccatcagccgtgcactggaaaaagaaggattgaaagacaaaaaatccccattaaacctttctcccgaattacaagacgaaatcggcacggcattctccctgttcaaaaccgatgaagacattacaggccgtctgaaagaccgtatacagcccgaaatcttagaagcgctgttgaaacacatcagcttcgataagttcgtccaaatttccttgaaagcattgcgccgaattgtgcctctaatggaacaaggcaaacgttacgatgaagcctgcgccgaaatctacggagaccattacggcaagaagaatacggaagaaaagatttatctgccgccgattcccgccgacgaaatccgcaaccccgtcgtcttgcgcgccttatctcaagcacgtaaggtcattaacggcgtggtacgccgttacggctccccagctcgtatccatattgaaactgcaagggaagtaggtaaatcgtttaaagaccgcaaagaaattgagaaacgccaagaagaaaaccgcaaagaccgggaaaaagccgccgccaaattccgagagtatttccccaattttgtcggagaacccaaatccaaagatattctgaaactgcgcctgtacgagcaacaacacggcaaatgcctgtattcgggcaaagaaatcaacttaggccgtctgaacgaaaaaggctatgtcgaaatcgaccatgccctgccgttctcgcgcacatgggacgacagtttcaacaataaagtactggtattgggcagcgaaaaccaaaacaaaggcaatcaaaccccttacgaatacttcaacggcaaagacaacagccgcgaatggcaggaatttaaagcgcgtgtcgaaaccagccgtttcccgcgcagtaaaaaacaacggattctgctgcaaaaattcgatgaagacggctttaaagaacgcaatctgaacgacacgcgctacgtcaaccgtttcctgtgtcaatttgttgccgaccgtatgcggctgacaggtaaaggcaagaaacgtgtctttgcatccaacggacaaattaccaatctgttgcgcggcttttggggattgcgcaaagtgcgtgcggaaaacgaccgccatcacgccttggacgccgtcgtcgttgcctgctcgaccgttgccatgcagcagaaaattacccgttttgtacgctataaagagatgaacgcgtttgacggtaaaaccatagacaaagaaacaggagaagtgctgcatcaaaaaacacacttcccacaaccttgggaatttttcgcacaagaagtcatgattcgcgtcttcggcaaaccggacggcaaacccgaattcgaagaagccgataccctagaaaaactgcgcacgttgcttgccgaaaaattatcatctcgccccgaagccgtacacgaatacgttacgccactgtttgtttcacgcgcgcccaatcggaagatgagcgggcaagggcatatggagaccgtcaaatccgccaaacgactggacgaaggcgtcagcgtgttgcgcgtaccgctgacacagttaaaactgaaagacttggaaaaaatggtcaatcgggagcgcgaacctaagctatacgaagcactgaaagcacggctggaagcacataaagacgatcctgccaaagcctttgccgagccgttttacaaatacgataaagcaggcaaccgcacccaacaggtaaaagccgtacgcgtagagcaagtacagaaaaccggcgtatgggtgcgcaaccataacggtattgccgacaacgcaaccatggtgcgcgtagatgtgtttgagaaaggcgacaagtattatctggtaccgatttacagttggcaggtagcgaaagggattttgccggatagggctgttgtacaaggaaaagatgaagaagattggcaacttattgatgatagtttcaactttaaattctcattacaccctaatgatttagtcgaggttataacaaaaaaagctagaatgtttggttactttgccagctgccatcgaggcacaggtaatatcaatatacgcattcatgatcttgatcataaaattggcaaaaatggaatactggaaggtatcggcgtcaaaaccgccctttcattccaaaaataccaaattgacgaactgggcaaagaaatcagaccatgccgtctgaaaaaacgcccgcctgtccgttacccatacgatgttccagattacgctgcagctccagcagcgaagaaaaagaagctggattaa

SEQ ID NO: 462 - DNA, 120 bp, Artificial Sequence
  source: /note="Description of Artificial Sequence: Synthetic polynucleotide"
gttgtagctccctttctcatttcggaaacgaaatgagaaccgttgctacaataaggccgtctgaaaagatgtgccgcaacgctctgccccttaaagcttctgctttaaggggcttttttt

SEQ ID NO: 463 - DNA, 144 bp, Artificial Sequence
  source: /note="Description of Artificial Sequence: Synthetic polynucleotide"
gttgtagctccctttctcatttcgcagtgctacaatgaaaattgtcgcactgcgaaatgagaaccgttgctacaataaggccgtctgaaaagatgtgccgcaacgctctgccccttaaagcttctgctttaaggggcttttttt

SEQ ID NO: 464 - DNA, 24 bp, Artificial Sequence
  source: /note="Description of Artificial Sequence: Synthetic primer"
tcgggtttattacagggacagcag

SEQ ID NO: 465 - DNA, 24 bp, Artificial Sequence
  source: /note="Description of Artificial Sequence: Synthetic primer"
tctaaggccgagtcttatgagcag

SEQ ID NO: 466 - DNA, 4564 bp, Artificial Sequence
  source: /note="Description of Artificial Sequence: Synthetic polynucleotide"
atggactacaaagaccatgacggtgattataaagatcatgacatcgattacaaggatgacgatgacaagatggcccccaagaagaagaggaaggtgggccgcggaatggacaagaagtactccattgggctcgccatcggcacaaacagcgtcggctgggccgtcattacggacgagtacaaggtgccgagcaaaaaattcaaagttctgggcaataccgatcgccacagcataaagaagaacctcattggcgccctcctgttcgactccggggaaaccgccgaagccacgcggctcaaaagaacagcacggcgcagatatacccgcagaaagaatcggatctgctacctgcaggagatctttagtaatgagatggctaaggtggatgactctttcttccataggctggaggagtcctttttggtggaggaggataaaaagcacgagcgccacccaatctttggcaatatcgtggacgaggtggcgtaccatgaaaagtacccaaccatatatcatctgaggaagaagcttgtagacagtactgataaggctgacttgcggttgatctatctcgcgctggcgcatatgatcaaatttcggggacacttcctcatcgagggggacctgaacccagacaacagcgatgtcgacaaactctttatccaactggttcagacttacaatcagcttttcgaagagaacccgatcaacgcatccggagttgacgccaaagcaatcctgagcgctaggctgtccaaatcccggcggctcgaaaacctcatcgcacagctccctggggagaagaagaacggcctgtttggtaatcttatcgccctgtcactcgggctgacccccaactttaaatctaacttcgacctggccgaagatgccaagcttcaactgagcaaagacacctacgatgatgatctcgacaatctgctggcccagatcggcgaccagtacgcagacctttttttggcggcaaagaacctgtcagacgccattctgctgagtgatattctgcgagtgaacacggagatcaccaaagctccgctgagcgctagtatgatcaagcgctatgatgagcaccaccaagacttgactttgctgaaggcccttgtcagacagcaactgcctgagaagtacaaggaaattttcttcgatcagtctaaaaatggctacgccggatacattgacggcggagcaagccaggaggaattttacaaatttattaagcccatcttggaaaaaatggacggcaccgaggagctgctggtaaagcttaacagagaagatctgttgcgcaaacagcgcactttcgacaatggaagcatcccccaccagattcacctgggcgaactgcacgctatcctcaggcggcaagaggatttctacccctttttgaaagataacagggaaaagattgagaaaatcctcacatttcggataccctactatgtaggccccctcgcccggggaaattccagattcgcgtggatgactcgcaaatcagaagagaccatcactccctggaacttcgaggaagtcgtggataagggggcctctgcccagtccttcatcgaaaggatgactaactttgataaaaatctgcctaacgaaaaggtgcttcctaaacactctctgctgtacgagtacttcacagtttataacgagctcaccaaggtcaaatacgtcacagaagggatgagaaagccagcattcctgtctggagagcagaagaaagctatcgtggacctcctcttcaagacgaaccggaaagttaccgtgaaacagctcaaagaagactatttcaaaaagattgaatgtttcgactctgttgaaatcagcggagtggaggatcgcttcaacgcatccctgggaacgtatcacgatctcctgaaaatcattaaagacaaggacttcctggacaatgaggagaacgaggacattcttgaggacattgtcctcacccttacgttgtttgaagatagggagatgattgaagaacgcttgaaaacttacgctcatctcttcgacgacaaagtcatgaaacagctcaagaggcgccgatatacaggatgggggcggctgtcaagaaaactgatcaatgggatccgagacaagcagagtggaaagacaatcctggattttcttaagtccgatggatttgccaaccggaacttcatgcagttgatccatgatgactctctcacctttaaggaggacatccagaaagcacaagtttctggccagggggacagtcttcacgagcacatcgctaatcttgcaggtagcccagctatcaaaaagggaatactgcagaccgttaaggtcgtggatgaactcgtcaaagtaatgggaaggcataagcccgagaatatcgttatcgagatggcccgagagaaccaaactacccagaagggacagaagaacagtagggaaaggatgaagaggattgaagagggtataaaagaactggggtcccaaatccttaaggaacacccagttgaaaacacccagcttcagaatgagaagctctacctgtactacctgcagaacggcagggacatgtacgtggatcaggaactggacatcaatcggctctccgactacgacgtggatgccatcgtgccccagtcttttctcaaagatgattctattgataataaagtgttgacaagatccgataaaaatagagggaagagtgataacgtcccctcagaagaagttgtcaagaaaatgaaaaattattggcggcagctgctgaacgccaaactgatcacacaacggaagttcgataatctgactaaggctgaacgaggtggcctgtctgagttggataaagccggcttcatcaaaaggcagcttgttgagacacgccagatcaccaagcacgtggcccaaattctcgattcacgcatgaacaccaagtacgatgaaaatgacaaactgattcgagaggtgaaagttattactctgaagtctaagctggtctcagatttcagaaaggactttcagttttataaggtgagagagatcaacaattaccaccatgcgcatgatgcctacctgaatgcagtggtaggcactgcacttatcaaaaaatatcccaagcttgaatctgaatttgtttacggagactataaagtgtacgatgttaggaaaatgatcgcaaagtctgagcaggaaataggcaaggccaccgctaagtacttcttttacagcaatattatgaattttttcaagaccgagattacactggccaatggagagattcggaagcgaccacttatcgaaacaaacggagaaacaggagaaatcgtgtgggacaagggtagggatttcgcgacagtccggaaggtcctgtccatgccgcaggtgaacatcgttaaaaagaccgaagtacagaccggaggcttctccaaggaaagtatcctcccgaaaaggaacagcgacaagctgatcgcacgcaaaaaagattgggaccccaagaaatacggcggattcgattctcctacagtcgcttacagtgtactggttgtggccaaagtggagaaagggaagtctaaaaaactcaaaagcgtcaaggaactgctgggcatcacaatcatggagcgatcaagcttcgaaaaaaaccccatcgactttctcgaggcgaaaggatataaagaggtcaaaaaagacctcatcattaagcttcccaagtactctctctttgagcttgaaaacggccggaaacgaatgctcgctagtgcgggcgagctgcagaaaggtaacgagctggcactgccctctaaatacgttaatttcttgtatctggccagccactatgaaaagctcaaagggtctcccgaagataatgagcagaagcagctgttcgtggaacaacacaaacactaccttgatgagatcatcgagcaaataagcgaattctccaaaagagtgatcctcgccgacgctaacctcgataaggtgctttctgcttacaataagcacagggataagcccatcagggagcaggcagaaaacattatccacttgtttactctgaccaacttgggcgcgcctgcagccttcaagtacttcgacaccaccatagacagaaagcggtacacctctacaaaggaggtcctggacgccacactgattcatcagtcaattacggggctctatgaaacaagaatcgacctctctcagctcggtggagacagcagggctgaccccaagaagaagaggaaggtggctagcgatgctaagtcactgactgcctggtcccggacactggtgaccttcaaggatgtgtttgtggacttcaccagggaggagtggaagctgctggacactgctcagcagatcctgtacagaaatgtgatgctggagaactataagaacctggtttccttgggttatcagcttactaagccagatgtgatcctccggttggagaagggagaagagccctggctggtggagagagaaattcaccaagagacccatcctgattcagagactgcatttgaaatcaaatcatcagttccgaaaaagaaacgcaaagttgctagcg

SEQ ID NO: 467 - DNA, 388 bp, Artificial Sequence
  source: /note="Description of Artificial Sequence: Synthetic polynucleotide"
taagcttcagtttttccttagttcctgttacatttctgtgtgtctccattagtgacctcccatagtccaagcatgagcagttctggccaggcccctgtcggggtcagtgccccacccccgccttctggttctgtgtaaccttctaagcaaaccttctggctcaagcacagcaatgctgagtcatgatgagtcatgctgaggcttagggtgtgtgcccagatgttctcagcctagagtgatgactcctatctgggtccccagcaggatgcttacagggcagatggcaaaaaaaaggagaagctgaccacctgactaaaactccacctcaaacggcatcataaagaaaatggatgcctgagacagaatgtgacatattctagaatatatt

SEQ ID NO: 468 - DNA, 19 bp, Artificial Sequence
  source: /note="Description of Artificial Sequence: Synthetic oligonucleotide"
cagccgctcgctgcagcag

SEQ ID NO: 469 - DNA, 19 bp, Artificial Sequence
  source: /note="Description of Artificial Sequence: Synthetic oligonucleotide"
ctgctgcagcgagcggctg

SEQ ID NO: 470 - DNA, 19 bp, Artificial Sequence
  source: /note="Description of Artificial Sequence: Synthetic oligonucleotide"
gctgggtgtcccattgaaa

SEQ ID NO: 471 - DNA, 19 bp, Artificial Sequence
  source: /note="Description of Artificial Sequence: Synthetic oligonucleotide"
tttcaatgggacacccagc

SEQ ID NO: 472 - DNA, 19 bp, Artificial Sequence
  source: /note="Description of Artificial Sequence: Synthetic oligonucleotide"
gtttattcagccgggagtc

SEQ ID NO: 473 - DNA, 19 bp, Artificial Sequence
  source: /note="Description of Artificial Sequence: Synthetic oligonucleotide"
gactcccggctgaataaac

SEQ ID NO: 474 - DNA, 19 bp, Artificial Sequence
  source: /note="Description of Artificial Sequence: Synthetic oligonucleotide"
tggagagtttgcaaggagc

SEQ ID NO: 475 - DNA, 19 bp, Artificial Sequence
  source: /note="Description of Artificial Sequence: Synthetic oligonucleotide"
gctccttgcaaactctcca

SEQ ID NO: 476 - DNA, 19 bp, Artificial Sequence
  source: /note="Description of Artificial Sequence: Synthetic oligonucleotide"
ccctccagactttccacct

SEQ ID NO: 477 - DNA, 19 bp, Artificial Sequence
  source: /note="Description of Artificial Sequence: Synthetic oligonucleotide"
aggtggaaagtctggaggg

SEQ ID NO: 478 - DNA, 19 bp, Artificial Sequence
  source: /note="Description of Artificial Sequence: Synthetic oligonucleotide"
aattttcttccaagttctc

SEQ ID NO: 479 - DNA, 19 bp, Artificial Sequence
  source: /note="Description of Artificial Sequence: Synthetic oligonucleotide"
gagaacttggaagaaaatt

SEQ ID NO: 480 - DNA, 19 bp, Artificial Sequence
  source: /note="Description of Artificial Sequence: Synthetic oligonucleotide"
ctgcggagagaagaaaggg

SEQ ID NO: 481 - DNA, 19 bp, Artificial Sequence
  source: /note="Description of Artificial Sequence: Synthetic oligonucleotide"
ccctttcttctctccgcag

SEQ ID NO: 482 - DNA, 19 bp, Artificial Sequence
  source: /note="Description of Artificial Sequence: Synthetic oligonucleotide"
agagccaccccctggctcc

SEQ ID NO: 483 - DNA, 19 bp, Artificial Sequence
  source: /note="Description of Artificial Sequence: Synthetic oligonucleotide"
ggagccagggggtggctct

SEQ ID NO: 484 - DNA, 19 bp, Artificial Sequence
  source: /note="Description of Artificial Sequence: Synthetic oligonucleotide"
cgaagccaaccgcggcggg

SEQ ID NO: 485 - DNA, 19 bp, Artificial Sequence
  source: /note="Description of Artificial Sequence: Synthetic oligonucleotide"
cccgccgcggttggcttcg

SEQ ID NO: 486 - DNA, 19 bp, Artificial Sequence
  source: /note="Description of Artificial Sequence: Synthetic oligonucleotide"
agagggaagacgatcgccc

SEQ ID NO: 487 - DNA, 19 bp, Artificial Sequence
  source: /note="Description of Artificial Sequence: Synthetic oligonucleotide"
gggcgatcgtcttccctct

SEQ ID NO: 488 - DNA, 19 bp, Artificial Sequence
  source: /note="Description of Artificial Sequence: Synthetic oligonucleotide"
cccctttaactttcctccg

SEQ ID NO: 489 - DNA, 19 bp, Artificial Sequence
  source: /note="Description of Artificial Sequence: Synthetic oligonucleotide"
cggaggaaagttaaagggg

SEQ ID NO: 490 - DNA, 19 bp, Artificial Sequence
  source: /note="Description of Artificial Sequence: Synthetic oligonucleotide"
gcagccccgcttccttcaa

SEQ ID NO: 491 - DNA, 19 bp, Artificial Sequence
  source: /note="Description of Artificial Sequence: Synthetic oligonucleotide"
ttgaaggaagcggggctgc

SEQ ID NO: 492 - DNA, 24 bp, Artificial Sequence
  source: /note="Description of Artificial Sequence: Synthetic oligonucleotide"
caccgcagccgctcgctgcagcag

SEQ ID NO: 493 - DNA, 24 bp, Artificial Sequence
  source: /note="Description of Artificial Sequence: Synthetic oligonucleotide"
aaacctgctgcagcgagcggctgc

SEQ ID NO: 494 - DNA, 24 bp, Artificial Sequence
  source: /note="Description of Artificial Sequence: Synthetic oligonucleotide"
caccggctgggtgtcccattgaaa

SEQ ID NO: 495 - DNA, 24 bp, Artificial Sequence
  source: /note="Description of Artificial Sequence: Synthetic oligonucleotide"
aaactttcaatgggacacccagcc

SEQ ID NO: 496 - DNA, 24 bp, Artificial Sequence
  source: /note="Description of Artificial Sequence: Synthetic oligonucleotide"
caccggtttattcagccgggagtc

SEQ ID NO: 497 - DNA, 24 bp, Artificial Sequence
  source: /note="Description of Artificial Sequence: Synthetic oligonucleotide"
aaacgactcccggctgaataaacc

SEQ ID NO: 498 - DNA, 24 bp, Artificial Sequence
  source: /note="Description of Artificial Sequence: Synthetic oligonucleotide"
caccgtggagagtttgcaaggagc

SEQ ID NO: 499 - DNA, 24 bp, Artificial Sequence
  source: /note="Description of Artificial Sequence: Synthetic oligonucleotide"
aaacgctccttgcaaactctccac

SEQ ID NO: 500 - DNA, 24 bp, Artificial Sequence
  source: /note="Description of Artificial Sequence: Synthetic oligonucleotide"
caccgccctccagactttccacct

SEQ ID NO: 501 - DNA, 24 bp, Artificial Sequence
  source: /note="Description of Artificial Sequence: Synthetic oligonucleotide"
aaacaggtggaaagtctggagggc

SEQ ID NO: 502 - DNA, 24 bp, Artificial Sequence
  source: /note="Description of Artificial Sequence: Synthetic oligonucleotide"
caccgaattttcttccaagttctc

SEQ ID NO: 503 - DNA, 24 bp, Artificial Sequence
  source: /note="Description of Artificial Sequence: Synthetic oligonucleotide"
aaacgagaacttggaagaaaattc

SEQ ID NO: 504 - DNA, 24 bp, Artificial Sequence
  source: /note="Description of Artificial Sequence: Synthetic oligonucleotide"
caccgctgcggagagaagaaaggg

SEQ ID NO: 505 - DNA, 24 bp, Artificial Sequence
  source: /note="Description of Artificial Sequence: Synthetic oligonucleotide"
aaacccctttcttctctccgcagc

SEQ ID NO: 506 - DNA, 24 bp, Artificial Sequence
  source: /note="Description of Artificial Sequence: Synthetic oligonucleotide"
caccgagagccaccccctggctcc

SEQ ID NO: 507 - DNA, 24 bp, Artificial Sequence
  source: /note="Description of Artificial Sequence: Synthetic oligonucleotide"
aaacggagccagggggtggctctc

SEQ ID NO: 508 - DNA, 24 bp, Artificial Sequence
  source: /note="Description of Artificial Sequence: Synthetic oligonucleotide"
caccgcgaagccaaccgcggcggg

SEQ ID NO: 509 - DNA, 24 bp, Artificial Sequence
  source: /note="Description of Artificial Sequence: Synthetic oligonucleotide"
aaaccccgccgcggttggcttcgc

SEQ ID NO: 510 - DNA, 24 bp, Artificial Sequence
  source: /note="Description of Artificial Sequence: Synthetic oligonucleotide"
caccgagagggaagacgatcgccc

SEQ ID NO: 511 - DNA, 24 bp, Artificial Sequence
  source: /note="Description of Artificial Sequence: Synthetic oligonucleotide"
aaacgggcgatcgtcttccctctc

SEQ ID NO: 512 - DNA, 24 bp, Artificial Sequence
  source: /note="Description of Artificial Sequence: Synthetic oligonucleotide"
caccgcccctttaactttcctccg

SEQ ID NO: 513 - DNA, 24 bp, Artificial Sequence
  source: /note="Description of Artificial Sequence: Synthetic oligonucleotide"
aaaccggaggaaagttaaaggggc

SEQ ID NO: 514 - DNA, 24 bp, Artificial Sequence
  source: /note="Description of Artificial Sequence: Synthetic oligonucleotide"
caccggcagccccgcttccttcaa

SEQ ID NO: 515 - DNA, 24 bp, Artificial Sequence
  source: /note="Description of Artificial Sequence: Synthetic oligonucleotide"
aaacttgaaggaagcggggctgcc

SEQ ID NO: 516 - DNA, 19 bp, Artificial Sequence
  source: /note="Description of Artificial Sequence: Synthetic oligonucleotide"
cgagagcgagaggagggag

SEQ ID NO: 517 - DNA, 19 bp, Artificial Sequence
  source: /note="Description of Artificial Sequence: Synthetic oligonucleotide"
ctccctcctctcgctctcg

SEQ ID NO: 518 - DNA, 19 bp, Artificial Sequence
  source: /note="Description of Artificial Sequence: Synthetic oligonucleotide"
gagagagcttgagagcgcg

SEQ ID NO: 519 - DNA, 19 bp, Artificial Sequence
  source: /note="Description of Artificial Sequence: Synthetic oligonucleotide"
cgcgctctcaagctctctc

SEQ ID NO: 520 - DNA, 19 bp, Artificial Sequence
  source: /note="Description of Artificial Sequence: Synthetic oligonucleotide"
ggtggagggggcggggccc

SEQ ID NO: 521 - DNA, 19 bp, Artificial Sequence
  source: /note="Description of Artificial Sequence: Synthetic oligonucleotide"
gggccccgccccctccacc

SEQ ID NO: 522 - DNA, 19 bp, Artificial Sequence
  source: /note="Description of Artificial Sequence: Synthetic oligonucleotide"
ggtatccacgtaaatcaaa

SEQ ID NO: 523 - DNA, 19 bp, Artificial Sequence
  source: /note="Description of Artificial Sequence: Synthetic oligonucleotide"
tttgatttacgtggatacc

SEQ ID NO: 524 - DNA, 19 bp, Artificial Sequence
  source: /note="Description of Artificial Sequence: Synthetic oligonucleotide"
ccaatcactggctccggtc

SEQ ID NO: 525 - DNA, 19 bp, Artificial Sequence
  source: /note="Description of Artificial Sequence: Synthetic oligonucleotide"
gaccggagccagtgattgg

SEQ ID NO: 526 - DNA, 19 bp, Artificial Sequence
  source: /note="Description of Artificial Sequence: Synthetic oligonucleotide"
ggcgcccgagggaagaaga

SEQ ID NO: 527 - DNA, 19 bp, Artificial Sequence
  source: /note="Description of Artificial Sequence: Synthetic oligonucleotide"
tcttcttccctcgggcgcc

SEQ ID NO: 528 - DNA, 19 bp, Artificial Sequence
  source: /note="Description of Artificial Sequence: Synthetic oligonucleotide"
gggtgggggtaccagagga

SEQ ID NO: 529 - DNA, 19 bp, Artificial Sequence
  source: /note="Description of Artificial Sequence: Synthetic oligonucleotide"
tcctctggtacccccaccc

SEQ ID NO: 530 - DNA, 19 bp, Artificial Sequence
  source: /note="Description of Artificial Sequence: Synthetic oligonucleotide"
ccggggacagaagagaggg

SEQ ID NO: 531 - DNA, 19 bp, Artificial Sequence
  source: /note="Description of Artificial Sequence: Synthetic oligonucleotide"
ccctctcttctgtccccgg

SEQ ID NO: 532 - DNA, 19 bp, Artificial Sequence
  source: /note="Description of Artificial Sequence: Synthetic oligonucleotide"
gagagagagtgggagaagc

SEQ ID NO: 533 - DNA, 19 bp, Artificial Sequence
  source: /note="Description of Artificial Sequence: Synthetic oligonucleotide"
gcttctcccactctctctc

SEQ ID NO: 534 - DNA, 19 bp, Artificial Sequence
  source: /note="Description of Artificial Sequence: Synthetic oligonucleotide"
aaagtaactgtcaaatgcg

SEQ ID NO: 535 - DNA, 19 bp, Artificial Sequence
  source: /note="Description of Artificial Sequence: Synthetic oligonucleotide"
cgcatttgacagttacttt

SEQ ID NO: 536 - DNA, 19 bp, Artificial Sequence
  source: /note="Description of Artificial Sequence: Synthetic oligonucleotide"
ttaaccagagcgcccagtc

SEQ ID NO: 537 - DNA, 19 bp, Artificial Sequence
  source: /note="Description of Artificial Sequence: Synthetic oligonucleotide"
gactgggcgctctggttaa

SEQ ID NO: 538 - DNA, 19 bp, Artificial Sequence
  source: /note="Description of Artificial Sequence: Synthetic oligonucleotide"
cgtcggagctgcccgctag

SEQ ID NO: 539 - DNA, 19 bp, Artificial Sequence
  source: /note="Description of Artificial Sequence: Synthetic oligonucleotide"
ctagcgggcagctccgacg

SEQ ID NO: 540 - DNA, 24 bp, Artificial Sequence
  source: /note="Description of Artificial Sequence: Synthetic oligonucleotide"
caccgcgagagcgagaggagggag

SEQ ID NO: 541 - DNA, 24 bp, Artificial Sequence
  source: /note="Description of Artificial Sequence: Synthetic oligonucleotide"
aaacctccctcctctcgctctcgc

SEQ ID NO: 542 - DNA, 24 bp, Artificial Sequence
  source: /note="Description of Artificial Sequence: Synthetic oligonucleotide"
caccggagagagcttgagagcgcg

SEQ ID NO: 543 - DNA, 24 bp, Artificial Sequence
  source: /note="Description of Artificial Sequence: Synthetic oligonucleotide"
aaaccgcgctctcaagctctctcc

SEQ ID NO: 544 - DNA, 24 bp, Artificial Sequence
  source: /note="Description of Artificial Sequence: Synthetic oligonucleotide"
caccgggtggagggggcggggccc

SEQ ID NO: 545 - DNA, 24 bp, Artificial Sequence
  source: /note="Description of Artificial Sequence: Synthetic oligonucleotide"
aaacgggccccgccccctccaccc

SEQ ID NO: 546 - DNA, 24 bp, Artificial Sequence
  source: /note="Description of Artificial Sequence: Synthetic oligonucleotide"
caccgggtatccacgtaaatcaaa

SEQ ID NO: 547 - DNA, 24 bp, Artificial Sequence
  source: /note="Description of Artificial Sequence: Synthetic oligonucleotide"
aaactttgatttacgtggataccc

SEQ ID NO: 548 - DNA, 24 bp, Artificial Sequence
  source: /note="Description of Artificial Sequence: Synthetic oligonucleotide"
caccgccaatcactggctccggtc

SEQ ID NO: 549 - DNA, 24 bp, Artificial Sequence
  source: /note="Description of Artificial Sequence: Synthetic oligonucleotide"
aaacgaccggagccagtgattggc

SEQ ID NO: 550 - DNA, 24 bp, Artificial Sequence
  source: /note="Description of Artificial Sequence: Synthetic oligonucleotide"
caccgggcgcccgagggaagaaga

SEQ ID NO: 551 - DNA, 24 bp, Artificial Sequence
  source: /note="Description of Artificial Sequence: Synthetic oligonucleotide"
aaactcttcttccctcgggcgccc

SEQ ID NO: 552 - DNA, 24 bp, Artificial Sequence
  source: /note="Description of Artificial Sequence: Synthetic oligonucleotide"
caccggggtgggggtaccagagga

SEQ ID NO: 553 - DNA, 24 bp, Artificial Sequence
  source: /note="Description of Artificial Sequence: Synthetic oligonucleotide"
aaactcctctggtacccccacccc

SEQ ID NO: 554 - DNA, 24 bp, Artificial Sequence
  source: /note="Description of Artificial Sequence: Synthetic oligonucleotide"
caccgccggggacagaagagaggg

SEQ ID NO: 555 - DNA, 24 bp, Artificial Sequence
  source: /note="Description of Artificial Sequence: Synthetic oligonucleotide"
aaacccctctcttctgtccccggc

SEQ ID NO: 556 - DNA, 24 bp, Artificial Sequence
  source: /note="Description of Artificial Sequence: Synthetic oligonucleotide"
caccggagagagagtgggagaagc

SEQ ID NO: 557 - DNA, 24 bp, Artificial Sequence
  source: /note="Description of Artificial Sequence: Synthetic oligonucleotide"
aaacgcttctcccactctctctcc

SEQ ID NO: 558 - DNA, 24 bp, Artificial Sequence
  source: /note="Description of Artificial Sequence: Synthetic oligonucleotide"
caccgaaagtaactgtcaaatgcg

SEQ ID NO: 559 - DNA, 24 bp, Artificial Sequence
  source: /note="Description of Artificial Sequence: Synthetic oligonucleotide"
aaaccgcatttgacagttactttc

SEQ ID NO: 560 - DNA, 24 bp, Artificial Sequence
  source: /note="Description of Artificial Sequence: Synthetic oligonucleotide"
caccgttaaccagagcgcccagtc

SEQ ID NO: 561 - DNA, 24 bp, Artificial Sequence
  source: /note="Description of Artificial Sequence: Synthetic oligonucleotide"
aaacgactgggcgctctggttaac

SEQ ID NO: 562 - DNA, 24 bp, Artificial Sequence
  source: /note="Description of Artificial Sequence: Synthetic oligonucleotide"
caccgcgtcggagctgcccgctag

SEQ ID NO: 563 - DNA, 24 bp, Artificial Sequence
  source: /note="Description of Artificial Sequence: Synthetic oligonucleotide"
aaacctagcgggcagctccgacgc

SEQ ID NO: 564 - DNA, 20 bp, Artificial Sequence
  source: /note="Description of Artificial Sequence: Synthetic oligonucleotide"
gagacacacagaaatgtaac

SEQ ID NO: 565 - DNA, 20 bp, Artificial Sequence
  source: /note="Description of Artificial Sequence: Synthetic oligonucleotide"
ggtggggcactgaccccgac

SEQ ID NO: 566 - DNA, 20 bp, Artificial Sequence
  source: /note="Description of Artificial Sequence: Synthetic oligonucleotide"
ctagagtgatgactcctatc

SEQ ID NO: 567 - DNA, 20 bp, Artificial Sequence
  source: /note="Description of Artificial Sequence: Synthetic oligonucleotide"
gactaaaactccacctcaaa

SEQ ID NO: 568 - DNA, 20 bp, Artificial Sequence
  source: /note="Description of Artificial Sequence: Synthetic oligonucleotide"
aatatgtcacattctgtctc

SEQ ID NO: 569 - DNA, 20 bp, Artificial Sequence
  source: /note="Description of Artificial Sequence: Synthetic oligonucleotide"
ggactatgggaggtcactaa

SEQ ID NO: 570 - DNA, 20 bp, Artificial Sequence
  source: /note="Description of Artificial Sequence: Synthetic oligonucleotide"
gctcatgcttggactatggg

SEQ ID NO: 571 - DNA, 20 bp, Artificial Sequence
  source: /note="Description of Artificial Sequence: Synthetic oligonucleotide"
gttctggccaggcccctgtc

SEQ ID NO: 572 - DNA, 20 bp, Artificial Sequence
  source: /note="Description of Artificial Sequence: Synthetic oligonucleotide"
agtgccccacccccgccttc

SEQ ID NO: 573 - DNA, 20 bp, Artificial Sequence
  source: /note="Description of Artificial Sequence: Synthetic oligonucleotide"
gtggggcactgaccccgaca

SEQ ID NO: 574 - DNA, 20 bp, Artificial Sequence
  source: /note="Description of Artificial Sequence: Synthetic oligonucleotide"
aaccttctaagcaaaccttc

SEQ ID NO: 575 - DNA, 20 bp, Artificial Sequence
  source: /note="Description of Artificial Sequence: Synthetic oligonucleotide"
gttacacagaaccagaaggc

SEQ ID NO: 576 - DNA, 20 bp, Artificial Sequence
  source: /note="Description of Artificial Sequence: Synthetic oligonucleotide"
gaaggttacacagaaccaga

SEQ ID NO: 577 - DNA, 20 bp, Artificial Sequence
  source: /note="Description of Artificial Sequence: Synthetic oligonucleotide"
agtcatgatgagtcatgctg

SEQ ID NO: 578 - DNA, 20 bp, Artificial Sequence
  source: /note="Description of Artificial Sequence: Synthetic oligonucleotide"
gatgagtcatgctgaggctt

SEQ ID NO: 579 - DNA, 20 bp, Artificial Sequence
  source: /note="Description of Artificial Sequence: Synthetic oligonucleotide"
actctaggctgagaacatct

SEQ ID NO: 580 - DNA, 20 bp, Artificial Sequence
  source: /note="Description of Artificial Sequence: Synthetic oligonucleotide"
gtccccagcaggatgcttac

SEQ ID NO: 581 - DNA, 20 bp, Artificial Sequence
  source: /note="Description of Artificial Sequence: Synthetic oligonucleotide"
gccctgtaagcatcctgctg

SEQ ID NO: 582 - DNA, 20 bp, Artificial Sequence
  source: /note="Description of Artificial Sequence: Synthetic oligonucleotide"
cagggcagatggcaaaaaaa

SEQ ID NO: 583 - DNA, 20 bp, Artificial Sequence
  source: /note="Description of Artificial Sequence: Synthetic oligonucleotide"
gaggtggagttttagtcagg

SEQ ID NO: 584 - DNA, 20 bp, Artificial Sequence
  source: /note="Description of Artificial Sequence: Synthetic oligonucleotide"
aaacggcatcataaagaaaa

SEQ ID NO: 585 - DNA, 105 bp, Artificial Sequence
  source: /note="Description of Artificial Sequence: Synthetic polynucleotide"
gagacacacagaaatgtaacgttttagagctagaaatagcaagttaaaataaggctagtccgttatcaacttgaaaaagtggcaccgagtcggtgctttttttcc

SEQ ID NO: 586 - DNA, 105 bp, Artificial Sequence
  source: /note="Description of Artificial Sequence: Synthetic polynucleotide"
ggtggggcactgaccccgacgttttagagctagaaatagcaagttaaaataaggctagtccgttatcaacttgaaaaagtggcaccgagtcggtgctttttttcc

SEQ ID NO: 587 - DNA, 105 bp, Artificial Sequence
  source: /note="Description of Artificial Sequence: Synthetic polynucleotide"
ctagagtgatgactcctatcgttttagagctagaaatagcaagttaaaataaggctagtccgttatcaacttgaaaaagtggcaccgagtcggtgctttttttcc

SEQ ID NO: 588 - DNA, 105 bp, Artificial Sequence
  source: /note="Description of Artificial Sequence: Synthetic polynucleotide"
gactaaaactccacctcaaagttttagagctagaaatagcaagttaaaataaggctagtccgttatcaacttgaaaaagtggcaccgagtcggtgctttttttcc

SEQ ID NO: 589 - DNA, 105 bp, Artificial Sequence
  source: /note="Description of Artificial Sequence: Synthetic polynucleotide"
aatatgtcacattctgtctcgttttagagctagaaatagcaagttaaaataaggctagtccgttatcaacttgaaaaagtggcaccgagtcggtgctttttttcc

SEQ ID NO: 590 - DNA, 105 bp, Artificial Sequence
  source: /note="Description of Artificial Sequence: Synthetic polynucleotide"
ggactatgggaggtcactaagttttagagctagaaatagcaagttaaaataaggctagtccgttatcaacttgaaaaagtggcaccgagtcggtgctttttttcc

SEQ ID NO: 591 - DNA, 105 bp, Artificial Sequence
  source: /note="Description of Artificial Sequence: Synthetic polynucleotide"
gctcatgcttggactatggggttttagagctagaaatagcaagttaaaataaggctagtccgttatcaacttgaaaaagtggcaccgagtcggtgctttttttcc

SEQ ID NO: 592 - DNA, 105 bp, Artificial Sequence
  source: /note="Description of Artificial Sequence: Synthetic polynucleotide"
gttctggccaggcccctgtcgttttagagctagaaatagcaagttaaaataaggctagtccgttatcaacttgaaaaagtggcaccgagtcggtgctttttttcc

SEQ ID NO: 593 - DNA, 105 bp, Artificial Sequence
  source: /note="Description of Artificial Sequence: Synthetic polynucleotide"
agtgccccacccccgccttcgttttagagctagaaatagcaagttaaaataaggctagtccgttatcaacttgaaaaagtggcaccgagtcggtgctttttttcc

SEQ ID NO: 594 - DNA, 105 bp, Artificial Sequence
  source: /note="Description of Artificial Sequence: Synthetic polynucleotide"
gtggggcactgaccccgacagttttagagctagaaatagcaagttaaaataaggctagtccgttatcaacttgaaaaagtggcaccgagtcggtgctttttttcc

SEQ ID NO: 595 - DNA, 105 bp, Artificial Sequence
  source: /note="Description of Artificial Sequence: Synthetic polynucleotide"
aaccttctaagcaaaccttcgttttagagctagaaatagcaagttaaaataaggctagtccgttatcaacttgaaaaagtggcaccgagtcggtgctttttttcc

SEQ ID NO: 596 - DNA, 105 bp, Artificial Sequence
  source: /note="Description of Artificial Sequence: Synthetic polynucleotide"
gttacacagaaccagaaggcgttttagagctagaaatagcaagttaaaataaggctagtccgttatcaacttgaaaaagtggcaccgagtcggtgctttttttcc

SEQ ID NO: 597 - DNA, 105 bp, Artificial Sequence
  source: /note="Description of Artificial Sequence: Synthetic polynucleotide"
gaaggttacacagaaccagagttttagagctagaaatagcaagttaaaataaggctagtccgttatcaacttgaaaaagtggcaccgagtcggtgctttttttcc

SEQ ID NO: 598 - DNA, 105 bp, Artificial Sequence
  source: /note="Description of Artificial Sequence: Synthetic polynucleotide"
agtcatgatgagtcatgctggttttagagctagaaatagcaagttaaaataaggctagtccgttatcaacttgaaaaagtggcaccgagtcggtgctttttttcc

SEQ ID NO: 599 - DNA, 105 bp, Artificial Sequence
  source: /note="Description of Artificial Sequence: Synthetic polynucleotide"
gatgagtcatgctgaggcttgttttagagctagaaatagcaagttaaaataaggctagtccgttatcaacttgaaaaagtggcaccgagtcggtgctttttttcc

SEQ ID NO: 600 - DNA, 105 bp, Artificial Sequence
  source: /note="Description of Artificial Sequence: Synthetic polynucleotide"
actctaggctgagaacatctgttttagagctagaaatagcaagttaaaataaggctagtccgttatcaacttgaaaaagtggcaccgagtcggtgctttttttcc

SEQ ID NO: 601 - DNA, 105 bp, Artificial Sequence
  source: /note="Description of Artificial Sequence: Synthetic polynucleotide"
gtccccagcaggatgcttacgttttagagctagaaatagcaagttaaaataaggctagtccgttatcaacttgaaaaagtggcaccgagtcggtgctttttttcc

SEQ ID NO: 602 - DNA, 105 bp, Artificial Sequence
  source: /note="Description of Artificial Sequence: Synthetic polynucleotide"
gccctgtaagcatcctgctggttttagagctagaaatagcaagttaaaataaggctagtccgttatcaacttgaaaaagtggcaccgagtcggtgctttttttcc

SEQ ID NO: 603 - DNA, 105 bp, Artificial Sequence
  source: /note="Description of Artificial Sequence: Synthetic polynucleotide"
cagggcagatggcaaaaaaagttttagagctagaaatagcaagttaaaataaggctagtccgttatcaacttgaaaaagtggcaccgagtcggtgctttttttcc

SEQ ID NO: 604 - DNA, 105 bp, Artificial Sequence
  source: /note="Description of Artificial Sequence: Synthetic polynucleotide"
gaggtggagttttagtcagggttttagagctagaaatagcaagttaaaataaggctagtccgttatcaacttgaaaaagtggcaccgagtcggtgctttttttcc

SEQ ID NO: 605 - DNA, 105 bp, Artificial Sequence
  source: /note="Description of Artificial Sequence: Synthetic polynucleotide"
aaacggcatcataaagaaaagttttagagctagaaatagcaagttaaaataaggctagtccgttatcaacttgaaaaagtggcaccgagtcggtgctttttttcc

SEQ ID NO: 606 - DNA, 19 bp, Artificial Sequence
  source: /note="Description of Artificial Sequence: Synthetic oligonucleotide"
tgtactctctgaggtgctc

SEQ ID NO: 607 - DNA, 19 bp, Artificial Sequence
  source: /note="Description of Artificial Sequence: Synthetic oligonucleotide"
acgcagataagaaccagtt

SEQ ID NO: 608 - DNA, 19 bp, Artificial Sequence
  source: /note="Description of Artificial Sequence: Synthetic oligonucleotide"
catcaagtcagccatcagc

SEQ ID NO: 609 - DNA, 19 bp, Artificial Sequence
  source: /note="Description of Artificial Sequence: Synthetic oligonucleotide"
gagtcaccctcctggaaac

SEQ ID NO: 610 - DNA, 19 bp, Artificial Sequence
  source: /note="Description of Artificial Sequence: Synthetic oligonucleotide"
cctgggctccggggcgttt

SEQ ID NO: 611 - DNA, 19 bp, Artificial Sequence
  source: /note="Description of Artificial Sequence: Synthetic oligonucleotide"
ggcccctgcggccaccccg

SEQ ID NO: 612 - DNA, 19 bp, Artificial Sequence
  source: /note="Description of Artificial Sequence: Synthetic oligonucleotide"
ctccctccctgcccggtag

SEQ ID NO: 613 - DNA, 19 bp, Artificial Sequence
  source: /note="Description of Artificial Sequence: Synthetic oligonucleotide"
aggtttggaaagggcgtgc

SEQ ID NO: 614 - DNA, 20 bp, Artificial Sequence
  source: /note="Description of Artificial Sequence: Synthetic oligonucleotide"
actccactgcactccagtct

SEQ ID NO: 615 - DNA, 20 bp, Artificial Sequence
  source: /note="Description of Artificial Sequence: Synthetic oligonucleotide"
tctgtgggggacctgcactg

SEQ ID NO: 616 - DNA, 20 bp, Artificial Sequence
  source: /note="Description of Artificial Sequence: Synthetic oligonucleotide"
ggggcgccagttgtgtctcc

SEQ ID NO: 617 - DNA, 20 bp, Artificial Sequence
  source: /note="Description of Artificial Sequence: Synthetic oligonucleotide"
acaccattgccaccaccatt

SEQ ID NO: 618 - DNA, 20 bp, Artificial Sequence
  source: /note="Description of Artificial Sequence: Synthetic primer"
caatgaccccttcattgacc

SEQ ID NO: 619 - DNA, 20 bp, Artificial Sequence
  source: /note="Description of Artificial Sequence: Synthetic primer"
ttgattttggagggatctcg

SEQ ID NO: 620 - DNA, 20 bp, Artificial Sequence
  source: /note="Description of Artificial Sequence: Synthetic primer"
ggaatccatggagggaagat

SEQ ID NO: 621 - DNA, 20 bp, Artificial Sequence
  source: /note="Description of Artificial Sequence: Synthetic primer"
tgttctcgctcaggtcagtg

SEQ ID NO: 622 - DNA, 20 bp, Artificial Sequence
  source: /note="Description of Artificial Sequence: Synthetic primer"
ctctctgctcctttgccaca

SEQ ID NO: 623 - DNA, 20 bp, Artificial Sequence
  source: /note="Description of Artificial Sequence: Synthetic primer"
gtgctcttcgggtttcagga

SEQ ID NO: 624 - DNA, 30 bp, Artificial Sequence
  source: /note="Description of Artificial Sequence: Synthetic primer"
cgaaagagaaagcgaaccagtatcgagaac

SEQ ID NO: 625 - DNA, 27 bp, Artificial Sequence
  source: /note="Description of Artificial Sequence: Synthetic primer"
cgttgtgcatagtcgctgcttgatcgc

SEQ ID NO: 626 - DNA, 25 bp, Artificial Sequence
  source: /note="Description of Artificial Sequence: Synthetic primer"
gagtttggctcaaattgttactctt

SEQ ID NO: 627 - DNA, 25 bp, Artificial Sequence
  source: /note="Description of Artificial Sequence: Synthetic primer"
gggaaatggtctaggagagtaaagt

SEQ ID NO: 628 - DNA, 23 bp, Artificial Sequence
  source: /note="Description of Artificial Sequence: Synthetic oligonucleotide"
gattggctttgatttccctaggg

SEQ ID NO: 629 - DNA, 23 bp, Artificial Sequence
  source: /note="Description of Artificial Sequence: Synthetic oligonucleotide"
gcctactcagactgttactctgg

SEQ ID NO: 630 - DNA, 23 bp, Artificial Sequence
  source: /note="Description of Artificial Sequence: Synthetic oligonucleotide"
gcagttgcctaagaactggtggg

SEQ ID NO: 631 - DNA, 23 bp, Artificial Sequence
  source: /note="Description of Artificial Sequence: Synthetic oligonucleotide"
ggggctccaccctcacgagtggg

SEQ ID NO: 632 - DNA, 23 bp, Artificial Sequence
  source: /note="Description of Artificial Sequence: Synthetic oligonucleotide"
gccttctttatcccctatcgagg

SEQ ID NO: 633 - DNA, 48 bp, Artificial Sequence
  source: /note="Description of Artificial Sequence: Synthetic oligonucleotide"
  CDS (1)..(45)
gaaggaccatttgacgttcagctcctactcagactgttactctggtga

SEQ ID NO: 634 - protein, 15 aa, Artificial Sequence
  source: /note="Description of Artificial Sequence: Synthetic peptide"
EGPFDVQLLLRLLLW

SEQ ID NO: 635 - DNA, 46 bp, Artificial Sequence
  source: /note="Description of Artificial Sequence: Synthetic oligonucleotide"
  CDS (1)..(42)
gaaggaccatttgacgttcagctcctactcagactgtctctggtga

SEQ ID NO: 636 - protein, 14 aa, Artificial Sequence
  source: /note="Description of Artificial Sequence: Synthetic peptide"
EGPFDVQLLLRLSL

SEQ ID NO: 637 - RNA, 20 nt, Artificial Sequence
  source: /note="Description of Artificial Sequence: Synthetic oligonucleotide"
gccuacucagacuguuacuc

SEQ ID NO: 638 - DNA, 19 bp, Artificial Sequence
  source: /note="Description of Artificial Sequence: Synthetic oligonucleotide"
cccaccagttcttaggcaa

SEQ ID NO: 639 - DNA, 20 bp, Artificial Sequence
  source: /note="Description of Artificial Sequence: Synthetic oligonucleotide"
cccaccagttcttaggcaac

SEQ ID NO: 640 - DNA, 20 bp, Artificial Sequence
  source: /note="Description of Artificial Sequence: Synthetic oligonucleotide"
tttgatttccagttcttagg

SEQ ID NO: 641 - DNA, 19 bp, Artificial Sequence
  source: /note="Description of Artificial Sequence: Synthetic oligonucleotide"
attaccatagagttcttag

SEQ ID NO: 642 - DNA, 19 bp, Artificial Sequence
  source: /note="Description of Artificial Sequence: Synthetic oligonucleotide"
gtggataaaggcaacaatg

SEQ ID NO: 643 - DNA, 16 bp, Artificial Sequence
  source: /note="Description of Artificial Sequence: Synthetic oligonucleotide"
cctcgataggggataa

SEQ ID NO: 644 - DNA, 23 bp, Artificial Sequence
  source: /note="Description of Artificial Sequence: Synthetic oligonucleotide"
accaaacccacttaggggataaa

SEQ ID NO: 645 - DNA, 21 bp, Artificial Sequence
  source: /note="Description of Artificial Sequence: Synthetic oligonucleotide"
ggtatcttaaggacctccaag

SEQ ID NO: 646 - DNA, 47 bp, Artificial Sequence
  source: /note="Description of Artificial Sequence: Synthetic oligonucleotide"
taggaagtaaattaatttgaagcttgccaattaatccaaatcttacc

SEQ ID NO: 647 - DNA, 83 bp, Artificial Sequence
  source: /note="Description of Artificial Sequence: Synthetic primer"
tttcctttttgcaaaacccaaaatattttagctcctactcagactgttagagtaggaggagaaggagggctgtggctcttgtg

SEQ ID NO: 648 - DNA, 83 bp, Artificial Sequence
  source: /note="Description of Artificial Sequence: Synthetic primer"
  modified_base (20)..(20): a, c, t, g, unknown or other
  modified_base (31)..(31): a, c, t, g, unknown or other
  modified_base (69)..(69): a, c, t, g, unknown or other
aaaacccccaaaccctcccnctttttcctcntactctaacagtgtgagtaggaggccacacttagctgnggctctagtaagtc

SEQ ID NO: 649 - DNA, 94 bp, Artificial Sequence
  source: /note="Description of Artificial Sequence: Synthetic primer"
  modified_base (50)..(50): a, c, t, g, unknown or other
cttcttttttcctttttgcaaaaacccaaaatattttagctcctactcanaccgttttcggggggtattttgtatttggatgaaacacttgatg

SEQ ID NO: 650 - DNA, 93 bp, Artificial Sequence
  source: /note="Description of Artificial Sequence: Synthetic primer"
tcttcttttttccttcccgcaaaaacccaaaatattttcgctcctactcaggacctggtcgtggggtattttgtatttggatgaaacacttga

SEQ ID NO: 651 - DNA, 104 bp, Artificial Sequence
  source: /note="Description of Artificial Sequence: Synthetic primer"
  modified_base (21)..(22): a, c, t, g, unknown or other
tcaaggaagatggcatttctnntttggagatggcagtttccttagtaaccacaggttgtgtcaccatggccagtaagaaggatgccacacttgtgtgtgtcgct

SEQ ID NO: 652 - DNA, 86 bp, Artificial Sequence
  source: /note="Description of Artificial Sequence: Synthetic primer"
  modified_base (35)..(36): a, c, t, g, unknown or other
  modified_base (42)..(44): a, c, t, g, unknown or other
ttggagatagcagtttccttggtaagtacaggttnntcaccnnnacagtgtgagtaggaggccacacttagctgtggctctagtaa

SEQ ID NO: 653 - DNA, 71 bp, Artificial Sequence
  source: /note="Description of Artificial Sequence: Synthetic primer"
  modified_base (54)..(54): a, c, t, g, unknown or other
  modified_base (61)..(63): a, c, t, g, unknown or other
  modified_base (69)..(69): a, c, t, g, unknown or other
tttctagtttggagatggcagtttccttagtaaccacaggttgtgtcaccaggnctcgagnnntggttntg

SEQ ID NO: 654 - DNA, 87 bp, Artificial Sequence
  source: /note="Description of Artificial Sequence: Synthetic primer"
cagttgccatagtcttcactaaccgcgtcaccagagctcaggacctggtcgtggggtattttgtatttggatgaaacacttgatggt

SEQ ID NO: 655 - DNA, 92 bp, Artificial Sequence
  source: /note="Description of Artificial Sequence: Synthetic primer"
  modified_base (52)..(52): a, c, t, g, unknown or other
  modified_base (59)..(59): a, c, t, g, unknown or other
  modified_base (78)..(78): a, c, t, g, unknown or other
tattgtatcttggtttttcttcactgctggccagtttactaacaatctgaantaagccnattaatccaaatcttaccngacgaaaaatcaaa

SEQ ID NO: 656 - DNA, 89 bp, Artificial Sequence
  source: /note="Description of Artificial Sequence: Synthetic primer"
  modified_base (6)..(6): a, c, t, g, unknown or other
  modified_base (10)..(10): a, c, t, g, unknown or other
  modified_base (19)..(19): a, c, t, g, unknown or other
  modified_base (30)..(30): a, c, t, g, unknown or other
  modified_base (57)..(57): a, c, t, g, unknown or other
atggtntttngtcattgcnggccagttttntaacaatgtgatcaatgccaattaatncaaatcttaccagaggaaaaatcaagccacag

SEQ ID NO: 657 - DNA, 94 bp, Artificial Sequence
  source: /note="Description of Artificial Sequence: Synthetic primer"
  modified_base (93)..(94): a, c, t, g, unknown or other
aataaaaagaaaaaaatatgataaactgctcccagtataaaatacagagctaagacaagaacgtttcattggctgttaaaagtcggaaatcgnn

SEQ ID NO: 658 - DNA, 94 bp, Artificial Sequence
  source: /note="Description of Artificial Sequence: Synthetic primer"
ttctgatttaaaattcccttgaataggaagtaaattaatttgaagcttgccaattaatccaaatcttaccagaggaaaaatcaagccacagata

SEQ ID NO: 659 - DNA, 90 bp, Artificial Sequence
  source: /note="Description of Artificial Sequence: Synthetic primer"
caaaacaagatgggataaaatcttctttctgatttaaaattcccttgaataggaagtaaattactagagctgttcaaggcctgaactcta

SEQ ID NO: 660 - DNA, 96 bp, Artificial Sequence
  source: /note="Description of Artificial Sequence: Synthetic primer"
  modified_base (49)..(49): a, c, t, g, unknown or other
  modified_base (51)..(52): a, c, t, g, unknown or other
  modified_base (54)..(54): a, c, t, g, unknown or other
ctgatttaaaattcccttgaataggaagtaaattactagagctgttcangnncngaactctaggctagcatttccagcccaaaacaaacacagttc

SEQ ID NO: 661 - DNA, 26 bp, Artificial Sequence
  source: /note="Description of Artificial Sequence: Synthetic oligonucleotide"
  modified_base (8)..(26): a, c, t, g, unknown or other
ttgtttgnnnnnnnnnnnnnnnnnnn

SEQ ID NO: 662 - DNA, 24 bp, Artificial Sequence
  source: /note="Description of Artificial Sequence: Synthetic oligonucleotide"
  modified_base (6)..(24): a, c, t, g, unknown or other
caccgnnnnnnnnnnnnnnnnnnn

SEQ ID NO: 663 - DNA, 24 bp, Artificial Sequence
  source: /note="Description of Artificial Sequence: Synthetic oligonucleotide"
  modified_base (6)..(24): a, c, t, g, unknown or other
tcccannnnnnnnnnnnnnnnnnn

SEQ ID NO: 664 - DNA, 24 bp, Artificial Sequence
  source: /note="Description of Artificial Sequence: Synthetic oligonucleotide"
  modified_base (6)..(24): a, c, t, g, unknown or other
cctcgnnnnnnnnnnnnnnnnnnn

SEQ ID NO: 665 - DNA, 26 bp, Artificial Sequence
  source: /note="Description of Artificial Sequence: Synthetic oligonucleotide"
  modified_base (5)..(23): a, c, t, g, unknown or other
aaacnnnnnnnnnnnnnnnnnnncaa

SEQ ID NO: 666 - DNA, 24 bp, Artificial Sequence
  source: /note="Description of Artificial Sequence: Synthetic oligonucleotide"
  modified_base (5)..(23): a, c, t, g, unknown or other
aaacnnnnnnnnnnnnnnnnnnnc

SEQ ID NO: 667 - DNA, 24 bp, Artificial Sequence
  source: /note="Description of Artificial Sequence: Synthetic oligonucleotide"
  modified_base (5)..(23): a, c, t, g, unknown or other
aaacnnnnnnnnnnnnnnnnnnnt

SEQ ID NO: 668 - DNA, 24 bp, Artificial Sequence
  source: /note="Description of Artificial Sequence: Synthetic oligonucleotide"
  modified_base (5)..(23): a, c, t, g, unknown or other
aaacnnnnnnnnnnnnnnnnnnnc

SEQ ID NO: 669 - DNA, 26 bp, Artificial Sequence
  source: /note="Description of Artificial Sequence: Synthetic oligonucleotide"
ttgtttgtcttcgagaagacctgttt

SEQ ID NO: 670 - DNA, 26 bp, Artificial Sequence
  source: /note="Description of Artificial Sequence: Synthetic oligonucleotide"
caccgggtcttcgagaagacctgttt

SEQ ID NO: 671 - DNA, 26 bp, Artificial Sequence
  source: /note="Description of Artificial Sequence: Synthetic oligonucleotide"
tcccaggtcttcgagaagacctgttt

SEQ ID NO: 672 - DNA, 26 bp, Artificial Sequence
  source: /note="Description of Artificial Sequence: Synthetic oligonucleotide"
cctcgggtcttcgagaagacctgttt

SEQ ID NO: 673 - DNA, 25 bp, Artificial Sequence
  source: /note="Description of Artificial Sequence: Synthetic oligonucleotide"
ggcctaccgctaaggctagcctagt

SEQ ID NO: 674 - protein, 1411 aa, Artificial Sequence
  source: /note="Description of Artificial Sequence: Synthetic polypeptide"
MDYKDHDGDYKDHDIDYKDDDDKMAPKKKRKVGRGMDKKYSIGLAIGTNSVGWAVITDEYKVPSKKFKVLGNTDRHSIKKNLIGALLFDSGETAEATRLKRTARRRYTRRKNRICYLQEIFSNEMAKVDDSFFHRLEESFLVEEDKKHERHPIFGNIVDEVAYHEKYPTIYHLRKKLVDSTDKADLRLIYLALAHMIKFRGHFLIEGDLNPDNSDVDKLFIQLVQTYNQLFEENPINASGVDAKAILSARLSKSRRLENLIAQLPGEKKNGLFGNLIALSLGLTPNFKSNFDLAEDAKLQLSKDTYDDDLDNLLAQIGDQYADLFLAAKNLSDAILLSDILRVNTEITKAPLSASMIKRYDEHHQDLTLLKALVRQQLPEKYKEIFFDQSKNGYAGYIDGGASQEEFYKFIKPILEKMDGTEELLVKLNREDLLRKQRTFDNGSIPHQIHLGELHAILRRQEDFYPFLKDNREKIEKILTFRIPYYVGPLARGNSRFAWMTRKSEETITPWNFEEVVDKGASAQSFIERMTNFDKNLPNEKVLPKHSLLYEYFTVYNELTKVKYVTEGMRKPAFLSGEQKKAIVDLLFKTNRKVTVKQLKEDYFKKIECFDSVEISGVEDRFNASLGTYHDLLKIIKDKDFLDNEENEDILEDIVLTLTLFEDREMIEERLKTYAHLFDDKVMKQLKRRRYTGWGRLSRKLINGIRDKQSGKTILDFLKSDGFANRNFMQLIHDDSLTFKEDIQKAQVSGQGDSLHEHIANLAGSPAIKKGILQTVKVVDELVKVMGRHKPENIVIEMARENQTTQKGQKNSRERMKRIEEGIKELGSQILKEHPVENTQLQNEKLYLYYLQNGRDMYVDQELDINRLSDYDVDHIVPQSFLKDDSIDNKVLTRSDKNRGKSDNVPSEEVVKKMKNYWRQLLNAKLITQRKFDNLTKAERGGLSELDKAGFIKRQLVETRQITKHVAQILDSRMNTKYDENDKLIREVKVITLKSKLVSDFRKDFQFYKVREINNYHHAHDAYLNAVVGTALIKKYPKLESEFVYGDYKVYDVRKMIAKSEQEIGKATAKYFFYSNIMNFFKTEITLANGEIRKRPLIETNGETGEIVWDKGRDFATVRKVLSMPQVNIVKKTEVQTGGFSKESILPKRNSDKLIARKKDWDPKKYGGFDSPTVAYSVLVVAKVEKGKSKKLKSVKELLGITIMERSSFEKNPIDFLEAKGYKEVKKDLIIKLPKYSLFELENGRKRMLASAGELQKGNELALPSKYVNFLYLASHYEKLKGSPEDNEQKQLFVEQHKHYLDEIIEQISEFSKRVILADANLDKVLSAYNKHRDKPIREQAENIIHLFTLTNLGAPAAFKYFDTTIDRKRYTSTKEVLDATLIHQSITGLYETRIDLSQLGGDPKKKRKVG

SEQ ID NO: 675 - protein, 1483 aa, Artificial Sequence; identical to SEQ ID NO: 1
  source: /note="Description of Artificial Sequence: Synthetic polypeptide"

SEQ ID NO: 676 - protein, 2048 aa, Artificial Sequence
  source: /note="Description of Artificial Sequence: Synthetic polypeptide"
MDYKDHDGDYKDHDIDYKDDDDKMAPKKKRKVGRGMDKKYSIGLAIGTNSVGWAVITDEYKVPSKKFKVLGNTDRHSIKKNLIGALLFDSGETAEATRLKRTARRRYTRRKNRICYLQEIFSNEMAKVDDSFFHRLEESFLVEEDKKHERHPIFGNIVDEVAYHEKYPTIYHLRKKLVDSTDKADLRLIYLALAHMIKFRGHFLIEGDLNPDNSDVDKLFIQLVQTYNQLFEENPINASGVDAKAILSARLSKSRRLENLIAQLPGEKKNGLFGNLIALSLGLTPNFKSNFDLAEDAKLQLSKDTYDDDLDNLLAQIGDQYADLFLAAKNLSDAILLSDILRVNTEITKAPLSASMIKRYDEHHQDLTLLKALVRQQLPEKYKEIFFDQSKNGYAGYIDGGASQEEFYKFIKPILEKMDGTEELLVKLNREDLLRKQRTFDNGSIPHQIHLGELHAILRRQEDFYPFLKDNREKIEKILTFRIPYYVGPLARGNSRFAWMTRKSEETITPWNFEEVVDKGASAQSFIERMTNFDKNLPNEKVLPKHSLLYEYFTVYNELTKVKYVTEGMRKPAFLSGEQKKAIVDLLFKTNRKVTVKQLKEDYFKKIECFDSVEISGVEDRFNASLGTYHDLLKIIKDKDFLDNEENEDILEDIVLTLTLFEDREMIEERLKTYAHLFDDKVMKQLKRRRYTGWGRLSRKLINGIRDKQSGKTILDFLKSDGFANRNFMQLIHDDSLTFKEDIQKAQVSGQGDSLHEHIANLAGSPAIKKGILQTVKVVDELVKVMGRHKPENIVIEMARENQTTQKGQKNSRERMKRIEEGIKELGSQILKEHPVENTQLQNEKLYLYYLQNGRDMYVDQELDINRLSDYDVDAIVPQSFLKDDSIDNKVLTRSDKNRGKSDNVPSEEVVKKMKNYWRQLLNAKLITQRKFDNLTKAERGGLSELDKAGFIKRQLVETRQITKHVAQILDSRMNTKYDENDKLIREVKVITLKSKLVSDFRKDFQFYKVREINNYHHAHDAYLNAVVGTALIKKYPKLESEFVYGDYKVYDVRKMIAKSEQEIGKATAKYFFYSNIMNFFKTEITLANGEIRKRPLIETNGETGEIVWDKGRDFATVRKVLSMPQVNIVKKTEVQTGGFSKESILPKRNSDKLIARKKDWDPKKYGGFDSPTVAYSVLVVAKVEKGKSKKLKSVKELLGITIMERSSFEKNPIDFLEAKGYKEVKKDLIIKLPKYSLFELENGRKRMLASAGELQKGNELALPSKYVNFLYLASHYEKLKGSPEDNEQKQLFVEQHKHYLDEIIEQISEFSKRVILADANLDKVLSAYNKHRDKPIREQAENIIHLFTLTNLGAPAAFKYFDTTIDRKRYTSTKEVLDATLIHQSITGLYETRIDLSQLGGDPIAGSKASPKKKRKVGRAIFKPEELRQALMPTLEALYRQDPESLPFRQPVDPQLLGIPDYFDIVKSPMDLSTIKRKLDTGQYQEPWQYVDDIWLMFNNAWLYNRKTSRVYKYCSKLSEVFEQEIDPVMQSLGYCCGRKLEFSPQTLCCYGKQLCTIPRDATYYSYQNRYHFCEKCFNEIQGESVSLGDDPSQPQTTINKEQFSKRKNDTLDPELFVECTECGRKMHQICVLHHEIIWPAGFVCDGCLKKSARTRKENKFSAKRLPSTRLGTFLENRVNDFLRRQNHPESGEVTVRVVHASDKTVEVKPGMKARFVDSGEMAESFPYRTKALFAFEEIDGVDLCFFGMHVQEYGSDCPPPNQRRVYISYLDSVHFFRPKCLRTAVYHEILIGYLEYVKKLGYTTGHIWACPPSEGDDYIFHCHPPDQKIPKPKRLQEWYKKMLDKAVSERIVHDYKDIFKQATEDRLTSAKELPYFEGDFWPNVLEESIKELEQEEEERKREENTSNESTDVTKGDSKNAKKKNNKKTSKNKSSLSRGNKKKPGMPNVSNDLSQKLYATMEKHKEVFFVIRLIAGPAANSLPPIVDPDPLIPCDLMDGRDAFLTLARDKHLEFSSLRRAQWSTMCMLVELHTQSQDYPYDVPDYAS